European Patent Application EP 4 219 549 A1, published August 2, 2023. Title: SPLIT INTEINS, CONJUGATES AND USES THEREOF. Applicant: THE TRUSTEES OF PRINCETON UNIVERSITY. The sequence listing filed with the application follows.

SEQUENCE LISTING (777 sequences)

SEQ ID NO: 1 - protein, 102 aa, Nostoc punctiforme
CLSYETEILTVEYGLLPIGKIVEKRIECTVYSVDNNGNIYTQPVAQWHDRGEQEVFEYCLEDGSLIRATKDHKFMTVDGQMLPIDEIFERELDLMRVDNLPN

SEQ ID NO: 2 - protein, 123 aa, Synechocystis PCC6803
CLSFGTEILTVEYGPLPIGKIVSEEINCSVYSVDPEGRVYTQAIAQWHDRGEQEVLEYELEDGSVIRATSDHRFLTTDYQLLAIEEIFARQLDLLTLENIKQTEEALDNHRLPFPLLDAGTIK

SEQ ID NO: 3 - protein, 110 aa, Aphanothece halophytica
CLSYDTEIWTVEYGAMPIGKIVEEKIECSVYTVDENGFVYTQPIAQWHPRGQQEIIEYTLEDGRKIRATKDHKMMTESGEMLPIEEIFQRELDLKVETFHEMSLLRRGAK

SEQ ID NO: 4 - protein, 101 aa, Aphanizomenon ovalisporum
CLSADTEILTVEYGFLPIGEIVGKAIECRVYSVDGNGNIYTQSIAQWHNRGEQEVFEYTLEDGSIIRATKDHKFMTTDGEMLPIDEIFARQLDLMQVQGLH

SEQ ID NO: 5 - protein, 102 aa, Anabaena PCC7120
CLSYDTEVLTVEYGFVPIGEIVEKGIECSVFSINNNGIVYTQPIAQWHHRGKQEVFEYCLEDGSIIKATKDHKFMTQDGKMLPIDEIFEQELDLLQVKGLPE

SEQ ID NO: 6 - protein, 102 aa, Anabaena variabilis
CLSYDTEVLTVEYGFVPIGEIVDKGIECSVFSIDSNGIVYTQPIAQWHHRGKQEVFEYCLEDGSIIKATKDHKFMTQDGKMLPIDEIFEQELDLLQVKGLPE

SEQ ID NO: 7 - protein, 118 aa, Cylindrospermopsis raciborskii
CLSYETEVLTLEYGFVPIGEIVNKQMVCTVFSLNDSGNVYTQPIGQWHDRGVQDLYEYCLDDGSTIRATKDHKFMTTQGEMVPIDEIFHQGWELVQVSGISKLVQQRTLPFIIVDRKL

SEQ ID NO: 8 - protein, 99 aa, Cyanothece CCY0110
CLSYDTEILTVEYGPMPIGKIVEENINCSVYTVNKNGFVYTQSIAQWHHRGEQEVFEYYLEDGETIRATKDHKFMTTEGKMLPIDEIFENNLDLKKLTV

SEQ ID NO: 9 - protein, 99 aa, Cyanothece PCC8801
CLSYDTEILTVEYGAIPIGKVVEENIDCTVYTVDKNGFVYTQNIAQWHLRGQQEVFEYYLDDGSILRATKDHQFMTLEGEMLPIHEIFERGLELKKIKI

SEQ ID NO: 10 - protein, 106 aa, Crocosphaera watsonii
CLSYDTEILTVEYGAMYIGKIVEENINCTVYTVDKNGFVYTQTIAQWHNRGEQEIFEYDLEDGSKIKATKDHKFMTIDGEMLPIDEIFEKNLDLKQVVSHPDDYLV

SEQ ID NO: 11 - protein, 100 aa, Microcystis aeruginosa
CLGGETLILTEEYGLLPIAKIVSEEINCTVYTVDQNGFVYSQPISQWHERGLQEVFEYTLENGQTIQATKDHKFMTSDGEMLAIDTIFERGLDLKSSDFS

SEQ ID NO: 12 - protein, 104 aa, Microcoleus chthonoplastes
CLSYDTQILTVEYGAVAIGEIVEKQIECTVYSVDENGYVYTQPIAQWHNRGEQEVFEYLLEDGATIRATKDHKFMTDEDQMLPIDQIFEQGLELKQVEVLQPVF

SEQ ID NO: 13 - protein, 112 aa, Oscillatoria limnetica
CLSYNTEVLTVEYGPLPIGKIVDEQIHCRVYSVDENGFVYTQAIAQWHDRGYQEIFAYELADGSVIRATKDHQFMTEDGQMFPIDEIWEKGLDLKKLPTVQDLPAAVGYTVS

SEQ ID NO: 14 - protein, 113 aa, Synechococcus elongatus
CLAADTEVLTVEYGPIAIGKLVEENIRCQVYCCNPDGYIYSQPIGQWHQRGEQEVIEYELSDGRIIRATADHRFMTEEGEMLSLDEIFERSLELKQIPTPLLAIAQPSPLATA

SEQ ID NO: 15 - protein, 107 aa, Synechococcus PCC7002
CLAGGTPVVTVEYGVLPIQTIVEQELLCHVYSVDAQGLIYAQLIEQWHQRGDRLLYEYELENGQMIRATPDHRFLTTTGELLPIDEIFTQNLDLAAWAVPDSLPRTA

SEQ ID NO: 16 - protein, 117 aa, Thermosynechococcus elongatus
CLSGETAVMTVEYGAVPIRRLVQERLSCHVYSLDGQGHLYTQPIAQWHFQGFRPVYEYQLEDGSTICATPDHRFMTTRGQMLPIEQIFQEGLELWQVAIAPRQALLQGLKPAVQMSG

SEQ ID NO: 17 - protein, 101 aa, Trichodesmium erythraeum
CLTYETEIMTVEYGPLPIGKIVEYRIECTVYTVDKNGYIYTQPIAQWHNRGMQEVYEYSLEDGTVIRATPEHKFMTEDGQMLPIDEIFERNLDLKCLGTLE

SEQ ID NO: 18 - protein, 117 aa, Thermosynechococcus vulcanus
CLSGETAVMTVEYGAIPIRRLVQERLICQVYSLDPQGHLYTQPIAQWHFQGFRPVYAYQLEDGSTICATPDHRFMTTSGQMLPIEQIFREGLELWQVAIAPPGALAQGLKPAVQMSC

SEQ ID NO: 19 - protein, 102 aa, synthetic construct
  REGION 1..102: note = Peptide consensus sequence
CLSYDTEILTVEYGAVPIGKIVEENIECTVYSVDENGFVYTQPIAQWHDRGEQEVFEYCLEDGSTIRATKDHKFMTEDGEMLPIDEIFEQGLDLKQVKGLPD

SEQ ID NO: 20 - protein, 102 aa, synthetic construct
  REGION 1..102: note = Peptide consensus sequence
CLSYETEILTVEYGLLPIGKIVEKRIESTVYSVDNNGNIYTQPVAQWHDRGEQEVFEYSLEDGSLIRATKDHKFMTVDGQMLPIDEIFERELDLMRVDNLPN

SEQ ID NO: 21 - protein, 102 aa, Nostoc punctiforme
  SITE 28: note = X is A or S
  SITE 59: note = X is A or S
CLSYETEILTVEYGLLPIGKIVEKRIEXTVYSVDNNGNIYTQPVAQWHDRGEQEVFEYXLEDGSLIRATKDHKFMTVDGQMLPIDEIFERELDLMRVDNLPN

SEQ ID NO: 22 - protein, 123 aa, Synechocystis PCC6803
  SITE 28: note = X is A or S
CLSFGTEILTVEYGPLPIGKIVSEEINXSVYSVDPEGRVYTQAIAQWHDRGEQEVLEYELEDGSVIRATSDHRFLTTDYQLLAIEEIFARQLDLLTLENIKQTEEALDNHRLPFPLLDAGTIK

SEQ ID NO: 23 - protein, 110 aa, Aphanothece halophytica
  SITE 28: note = X is A or S
CLSYDTEIWTVEYGAMPIGKIVEEKIEXSVYTVDENGFVYTQPIAQWHPRGQQEIIEYTLEDGRKIRATKDHKMMTESGEMLPIEEIFQRELDLKVETFHEMSLLRRGAK

SEQ ID NO: 24 - protein, 101 aa, Aphanizomenon ovalisporum
  SITE 28: note = X is A or S
CLSADTEILTVEYGFLPIGEIVGKAIEXRVYSVDGNGNIYTQSIAQWHNRGEQEVFEYTLEDGSIIRATKDHKFMTTDGEMLPIDEIFARQLDLMQVQGLH

SEQ ID NO: 25 - protein, 102 aa, Anabaena PCC7120
  SITE 28: note = X is A or S
  SITE 59: note = X is A or S
CLSYDTEVLTVEYGFVPIGEIVEKGIEXSVFSINNNGIVYTQPIAQWHHRGKQEVFEYXLEDGSIIKATKDHKFMTQDGKMLPIDEIFEQELDLLQVKGLPE

SEQ ID NO: 26 - protein, 102 aa, Anabaena variabilis
  SITE 28: note = X is A or S
  SITE 59: note = X is A or S
CLSYDTEVLTVEYGFVPIGEIVDKGIEXSVFSIDSNGIVYTQPIAQWHHRGKQEVFEYXLEDGSIIKATKDHKFMTQDGKMLPIDEIFEQELDLLQVKGLPE

SEQ ID NO: 27 - protein, 118 aa, Cylindrospermopsis raciborskii
  SITE 28: note = X is A or S
  SITE 59: note = X is A or S
CLSYETEVLTLEYGFVPIGEIVNKQMVXTVFSLNDSGNVYTQPIGQWHDRGVQDLYEYXLDDGSTIRATKDHKFMTTQGEMVPIDEIFHQGWELVQVSGISKLVQQRTLPFIIVDRKL

SEQ ID NO: 28 - protein, 99 aa, Cyanothece CCY0110
  SITE 28: note = X is A or S
CLSYDTEILTVEYGPMPIGKIVEENINXSVYTVNKNGFVYTQSIAQWHHRGEQEVFEYYLEDGETIRATKDHKFMTTEGKMLPIDEIFENNLDLKKLTV

SEQ ID NO: 29 - protein, 99 aa, Cyanothece PCC8801
  SITE 28: note = X is A or S
CLSYDTEILTVEYGAIPIGKVVEENIDXTVYTVDKNGFVYTQNIAQWHLRGQQEVFEYYLDDGSILRATKDHQFMTLEGEMLPIHEIFERGLELKKIKI

SEQ ID NO: 30 - protein, 106 aa, Crocosphaera watsonii
  SITE 28: note = X is A or S
CLSYDTEILTVEYGAMYIGKIVEENINXTVYTVDKNGFVYTQTIAQWHNRGEQEIFEYDLEDGSKIKATKDHKFMTIDGEMLPIDEIFEKNLDLKQVVSHPDDYLV

SEQ ID NO: 31 - protein, 100 aa, Microcystis aeruginosa
  SITE 28: note = X is A or S
CLGGETLILTEEYGLLPIAKIVSEEINXTVYTVDQNGFVYSQPISQWHERGLQEVFEYTLENGQTIQATKDHKFMTSDGEMLAIDTIFERGLDLKSSDFS

SEQ ID NO: 32 - protein, 104 aa, Microcoleus chthonoplastes
  SITE 28: note = X is A or S
CLSYDTQILTVEYGAVAIGEIVEKQIEXTVYSVDENGYVYTQPIAQWHNRGEQEVFEYLLEDGATIRATKDHKFMTDEDQMLPIDQIFEQGLELKQVEVLQPVF

SEQ ID NO: 33 - protein, 112 aa, Oscillatoria limnetica
  SITE 28: note = X is A or S
CLSYNTEVLTVEYGPLPIGKIVDEQIHXRVYSVDENGFVYTQAIAQWHDRGYQEIFAYELADGSVIRATKDHQFMTEDGQMFPIDEIWEKGLDLKKLPTVQDLPAAVGYTVS

SEQ ID NO: 34 - protein, 113 aa, Synechococcus elongatus
  SITE 28: note = X is A or S
  SITE 32: note = X is A or S
  SITE 33: note = X is A or S
CLAADTEVLTVEYGPIAIGKLVEENIRXQVYXXNPDGYIYSQPIGQWHQRGEQEVIEYELSDGRIIRATADHRFMTEEGEMLSLDEIFERSLELKQIPTPLLAIAQPSPLATA

SEQ ID NO: 35 - protein, 107 aa, Synechococcus PCC7002
  SITE 28: note = X is A or S
CLAGGTPVVTVEYGVLPIQTIVEQELLXHVYSVDAQGLIYAQLIEQWHQRGDRLLYEYELENGQMIRATPDHRFLTTTGELLPIDEIFTQNLDLAAWAVPDSLPRTA

SEQ ID NO: 36 - protein, 117 aa, Thermosynechococcus elongatus
  SITE 28: note = X is A or S
  SITE 67: note = X is A or S
CLSGETAVMTVEYGAVPIRRLVQERLSXHVYSLDGQGHLYTQPIAQWHFQGFRPVYEYQLEDGSTIXATPDHRFMTTRGQMLPIEQIFQEGLELWQVAIAPRQALLQGLKPAVQMSG

SEQ ID NO: 37 - protein, 101 aa, Trichodesmium erythraeum
  SITE 28: note = X is A or S
  SITE 96: note = X is A or S
CLTYETEIMTVEYGPLPIGKIVEYRIEXTVYTVDKNGYIYTQPIAQWHNRGMQEVYEYSLEDGTVIRATPEHKFMTEDGQMLPIDEIFERNLDLKXLGTLE

SEQ ID NO: 38 - protein, 117 aa, Thermosynechococcus vulcanus
  SITE 28: note = X is A or S
  SITE 67: note = X is A or S
  SITE 117: note = X is A or S
CLSGETAVMTVEYGAIPIRRLVQERLIXQVYSLDPQGHLYTQPIAQWHFQGFRPVYAYQLEDGSTIXATPDHRFMTTSGQMLPIEQIFREGLELWQVAIAPPGALAQGLKPAVQMSX

SEQ ID NO: 39 - protein, 36 aa, Nostoc punctiforme
MIKIATRKYLGKQNVYDIGVERDHNFALKNGFIASN

SEQ ID NO: 40 - protein, 36 aa, Synechocystis PCC6803
MVKVIGRRSLGVQRIFDIGLPQDHNFLLANGAIAAN

SEQ ID NO: 41 - protein, 36 aa, Aphanothece halophytica
MVKIIKRQSLGRQNVYDVCVETDHNFVLANGCVASN

SEQ ID NO: 42 - protein, 36 aa, Aphanizomenon ovalisporum
MVKITARKFVGRENVYDIGVEHHHNFAIKNGLIASN

SEQ ID NO: 43 - protein, 36 aa, Anabaena PCC7120
MIKIASRKFLGVENVYDIGVRRDHNFFIKNGLIASN

SEQ ID NO: 44 - protein, 36 aa, Anabaena variabilis
MIKIASRKFLGVENVYDIGVGRDHNFFVKNGLIASN

SEQ ID NO: 45 - protein, 36 aa, Cylindrospermopsis raciborskii
MVKIVSRRYLGKADVYDIGVAKDHNFIIKNGLVASN

SEQ ID NO: 46 - protein, 36 aa, Cyanothece CCY0110
MVKIIERRSLGKQNVYDIGVEKDHNFLLSNNLIASN

SEQ ID NO: 47 - protein, 36 aa, Cyanothece PCC8801
MVKIVSYRSLGKQFVYDIGVAQDHNFLLANGSIASN

SEQ ID NO: 48 - protein, 36 aa, Crocosphaera watsonii
MVKIIGCRSLGTQKVYDIGVEKDHNFLLANGSIASN

SEQ ID NO: 49 - protein, 36 aa, Microcystis aeruginosa
MVKIIGRQSLGRKPVYDIGVEKDHNFLLGNGLIASN

SEQ ID NO: 50 - protein, 36 aa, Microcoleus chthonoplastes
MVKIVRRQSLGVQNVYDIGVEKDHNFCLASGEIASN

SEQ ID NO: 51 - protein, 36 aa, Oscillatoria limnetica; identical to SEQ ID NO: 50

SEQ ID NO: 52 - protein, 36 aa, Synechococcus elongatus
MVKIVRRRSLGVQPVYDLGVATVHNFVLANGLVASN

SEQ ID NO: 53 - protein, 36 aa, Synechococcus PCC7002
MVKIIRRKFIGHAPTYDIGLSQDHNFLLGQGLIAAN

SEQ ID NO: 54 - protein, 35 aa, Thermosynechococcus elongatus
MKIVGRRLMGWQAVYDIGLAADHNFVLANGAIAAN

SEQ ID NO: 55 - protein, 36 aa, Trichodesmium erythraeum
MVKIVSRKLAKTENVYDIGVTKDHNFVLANGLIASN

SEQ ID NO: 56 - protein, 35 aa, Thermosynechococcus vulcanus
MKIVGRRLVGWQAVYDIGLAGDHNFLLANGAIAAN

SEQ ID NO: 57 - protein, 36 aa, Nostoc punctiforme
  SITE 36: note = X is any amino acid excluding N and/or Q
MIKIATRKYLGKQNVYDIGVERDHNFALKNGFIASX

SEQ ID NO: 58 - protein, 36 aa, Synechocystis PCC6803
  SITE 36: note = X is any amino acid excluding N and/or Q
MVKVIGRRSLGVQRIFDIGLPQDHNFLLANGAIAAX

SEQ ID NO: 59 - protein, 36 aa, Aphanothece halophytica
  SITE 36: note = X is any amino acid excluding N and/or Q
MVKIIKRQSLGRQNVYDVCVETDHNFVLANGCVASX

SEQ ID NO: 60 - protein, 36 aa, Aphanizomenon ovalisporum
  SITE 36: note = X is any amino acid excluding N and/or Q
MVKITARKFVGRENVYDIGVEHHHNFAIKNGLIASX

SEQ ID NO: 61 - protein, 36 aa, Anabaena PCC7120
  SITE 36: note = X is any amino acid excluding N and/or Q
MIKIASRKFLGVENVYDIGVRRDHNFFIKNGLIASX

SEQ ID NO: 62 - protein, 36 aa, Anabaena variabilis
  SITE 36: note = X is any amino acid excluding N and/or Q
MIKIASRKFLGVENVYDIGVGRDHNFFVKNGLIASX

SEQ ID NO: 63 - protein, 36 aa, Cylindrospermopsis raciborskii
  SITE 36: note = X is any amino acid excluding N and/or Q
MVKIVSRRYLGKADVYDIGVAKDHNFIIKNGLVASX

SEQ ID NO: 64 - protein, 36 aa, Cyanothece CCY0110
  SITE 36: note = X is any amino acid excluding N and/or Q
MVKIIERRSLGKQNVYDIGVEKDHNFLLSNNLIASX

SEQ ID NO: 65 - protein, 36 aa, Cyanothece PCC8801
  SITE 36: note = X is any amino acid excluding N and/or Q
MVKIVSYRSLGKQFVYDIGVAQDHNFLLANGSIASX

SEQ ID NO: 66 - protein, 36 aa, Crocosphaera watsonii
  SITE 36: note = X is any amino acid excluding N and/or Q
MVKIIGCRSLGTQKVYDIGVEKDHNFLLANGSIASX

SEQ ID NO: 67 - protein, 36 aa, Microcystis aeruginosa
  SITE 36: note = X is any amino acid excluding N and/or Q
MVKIIGRQSLGRKPVYDIGVEKDHNFLLGNGLIASX

SEQ ID NO: 68 - protein, 36 aa, Microcoleus chthonoplastes
  SITE 36: note = X is any amino acid excluding N and/or Q
MVKIVRRQSLGVQNVYDIGVEKDHNFCLASGEIASX

SEQ ID NO: 69 - protein, 36 aa, Oscillatoria limnetica; identical to SEQ ID NO: 68
  SITE 36: note = X is any amino acid excluding N and/or Q

SEQ ID NO: 70 - protein, 36 aa, Synechococcus elongatus
  SITE 36: note = X is any amino acid excluding N and/or Q
MVKIVRRRSLGVQPVYDLGVATVHNFVLANGLVASX

SEQ ID NO: 71 - protein, 36 aa, Synechococcus PCC7002
  SITE 36: note = X is any amino acid excluding N and/or Q
MVKIIRRKFIGHAPTYDIGLSQDHNFLLGQGLIAAX

SEQ ID NO: 72 - protein, 35 aa, Thermosynechococcus elongatus
  SITE 35: note = X is any amino acid excluding N and/or Q
MKIVGRRLMGWQAVYDIGLAADHNFVLANGAIAAX

SEQ ID NO: 73 - protein, 36 aa, Trichodesmium erythraeum
  SITE 36: note = X is any amino acid excluding N and/or Q
MVKIVSRKLAKTENVYDIGVTKDHNFVLANGLIASX

SEQ ID NO: 74 - protein, 35 aa, Thermosynechococcus vulcanus
  SITE 35: note = X is any amino acid excluding N and/or Q
MKIVGRRLVGWQAVYDIGLAGDHNFLLANGAIAAX

SEQ ID NO: 75 - protein, 36 aa, Nostoc punctiforme; identical to SEQ ID NO: 57
  SITE 36: note = X is A, V, I, S, M, H, L, F, Y, G or W or can be a unnatural aliphatic amino acid residue such as Nle, Abu, Nva, 2-aminopentoic acid,or 2-aminohexaanoic acid

SEQ ID NO: 76 - protein, 36 aa, Synechocystis PCC6803; identical to SEQ ID NO: 58
  SITE 36: note = X is A, V, I, S, M, H, L, F, Y, G or W or can be a unnatural aliphatic amino acid residue such as Nle, Abu, Nva, 2-aminopentoic acid,or 2-aminohexaanoic acid

SEQ ID NO: 77 - protein, 36 aa, Aphanothece halophytica; identical to SEQ ID NO: 59
  SITE 36: note = X is A, V, I, S, M, H, L, F, Y, G or W or can be a unnatural aliphatic amino acid residue such as Nle, Abu, Nva, 2-aminopentoic acid,or 2-aminohexaanoic acid

SEQ ID NO: 78 - protein, 36 aa, Aphanizomenon ovalisporum; identical to SEQ ID NO: 60
  SITE 36: note = X is A, V, I, S, M, H, L, F, Y, G or W or can be a unnatural aliphatic amino acid residue such as Nle, Abu, Nva, 2-aminopentoic acid,or 2-aminohexaanoic acid

SEQ ID NO: 79 - protein, 36 aa, Anabaena PCC7120; identical to SEQ ID NO: 61
  SITE 36: note = X is A, V, I, S, M, H, L, F, Y, G or W or can be a unnatural aliphatic amino acid residue such as Nle, Abu, Nva, 2-aminopentoic acid,or 2-aminohexaanoic acid

SEQ ID NO: 80 - protein, 36 aa, Anabaena variabilis; identical to SEQ ID NO: 62
  SITE 36: note = X is A, V, I, S, M, H, L, F, Y, G or W or can be a unnatural aliphatic amino acid residue such as Nle, Abu, Nva, 2-aminopentoic acid,or 2-aminohexaanoic acid

SEQ ID NO: 81 - protein, 36 aa, Cylindrospermopsis raciborskii; identical to SEQ ID NO: 63
  SITE 36: note = X is A, V, I, S, M, H, L, F, Y, G or W or can be a unnatural aliphatic amino acid residue such as Nle, Abu, Nva, 2-aminopentoic acid,or 2-aminohexaanoic acid

SEQ ID NO: 82 - protein, 36 aa, Cyanothece CCY0110; identical to SEQ ID NO: 64
  SITE 36: note = X is A, V, I, S, M, H, L, F, Y, G or W or can be a unnatural aliphatic amino acid residue such as Nle, Abu, Nva, 2-aminopentoic acid,or 2-aminohexaanoic acid

SEQ ID NO: 83 - protein, 36 aa, Cyanothece PCC8801; identical to SEQ ID NO: 65
  SITE 36: note = X is A, V, I, S, M, H, L, F, Y, G or W or can be a unnatural aliphatic amino acid residue such as Nle, Abu, Nva, 2-aminopentoic acid,or 2-aminohexaanoic acid

SEQ ID NO: 84 - protein, 36 aa, Crocosphaera watsonii; identical to SEQ ID NO: 66
  SITE 36: note = X is A, V, I, S, M, H, L, F, Y, G or W or can be a unnatural aliphatic amino acid residue such as Nle, Abu, Nva, 2-aminopentoic acid,or 2-aminohexaanoic acid

SEQ ID NO: 85 - protein, 36 aa, Microcystis aeruginosa; identical to SEQ ID NO: 67
  SITE 36: note = X is A, V, I, S, M, H, L, F, Y, G or W or can be a unnatural aliphatic amino acid residue such as Nle, Abu, Nva, 2-aminopentoic acid,or 2-aminohexaanoic acid

SEQ ID NO: 86 - protein, 36 aa, Microcoleus chthonoplastes; identical to SEQ ID NO: 68
  SITE 36: note = X is A, V, I, S, M, H, L, F, Y, G or W or can be a unnatural aliphatic amino acid residue such as Nle, Abu, Nva, 2-aminopentoic acid,or 2-aminohexaanoic acid

SEQ ID NO: 87 - protein, 36 aa, Oscillatoria limnetica; identical to SEQ ID NO: 68
  SITE 36: note = X is A, V, I, S, M, H, L, F, Y, G or W or can be a unnatural aliphatic amino acid residue such as Nle, Abu, Nva, 2-aminopentoic acid,or 2-aminohexaanoic acid

SEQ ID NO: 88 - protein, 36 aa, Synechococcus elongatus; identical to SEQ ID NO: 70
  SITE 36: note = X is A, V, I, S, M, H, L, F, Y, G or W or can be a unnatural aliphatic amino acid residue such as Nle, Abu, Nva, 2-aminopentoic acid,or 2-aminohexaanoic acid

SEQ ID NO: 89 - protein, 36 aa, Synechococcus PCC7002; identical to SEQ ID NO: 71
  SITE 36: note = X is A, V, I, S, M, H, L, F, Y, G or W or can be a unnatural aliphatic amino acid residue such as Nle, Abu, Nva, 2-aminopentoic acid,or 2-aminohexaanoic acid

SEQ ID NO: 90 - protein, 35 aa, Thermosynechococcus elongatus; identical to SEQ ID NO: 72
  SITE 35: note = X is A, V, I, S, M, H, L, F, Y, G or W or can be a unnatural aliphatic amino acid residue such as Nle, Abu, Nva, 2-aminopentoic acid,or 2-aminohexaanoic acid

SEQ ID NO: 91 - protein, 36 aa, Trichodesmium erythraeum; identical to SEQ ID NO: 73
  SITE 36: note = X is A, V, I, S, M, H, L, F, Y, G or W or can be a unnatural aliphatic amino acid residue such as Nle, Abu, Nva, 2-aminopentoic acid,or 2-aminohexaanoic acid

SEQ ID NO: 92 - protein, 35 aa, Thermosynechococcus vulcanus; identical to SEQ ID NO: 74
  SITE 35: note = X is A, V, I, S, M, H, L, F, Y, G or W or can be a unnatural aliphatic amino acid residue such as Nle, Abu, Nva, 2-aminopentoic acid,or 2-aminohexaanoic acid

SEQ ID NO: 93 - protein, 36 aa, Nostoc punctiforme; identical to SEQ ID NO: 57
  SITE 36: note = X is A, I, V, L, Y, G or F

SEQ ID NO: 94 - protein, 36 aa, Synechocystis PCC6803; identical to SEQ ID NO: 58
  SITE 36: note = X is A, I, V, L, Y, G or F

SEQ ID NO: 95 - protein, 36 aa, Aphanothece halophytica; identical to SEQ ID NO: 59
  SITE 36: note = X is A, I, V, L, Y, G or F

SEQ ID NO: 96 - protein, 36 aa, Aphanizomenon ovalisporum; identical to SEQ ID NO: 60
  SITE 36: note = X is A, I, V, L, Y, G or F

SEQ ID NO: 97 - protein, 36 aa, Anabaena PCC7120; identical to SEQ ID NO: 61
  SITE 36: note = MISC_FEATURE - Xaa is Ala, Ile, Val, Leu, Tyr, Gly or Phe

SEQ ID NO: 98 - protein, 36 aa, Anabaena variabilis; identical to SEQ ID NO: 62
  SITE 36: note = X is A, I, V, L, Y, G or F

SEQ ID NO: 99 - protein, 36 aa, Cylindrospermopsis raciborskii; identical to SEQ ID NO: 63
  SITE 36: note = X is A, I, V, L, Y, G or F

SEQ ID NO: 100 - protein, 36 aa, Cyanothece CCY0110; identical to SEQ ID NO: 64
  SITE 36: note = X is A, I, V, L, Y, G or F

SEQ ID NO: 101 - protein, 36 aa, Cyanothece PCC8801; identical to SEQ ID NO: 65
  SITE 36: note = X is A, I, V, L, Y, G or F

SEQ ID NO: 102 - protein, 36 aa, Crocosphaera watsonii; identical to SEQ ID NO: 66
  SITE 36: note = X is A, I, V, L, Y, G or F

SEQ ID NO: 103 - protein, 36 aa, Microcystis aeruginosa; identical to SEQ ID NO: 67
  SITE 36: note = X is A, I, V, L, Y, G or F

SEQ ID NO: 104 - protein, 36 aa, Microcoleus chthonoplastes; identical to SEQ ID NO: 68
  SITE 36: note = X is A, I, V, L, Y, G or F

SEQ ID NO: 105 - protein, 36 aa, Oscillatoria limnetica; identical to SEQ ID NO: 68
  SITE 36: note = X is A, I, V, L, Y, G or F

SEQ ID NO: 106 - protein, 36 aa, Synechococcus elongatus; identical to SEQ ID NO: 70
  SITE 36: note = X is A, I, V, L, Y, G or F

SEQ ID NO: 107 - protein, 36 aa, Synechococcus PCC7002; identical to SEQ ID NO: 71
  SITE 36: note = X is A, I, V, L, Y, G or F

SEQ ID NO: 108 - protein, 35 aa, Thermosynechococcus elongatus; identical to SEQ ID NO: 72
  SITE 35: note = X is A, I, V, L, Y, G or F

SEQ ID NO: 109 - protein, 36 aa, Trichodesmium erythraeum; identical to SEQ ID NO: 73
  SITE 36: note = X is A, I, V, L, Y, G or F

SEQ ID NO: 110 - protein, 35 aa, Thermosynechococcus vulcanus; identical to SEQ ID NO: 74
  SITE 35: note = X is A, I, V, L, Y, G or F

SEQ ID NO: 111 - protein, 36 aa, Nostoc punctiforme
MIKIATRKYLGKQNVYDIGVERDHNFALKNGFIASA

SEQ ID NO: 112 - protein, 36 aa, Synechocystis PCC6803
MVKVIGRRSLGVQRIFDIGLPQDHNFLLANGAIAAA

SEQ ID NO: 113 - protein, 36 aa, Aphanothece halophytica
MVKIIKRQSLGRQNVYDVCVETDHNFVLANGCVASA

SEQ ID NO: 114 - protein, 36 aa, Aphanizomenon ovalisporum
MVKITARKFVGRENVYDIGVEHHHNFAIKNGLIASA

SEQ ID NO: 115 - protein, 36 aa, Anabaena PCC7120
MIKIASRKFLGVENVYDIGVRRDHNFFIKNGLIASA

SEQ ID NO: 116 - protein, 36 aa, Anabaena variabilis
MIKIASRKFLGVENVYDIGVGRDHNFFVKNGLIASA

SEQ ID NO: 117 - protein, 36 aa, Cylindrospermopsis raciborskii
MVKIVSRRYLGKADVYDIGVAKDHNFIIKNGLVASA

SEQ ID NO: 118 - protein, 36 aa, Cyanothece CCY0110
MVKIIERRSLGKQNVYDIGVEKDHNFLLSNNLIASA

SEQ ID NO: 119 - protein, 36 aa, Cyanothece PCC8801
MVKIVSYRSLGKQFVYDIGVAQDHNFLLANGSIASA

SEQ ID NO: 120 - protein, 36 aa, Crocosphaera watsonii
MVKIIGCRSLGTQKVYDIGVEKDHNFLLANGSIASA

SEQ ID NO: 121 - protein, 36 aa, Microcystis aeruginosa
MVKIIGRQSLGRKPVYDIGVEKDHNFLLGNGLIASA

SEQ ID NO: 122 - protein, 36 aa, Microcoleus chthonoplastes
MVKIVRRQSLGVQNVYDIGVEKDHNFCLASGEIASA

SEQ ID NO: 123 - protein, 36 aa, Oscillatoria limnetica; identical to SEQ ID NO: 122

SEQ ID NO: 124 - protein, 36 aa, Synechococcus elongatus
MVKIVRRRSLGVQPVYDLGVATVHNFVLANGLVASA

SEQ ID NO: 125 - protein, 36 aa, Synechococcus PCC7002
MVKIIRRKFIGHAPTYDIGLSQDHNFLLGQGLIAAA

SEQ ID NO: 126 - protein, 35 aa, Thermosynechococcus elongatus
MKIVGRRLMGWQAVYDIGLAADHNFVLANGAIAAA

SEQ ID NO: 127 - protein, 36 aa, Trichodesmium erythraeum
MVKIVSRKLAKTENVYDIGVTKDHNFVLANGLIASA

SEQ ID NO: 128 - protein, 35 aa, Thermosynechococcus vulcanus
MKIVGRRLVGWQAVYDIGLAGDHNFLLANGAIAAA

SEQ ID NO: 129 - protein, 39 aa, Nostoc punctiforme
  SITE 36: note = X is any amino acid excluding N and/or Q
  SITE 37: note = X is any amino acid excluding C
MIKIATRKYLGKQNVYDIGVERDHNFALKNGFIASXXFN

SEQ ID NO: 130 - protein, 39 aa, Synechocystis PCC6803
  SITE 36: note = X is any amino acid excluding N and/or Q
  SITE 37: note = X is any amino acid excluding C
MVKVIGRRSLGVQRIFDIGLPQDHNFLLANGAIAAXXFN

SEQ ID NO: 131 - protein, 39 aa, Aphanothece halophytica
  SITE 36: note = X is any amino acid excluding N and/or Q
  SITE 37: note = X is any amino acid excluding C
MVKIIKRQSLGRQNVYDVCVETDHNFVLANGCVASXXFN

SEQ ID NO: 132 - protein, 39 aa, Aphanizomenon ovalisporum
  SITE 36: note = Xis any amino acid excluding N and/or Q
  SITE 37: note = X is any amino acid excluding C
MVKITARKFVGRENVYDIGVEHHHNFAIKNGLIASXXFN

SEQ ID NO: 133 - protein, 39 aa, Anabaena PCC7120
  SITE 36: note = X is any amino acid excluding N and/or Q
  SITE 37: note = X is any amino acid excluding C
MIKIASRKFLGVENVYDIGVRRDHNFFIKNGLIASXXFN

SEQ ID NO: 134 - protein, 39 aa, Anabaena variabilis
  SITE 36: note = X is any amino acid excluding N and/or Q
  SITE 37: note = X is any amino acid excluding C
MIKIASRKFLGVENVYDIGVGRDHNFFVKNGLIASXXFN

SEQ ID NO: 135 - protein, 39 aa, Cylindrospermopsis raciborskii
  SITE 36: note = X is any amino acid excluding N and/or Q
  SITE 37: note = X is any amino acid excluding C
MVKIVSRRYLGKADVYDIGVAKDHNFIIKNGLVASXXFN

SEQ ID NO: 136 - protein, 39 aa, Cyanothece CCY0110
  SITE 36: note = X is any amino acid excluding N and/or Q
  SITE 37: note = X is any amino acid excluding C
MVKIIERRSLGKQNVYDIGVEKDHNFLLSNNLIASXXFN

SEQ ID NO: 137 - protein, 39 aa, Cyanothece PCC8801
  SITE 36: note = X is any amino acid excluding N and/or Q
  SITE 37: note = X is any amino acid excluding C
MVKIVSYRSLGKQFVYDIGVAQDHNFLLANGSIASXXFN

SEQ ID NO: 138 - protein, 39 aa, Crocosphaera watsonii
  SITE 36: note = X is any amino acid excluding N and/or Q
  SITE 37: note = X is any amino acid excluding C
MVKIIGCRSLGTQKVYDIGVEKDHNFLLANGSIASXXFN

SEQ ID NO: 139 - protein, 39 aa, Microcystis aeruginosa
  SITE 36: note = X is any amino acid excluding N and/or Q
  SITE 37: note = X is any amino acid excluding C
MVKIIGRQSLGRKPVYDIGVEKDHNFLLGNGLIASXXFN

SEQ ID NO: 140 - protein, 39 aa, Microcoleus chthonoplastes
  SITE 36: note = X is any amino acid excluding N and/or Q
  SITE 37: note = X is any amino acid excluding C
MVKIVRRQSLGVQNVYDIGVEKDHNFCLASGEIASXXFN

SEQ ID NO: 141 - protein, 39 aa, Oscillatoria limnetica; identical to SEQ ID NO: 140
  SITE 36: note = X is any amino acid excluding N and/or Q
  SITE 37: note = X is any amino acid excluding C

SEQ ID NO: 142 - protein, 39 aa, Synechococcus elongatus
  SITE 36: note = X is any amino acid excluding N and/or Q
  SITE 37: note = X is any amino acid excluding C
MVKIVRRRSLGVQPVYDLGVATVHNFVLANGLVASXXFN

SEQ ID NO: 143 - protein, 39 aa, Synechococcus PCC7002
  SITE 36: note = X is any amino acid excluding N and/or Q
  SITE 37: note = X is any amino acid excluding C
MVKIIRRKFIGHAPTYDIGLSQDHNFLLGQGLIAAXXFN

SEQ ID NO: 144 - protein, 38 aa, Thermosynechococcus elongatus
  SITE 35: note = X is any amino acid excluding N and/or Q
  SITE 36: note = X is any amino acid excluding C
MKIVGRRLMGWQAVYDIGLAADHNFVLANGAIAAXXFN

SEQ ID NO: 145 - protein, 39 aa, Trichodesmium erythraeum
  SITE 36: note = X is any amino acid excluding N and/or Q
  SITE 37: note = X is any amino acid excluding N
MVKIVSRKLAKTENVYDIGVTKDHNFVLANGLIASXXFN

SEQ ID NO: 146 - protein, 38 aa, Thermosynechococcus vulcanus
  SITE 35: note = Xa is any amino acid excluding N and/or Q
  SITE 36: note = X is any amino acid excluding C
MKIVGRRLVGWQAVYDIGLAGDHNFLLANGAIAAXXFN

SEQ ID NO: 147 - protein, 39 aa, Nostoc punctiforme; identical to SEQ ID NO: 129
  SITE 36: note = X is any amino acid excluding N and/or Q
  SITE 37: note = X is A, V, I, S, M, H, L, F, Y, G or W or can be a unnatural aliphatic amino acid residue such as Nle, Abu, Nva, 2-aminopentoic acid, or 2-aminohexaanoic acid

SEQ ID NO: 148 - protein, 39 aa, Synechocystis PCC6803; identical to SEQ ID NO: 130
  SITE 36: note = X is any amino acid excluding N and/or Q
  SITE 37: note = X is A, V, I, S, M, H, L, F, Y, G or W or can be a unnatural aliphatic amino acid residue such as Nle, Abu, Nva, 2-aminopentoic acid, or 2-aminohexaanoic acid

SEQ ID NO: 149 - protein, 39 aa, Aphanothece halophytica; identical to SEQ ID NO: 131
  SITE 36: note = X is any amino acid excluding N and/or Q
  SITE 37: note = X is A, V, I, S, M, H, L, F, Y, G or W or can be a unnatural aliphatic amino acid residue such as Nle, Abu, Nva, 2-aminopentoic acid, or 2-aminohexaanoic acid

SEQ ID NO: 150 - protein, 39 aa, Aphanizomenon ovalisporum; identical to SEQ ID NO: 132
  SITE 36: note = X is any amino acid excluding N and/or Q
  SITE 37: note = X is A, V, I, S, M, H, L, F, Y, G or W or can be a unnatural aliphatic amino acid residue such as Nle, Abu, Nva, 2-aminopentoic acid, or 2-aminohexaanoic acid

SEQ ID NO: 151 - protein, 39 aa, Anabaena PCC7120; identical to SEQ ID NO: 133
  SITE 36: note = X is any amino acid excluding N and/or Q
  SITE 37: note = X is A, V, I, S, M, H, L, F, Y, G or W or can be a unnatural aliphatic amino acid residue such as Nle, Abu, Nva, 2-aminopentoic acid, or 2-aminohexaanoic acid

SEQ ID NO: 152 - protein, 39 aa, Anabaena variabilis; identical to SEQ ID NO: 134
  SITE 36: note = X is any amino acid excluding N and/or Q
  SITE 37: note = X is A, V, I, S, M, H, L, F, Y, G or W or can be a unnatural aliphatic amino acid residue such as Nle, Abu, Nva, 2-aminopentoic acid, or 2-aminohexaanoic acid

SEQ ID NO: 153 - protein, 39 aa, Cylindrospermopsis raciborskii; identical to SEQ ID NO: 135
  SITE 36: note = X is any amino acid excluding N and/or Q
  SITE 37: note = X is A, V, I, S, M, H, L, F, Y, G or W or can be a unnatural aliphatic amino acid residue such as Nle, Abu, Nva, 2-aminopentoic acid, or 2-aminohexaanoic acid

SEQ ID NO: 154 - protein, 39 aa, Cyanothece CCY0110; identical to SEQ ID NO: 136
  SITE 36: note = X is any amino acid excluding N and/or Q
  SITE 37: note = X is A, V, I, S, M, H, L, F, Y, G or W or can be a unnatural aliphatic amino acid residue such as Nle, Abu, Nva, 2-aminopentoic acid, or 2-aminohexaanoic acid

SEQ ID NO: 155 - protein, 39 aa, Cyanothece PCC8801; identical to SEQ ID NO: 137
  SITE 36: note = X is any amino acid excluding N and/or Q
  SITE 37: note = X is A, V, I, S, M, H, L, F, Y, G or W or can be a unnatural aliphatic amino acid residue such as Nle, Abu, Nva, 2-aminopentoic acid, or 2-aminohexaanoic acid

SEQ ID NO: 156 - protein, 39 aa, Crocosphaera watsonii; identical to SEQ ID NO: 138
  SITE 36: note = X is any amino acid excluding N and/or Q
  SITE 37: note = X is A, V, I, S, M, H, L, F, Y, G or W or can be a unnatural aliphatic amino acid residue such as Nle, Abu, Nva, 2-aminopentoic acid, or 2-aminohexaanoic acid

SEQ ID NO: 157 - protein, 39 aa, Microcystis aeruginosa; identical to SEQ ID NO: 139
  SITE 36: note = X is any amino acid excluding N and/or Q
  SITE 37: note = X is A, V, I, S, M, H, L, F, Y, G or W or can be a unnatural aliphatic amino acid residue such as Nle, Abu, Nva, 2-aminopentoic acid, or 2-aminohexaanoic acid

SEQ ID NO: 158 - protein, 39 aa, Microcoleus chthonoplastes; identical to SEQ ID NO: 140
  SITE 36: note = X is any amino acid excluding N and/or Q
  SITE 37: note = X is A, V, I, S, M, H, L, F, Y, G or W or can be a unnatural aliphatic amino acid residue such as Nle, Abu, Nva, 2-aminopentoic acid, or 2-aminohexaanoic acid

SEQ ID NO: 159 - protein, 39 aa, Oscillatoria limnetica; identical to SEQ ID NO: 140
  SITE 36: note = X is any amino acid excluding N and/or Q
  SITE 37: note = X is A, V, I, S, M, H, L, F, Y, G or W or can be a unnatural aliphatic amino acid residue such as Nle, Abu, Nva, 2-aminopentoic acid, or 2-aminohexaanoic acid

SEQ ID NO: 160 - protein, 39 aa, Synechococcus elongatus; identical to SEQ ID NO: 142
  SITE 36: note = X is any amino acid excluding N and/or Q
  SITE 37: note = X is A, V, I, S, M, H, L, F, Y, G or W or can be a unnatural aliphatic amino acid residue such as Nle, Abu, Nva, 2-aminopentoic acid, or 2-aminohexaanoic acid

SEQ ID NO: 161 - protein, 39 aa, Synechococcus PCC7002; identical to SEQ ID NO: 143
  SITE 36: note = X is any amino acid excluding N and/or Q
  SITE 37: note = X is A, V, I, S, M, H, L, F, Y, G or W or can be a unnatural aliphatic amino acid residue such as Nle, Abu, Nva, 2-aminopentoic acid, or 2-aminohexaanoic acid

SEQ ID NO: 162 - protein, 38 aa, Thermosynechococcus elongatus; identical to SEQ ID NO: 144
  SITE 35: note = X is any amino acid excluding N and/or Q
  SITE 36: note = X is A, V, I, S, M, H, L, F, Y, G or W or can be a unnatural aliphatic amino acid residue such as Nle, Abu, Nva, 2-aminopentoic acid, or 2-aminohexaanoic acid

SEQ ID NO: 163 - protein, 39 aa, Trichodesmium erythraeum; identical to SEQ ID NO: 145
  SITE 36: note = X is any amino acid excluding N and/or Q
  SITE 37: note = X is A, V, I, S, M, H, L, F, Y, G or W or can be a unnatural aliphatic amino acid residue such as Nle, Abu, Nva, 2-aminopentoic acid, or 2-aminohexaanoic acid

SEQ ID NO: 164 - protein, 38 aa, Thermosynechococcus vulcanus; identical to SEQ ID NO: 146
  SITE 35: note = X is any amino acid excluding N and/or Q
  SITE 36: note = X is A, V, I, S, M, H, L, F, Y, G or W or can be a unnatural aliphatic amino acid residue such as Nle, Abu, Nva, 2-aminopentoic acid, or 2-aminohexaanoic acid

SEQ ID NO: 165 - protein, 39 aa, Nostoc punctiforme; identical to SEQ ID NO: 129
  SITE 36: note = X is any amino acid excluding N and/or Q
  SITE 37: note = X is A, I, V, L, Y, G or F

SEQ ID NO: 166 - protein, 39 aa, Synechocystis PCC6803; identical to SEQ ID NO: 130
  SITE 36: note = X is any amino acid excluding N and/or Q
  SITE 37: note = X is A, I, V, L, Y, G or F

SEQ ID NO: 167 - protein, 39 aa, Aphanothece halophytica; identical to SEQ ID NO: 131
  SITE 36: note = X is any amino acid excluding N and/or Q
  SITE 37: note = X is A, I, V, L, Y, G or F

SEQ ID NO: 168 - protein, 39 aa, Aphanizomenon ovalisporum; identical to SEQ ID NO: 132
  SITE 36: note = X is any amino acid excluding N and/or Q
  SITE 37: note = X is A, I, V, L, Y, G or F

SEQ ID NO: 169 - protein, 39 aa, Anabaena PCC7120; identical to SEQ ID NO: 133
  SITE 36: note = X is any amino acid excluding N and/or Q
  SITE 37: note = X is A, I, V, L, Y, G or F

SEQ ID NO: 170 - protein, 39 aa, Anabaena variabilis; identical to SEQ ID NO: 134
  SITE 36: note = X is any amino acid excluding N and/or Q
  SITE 37: note = X is A, I, V, L, Y, G or F

SEQ ID NO: 171 - protein, 39 aa, Cylindrospermopsis raciborskii; identical to SEQ ID NO: 135
  SITE 36: note = X is any amino acid excluding N and/or Q
  SITE 37: note = X is A, I, V, L, Y, G or F

SEQ ID NO: 172 - protein, 39 aa, Cyanothece CCY0110; identical to SEQ ID NO: 136
  SITE 36: note = X is any amino acid excluding N and/or Q
  SITE 37: note = X is A, I, V, L, Y, G or F

SEQ ID NO: 173 - protein, 39 aa, Cyanothece PCC8801; identical to SEQ ID NO: 137
  SITE 36: note = X is any amino acid excluding N and/or Q
  SITE 37: note = X is A, I, V, L, Y, G or F

SEQ ID NO: 174 - protein, 39 aa, Crocosphaera watsonii; identical to SEQ ID NO: 138
  SITE 36: note = X is any amino acid excluding N and/or Q
  SITE 37: note = X is A, I, V, L, Y, G or F

SEQ ID NO: 175 - protein, 39 aa, Microcystis aeruginosa; identical to SEQ ID NO: 139
  SITE 36: note = X is any amino acid excluding N and/or Q
  SITE 37: note = X is A, I, V, L, Y, G or F

SEQ ID NO: 176 - protein, 39 aa, Microcoleus chthonoplastes; identical to SEQ ID NO: 140
  SITE 36: note = X is any amino acid excluding N and/or Q
  SITE 37: note = X is A, I, V, L, Y, G or F

SEQ ID NO: 177 - protein, 39 aa, Oscillatoria limnetica; identical to SEQ ID NO: 140
  SITE 36: note = X is any amino acid excluding N and/or Q
  SITE 37: note = X is A, I, V, L, Y, G or F

SEQ ID NO: 178 - protein, 39 aa, Synechococcus elongatus; identical to SEQ ID NO: 142
  SITE 36: note = X is any amino acid excluding N and/or Q
  SITE 37: note = X is A, I, V, L, Y, G or F

SEQ ID NO: 179 - protein, 39 aa, Synechococcus PCC7002; identical to SEQ ID NO: 143
  SITE 36: note = X is any amino acid excluding N and/or Q
  SITE 37: note = X is A, I, V, L, Y, G or F

SEQ ID NO: 180 - protein, 38 aa, Thermosynechococcus elongatus; identical to SEQ ID NO: 144
  SITE 35: note = X is any amino acid excluding N and/or Q
  SITE 36: note = X is A, I, V, L, Y, G or F

SEQ ID NO: 181 - protein, 39 aa, Trichodesmium erythraeum; identical to SEQ ID NO: 145
  SITE 36: note = X is any amino acid excluding N and/or Q
  SITE 37: note = X is A, I, V, L, Y, G or F

SEQ ID NO: 182 - protein, 38 aa, Thermosynechococcus vulcanus; identical to SEQ ID NO: 146
  SITE 35: note = X is any amino acid excluding N and/or Q
  SITE 36: note = X is A, I, V, L, Y, G or F

SEQ ID NO: 183 - protein, 39 aa, Nostoc punctiforme
  SITE 36: note = X is any amino acid excluding N and/or Q
MIKIATRKYLGKQNVYDIGVERDHNFALKNGFIASXAFN

SEQ ID NO: 184 - protein, 39 aa, Synechocystis PCC6803
  SITE 36: note = X is any amino acid excluding N and/or Q
MVKVIGRRSLGVQRIFDIGLPQDHNFLLANGAIAAXAFN

SEQ ID NO: 185 - protein, 39 aa, Aphanothece halophytica
  SITE 36: note = X is any amino acid excluding N and/or Q
MVKIIKRQSLGRQNVYDVCVETDHNFVLANGCVASXAFN

SEQ ID NO: 186 - protein, 39 aa, Aphanizomenon ovalisporum
  SITE 36: note = X is any amino acid excluding N and/or Q
MVKITARKFVGRENVYDIGVEHHHNFAIKNGLIASXAFN

SEQ ID NO: 187 - protein, 39 aa, Anabaena PCC7120
  SITE 36: note = X is any amino acid excluding N and/or Q
MIKIASRKFLGVENVYDIGVRRDHNFFIKNGLIASXAFN

SEQ ID NO: 188 - protein, 39 aa, Anabaena variabilis
  SITE 36: note = X is any amino acid excluding N and/or Q
MIKIASRKFLGVENVYDIGVGRDHNFFVKNGLIASXAFN

SEQ ID NO: 189 - protein, 39 aa, Cylindrospermopsis raciborskii
  SITE 36: note = X is any amino acid excluding N and/or Q
MVKIVSRRYLGKADVYDIGVAKDHNFIIKNGLVASXAFN

SEQ ID NO: 190 - protein, 39 aa, Cyanothece CCY0110
  SITE 36: note = X is any amino acid excluding N and/or Q
MVKIIERRSLGKQNVYDIGVEKDHNFLLSNNLIASXAFN

SEQ ID NO: 191 - protein, 39 aa, Cyanothece PCC8801
  SITE 36: note = X is any amino acid excluding N and/or Q
MVKIVSYRSLGKQFVYDIGVAQDHNFLLANGSIASXAFN

SEQ ID NO: 192 - protein, 39 aa, Crocosphaera watsonii
  SITE 36: note = X is any amino acid excluding N and/or Q
MVKIIGCRSLGTQKVYDIGVEKDHNFLLANGSIASXAFN

SEQ ID NO: 193 - protein, 39 aa, Microcystis aeruginosa
  SITE 36: note = X is any amino acid excluding N and/or Q
MVKIIGRQSLGRKPVYDIGVEKDHNFLLGNGLIASXAFN

SEQ ID NO: 194 - protein, 39 aa, Microcoleus chthonoplastes
  SITE 36: note = X is any amino acid excluding N and/or Q
MVKIVRRQSLGVQNVYDIGVEKDHNFCLASGEIASXAFN

SEQ ID NO: 195 - protein, 39 aa, Oscillatoria limnetica; identical to SEQ ID NO: 194
  SITE 36: note = X is any amino acid excluding N and/or Q

SEQ ID NO: 196 - protein, 39 aa, Synechococcus elongatus
  SITE 36: note = X is any amino acid excluding N and/or Q
MVKIVRRRSLGVQPVYDLGVATVHNFVLANGLVASXAFN

SEQ ID NO: 197 - protein, 39 aa, Synechococcus PCC7002
  SITE 36: note = X is any amino acid excluding N and/or Q
MVKIIRRKFIGHAPTYDIGLSQDHNFLLGQGLIAAXAFN

SEQ ID NO: 198 - protein, 38 aa, Thermosynechococcus elongatus
  SITE 35: note = X is any amino acid excluding N and/or Q
MKIVGRRLMGWQAVYDIGLAADHNFVLANGAIAAXAFN

SEQ ID NO: 199 - protein, 39 aa, Trichodesmium erythraeum
  SITE 36: note = X is any amino acid excluding N and/or Q
MVKIVSRKLAKTENVYDIGVTKDHNFVLANGLIASXAFN

SEQ ID NO: 200 - protein, 38 aa, Thermosynechococcus vulcanus
  SITE 35: note = X is any amino acid excluding N and/or Q
MKIVGRRLVGWQAVYDIGLAGDHNFLLANGAIAAXAFN

SEQ ID NO: 201 - protein, 39 aa, Nostoc punctiforme; identical to SEQ ID NO: 129
  SITE 36: note = X is A, V, I, S, M, H, L, F, Y, G or W or can be a unnatural aliphatic amino acid residue such as Nle, Abu, Nva, 2-aminopentoic acid,or 2-aminohexaanoic acid
  SITE 37: note = X is any amino acid excluding C

SEQ ID NO: 202 - protein, 39 aa, Synechocystis PCC6803; identical to SEQ ID NO: 130
  SITE 36: note = X is A, V, I, S, M, H, L, F, Y, G or W or can be a unnatural aliphatic amino acid residue such as Nle, Abu, Nva, 2-aminopentoic acid,or 2-aminohexaanoic acid
  SITE 37: note = X is any amino acid excluding C

SEQ ID NO: 203 - protein, 39 aa, Aphanothece halophytica; identical to SEQ ID NO: 131
  SITE 36: note = X is A, V, I, S, M, H, L, F, Y, G or W or can be a unnatural aliphatic amino acid residue such as Nle, Abu, Nva, 2-aminopentoic acid,or 2-aminohexaanoic acid
  SITE 37: note = X is any amino acid excluding C

SEQ ID NO: 204 - protein, 39 aa, Aphanizomenon ovalisporum; identical to SEQ ID NO: 132
  SITE 36: note = X is A, V, I, S, M, H, L, F, Y, G or W or can be a unnatural aliphatic amino acid residue such as Nle, Abu, Nva, 2-aminopentoic acid,or 2-aminohexaanoic acid
  SITE 37: note = X is any amino acid excluding C

SEQ ID NO: 205 - protein, 39 aa, Anabaena PCC7120; identical to SEQ ID NO: 133
  SITE 36: note = X is A, V, I, S, M, H, L, F, Y, G or W or can be a unnatural aliphatic amino acid residue such as Nle, Abu, Nva, 2-aminopentoic acid,or 2-aminohexaanoic acid
  SITE 37: note = X is any amino acid excluding C

SEQ ID NO: 206 - protein, 39 aa, Anabaena variabilis; identical to SEQ ID NO: 134
  SITE 36: note = X is A, V, I, S, M, H, L, F, Y, G or W or can be a unnatural aliphatic amino acid residue such as Nle, Abu, Nva, 2-aminopentoic acid,or 2-aminohexaanoic acid
  SITE 37: note = X is any amino acid excluding C

SEQ ID NO: 207 - protein, 39 aa, Cylindrospermopsis raciborskii; identical to SEQ ID NO: 135
  SITE 36: note = X is A, V, I, S, M, H, L, F, Y, G or W or can be a unnatural aliphatic amino acid residue such as Nle, Abu, Nva, 2-aminopentoic acid,or 2-aminohexaanoic acid
  SITE 37: note = X is any amino acid excluding C

SEQ ID NO: 208 - protein, 39 aa, Cyanothece CCY0110; identical to SEQ ID NO: 136
  SITE 36: note = X is A, V, I, S, M, H, L, F, Y, G or W or can be a unnatural aliphatic amino acid residue such as Nle, Abu, Nva, 2-aminopentoic acid,or 2-aminohexaanoic acid
  SITE 37: note = X is any amino acid excluding C

SEQ ID NO: 209 - protein, 39 aa, Cyanothece PCC8801; identical to SEQ ID NO: 137
  SITE 36: note = X is A, V, I, S, M, H, L, F, Y, G or W or can be a unnatural aliphatic amino acid residue such as Nle, Abu, Nva, 2-aminopentoic acid,or 2-aminohexaanoic acid
  SITE 37: note = X is any amino acid excluding C

SEQ ID NO: 210 - protein, 39 aa, Crocosphaera watsonii; identical to SEQ ID NO: 138
  SITE 36: note = X is A, V, I, S, M, H, L, F, Y, G or W or can be a unnatural aliphatic amino acid residue such as Nle, Abu, Nva, 2-aminopentoic acid,or 2-aminohexaanoic acid
  SITE 37: note = X is any amino acid excluding C

SEQ ID NO: 211 - protein, 39 aa, Microcystis aeruginosa; identical to SEQ ID NO: 139
  SITE 36: note = X is A, V, I, S, M, H, L, F, Y, G or W or can be a unnatural aliphatic amino acid residue such as Nle, Abu, Nva, 2-aminopentoic acid,or 2-aminohexaanoic acid
  SITE 37: note = X is any amino acid excluding C

SEQ ID NO: 212 - protein, 39 aa, Microcoleus chthonoplastes; identical to SEQ ID NO: 140
  SITE 36: note = X is A, V, I, S, M, H, L, F, Y, G or W or can be a unnatural aliphatic amino acid residue such as Nle, Abu, Nva, 2-aminopentoic acid,or 2-aminohexaanoic acid
  SITE 37: note = X is any amino acid excluding C

SEQ ID NO: 213 - protein, 39 aa, Oscillatoria limnetica; identical to SEQ ID NO: 140
  SITE 36: note = X is A, V, I, S, M, H, L, F, Y, G or W or can be a unnatural aliphatic amino acid residue such as Nle, Abu, Nva, 2-aminopentoic acid,or 2-aminohexaanoic acid
  SITE 37: note = X is any amino acid excluding C

SEQ ID NO: 214 - protein, 39 aa, Synechococcus elongatus; identical to SEQ ID NO: 142
  SITE 36: note = X is A, V, I, S, M, H, L, F, Y, G or W or can be a unnatural aliphatic amino acid residue such as Nle, Abu, Nva, 2-aminopentoic acid,or 2-aminohexaanoic acid
  SITE 37: note = X is any amino acid excluding C

SEQ ID NO: 215 - protein, 39 aa, Synechococcus PCC7002; identical to SEQ ID NO: 143
  SITE 36: note = X is A, V, I, S, M, H, L, F, Y, G or W or can be a unnatural aliphatic amino acid residue such as Nle, Abu, Nva, 2-aminopentoic acid,or 2-aminohexaanoic acid
  SITE 37: note = X is any amino acid excluding C

SEQ ID NO: 216 - protein, 38 aa, Thermosynechococcus elongatus; identical to SEQ ID NO: 144
  SITE 35: note = X is A, V, I, S, M, H, L, F, Y, G or W or can be a unnatural aliphatic amino acid residue such as Nle, Abu, Nva, 2-aminopentoic acid,or 2-aminohexaanoic acid
  SITE 36: note = X is any amino acid excluding C

SEQ ID NO: 217 - protein, 39 aa, Trichodesmium erythraeum; identical to SEQ ID NO: 145
  SITE 36: note = X is A, V, I, S, M, H, L, F, Y, G or W or can be a unnatural aliphatic amino acid residue such as Nle, Abu, Nva, 2-aminopentoic acid,or 2-aminohexaanoic acid
  SITE 37: note = X is any amino acid excluding N

SEQ ID NO: 218 - protein, 38 aa, Thermosynechococcus vulcanus; identical to SEQ ID NO: 146
  SITE 35: note = X is A, V, I, S, M, H, L, F, Y, G or W or can be a unnatural aliphatic amino acid residue such as Nle, Abu, Nva, 2-aminopentoic acid,or 2-aminohexaanoic acid
  SITE 36: note = X is any amino acid excluding C

SEQ ID NO: 219 - protein, 39 aa, Nostoc punctiforme; identical to SEQ ID NO: 129
  SITE 36: note = X is A, V, I, S, M, H, L, F, Y, G or W or can be a unnatural aliphatic amino acid residue such as Nle, Abu, Nva, 2-aminopentoic acid,or 2-aminohexaanoic acid
  SITE 37: note = X is A, V, I, S, M, H, L, F, Y, G or W or can be a unnatural aliphatic amino acid residue such as Nle, Abu, Nva, 2-aminopentoic acid,or 2-aminohexaanoic acid

SEQ ID NO: 220 - protein, 39 aa, Synechocystis PCC6803; identical to SEQ ID NO: 130
  SITE 36: note = X is A, V, I, S, M, H, L, F, Y, G or W or can be a unnatural aliphatic amino acid residue such as Nle, Abu, Nva, 2-aminopentoic acid,or 2-aminohexaanoic acid
  SITE 37: note = X is A, V, I, S, M, H, L, F, Y, G or W or can be a unnatural aliphatic amino acid residue such as Nle, Abu, Nva, 2-aminopentoic acid,or 2-aminohexaanoic acid

SEQ ID NO: 221 - protein, 39 aa, Aphanothece halophytica; identical to SEQ ID NO: 131
  SITE 36: note = X is A, V, I, S, M, H, L, F, Y, G or W or can be a unnatural aliphatic amino acid residue such as Nle, Abu, Nva, 2-aminopentoic acid,or 2-aminohexaanoic acid
  SITE 37: note = X is A, V, I, S, M, H, L, F, Y, G or W or can be a unnatural aliphatic amino acid residue such as Nle, Abu, Nva, 2-aminopentoic acid,or 2-aminohexaanoic acid

SEQ ID NO: 222 - protein, 39 aa, Aphanizomenon ovalisporum; identical to SEQ ID NO: 132
  SITE 36: note = X is A, V, I, S, M, H, L, F, Y, G or W or can be a unnatural aliphatic amino acid residue such as Nle, Abu, Nva, 2-aminopentoic acid,or 2-aminohexaanoic acid
  SITE 37: note = X is A, V, I, S, M, H, L, F, Y, G or W or can be a unnatural aliphatic amino acid residue such as Nle, Abu, Nva, 2-aminopentoic acid,or 2-aminohexaanoic acid

SEQ ID NO: 223 - protein, 39 aa, Anabaena PCC7120; identical to SEQ ID NO: 133
  SITE 36: note = X is A, V, I, S, M, H, L, F, Y, G or W or can be a unnatural aliphatic amino acid residue such as Nle, Abu, Nva, 2-aminopentoic acid,or 2-aminohexaanoic acid
  SITE 37: note = X is A, V, I, S, M, H, L, F, Y, G or W or can be a unnatural aliphatic amino acid residue such as Nle, Abu, Nva, 2-aminopentoic acid,or 2-aminohexaanoic acid

SEQ ID NO: 224 - protein, 39 aa, Anabaena variabilis; identical to SEQ ID NO: 134
  SITE 36: note = X is A, V, I, S, M, H, L, F, Y, G or W or can be a unnatural aliphatic amino acid residue such as Nle, Abu, Nva, 2-aminopentoic acid,or 2-aminohexaanoic acid
  SITE 37: note = X is A, V, I, S, M, H, L, F, Y, G or W or can be a unnatural aliphatic amino acid residue such as Nle, Abu, Nva, 2-aminopentoic acid,or 2-aminohexaanoic acid

SEQ ID NO: 225 - protein, 39 aa, Cylindrospermopsis raciborskii; identical to SEQ ID NO: 135
  SITE 36: note = X is A, V, I, S, M, H, L, F, Y, G or W or can be a unnatural aliphatic amino acid residue such as Nle, Abu, Nva, 2-aminopentoic acid,or 2-aminohexaanoic acid
  SITE 37: note = X is A, V, I, S, M, H, L, F, Y, G or W or can be a unnatural aliphatic amino acid residue such as Nle, Abu, Nva, 2-aminopentoic acid,or 2-aminohexaanoic acid

SEQ ID NO: 226 - protein, 39 aa, Cyanothece CCY0110; identical to SEQ ID NO: 136
  SITE 36: note = X is A, V, I, S, M, H, L, F, Y, G or W or can be a unnatural aliphatic amino acid residue such as Nle, Abu, Nva, 2-aminopentoic acid,or 2-aminohexaanoic acid
  SITE 37: note = X is A, V, I, S, M, H, L, F, Y, G or W or can be a unnatural aliphatic amino acid residue such as Nle, Abu, Nva, 2-aminopentoic acid,or 2-aminohexaanoic acid

SEQ ID NO: 227 - protein, 39 aa, Cyanothece PCC8801; identical to SEQ ID NO: 137
  SITE 36: note = X is A, V, I, S, M, H, L, F, Y, G or W or can be a unnatural aliphatic amino acid residue such as Nle, Abu, Nva, 2-aminopentoic acid,or 2-aminohexaanoic acid
  SITE 37: note = X is A, V, I, S, M, H, L, F, Y, G or W or can be a unnatural aliphatic amino acid residue such as Nle, Abu, Nva, 2-aminopentoic acid,or 2-aminohexaanoic acid

SEQ ID NO: 228 - protein, 39 aa, Crocosphaera watsonii; identical to SEQ ID NO: 138
  SITE 36: note = X is A, V, I, S, M, H, L, F, Y, G or W or can be a unnatural aliphatic amino acid residue such as Nle, Abu, Nva, 2-aminopentoic acid,or 2-aminohexaanoic acid
  SITE 37: note = X is A, V, I, S, M, H, L, F, Y, G or W or can be a unnatural aliphatic amino acid residue such as Nle, Abu, Nva, 2-aminopentoic acid,or 2-aminohexaanoic acid

SEQ ID NO: 229 - protein, 39 aa, Microcystis aeruginosa; identical to SEQ ID NO: 139
  SITE 36: note = X is A, V, I, S, M, H, L, F, Y, G or W or can be a unnatural aliphatic amino acid residue such as Nle, Abu, Nva, 2-aminopentoic acid,or 2-aminohexaanoic acid
  SITE 37: note = X is A, V, I, S, M, H, L, F, Y, G or W or can be a unnatural aliphatic amino acid residue such as Nle, Abu, Nva, 2-aminopentoic acid,or 2-aminohexaanoic acid

SEQ ID NO: 230 - protein, 39 aa, Microcoleus chthonoplastes; identical to SEQ ID NO: 140
  SITE 36: note = X is A, V, I, S, M, H, L, F, Y, G or W or can be a unnatural aliphatic amino acid residue such as Nle, Abu, Nva, 2-aminopentoic acid,or 2-aminohexaanoic acid
  SITE 37: note = X is A, V, I, S, M, H, L, F, Y, G or W or can be a unnatural aliphatic amino acid residue such as Nle, Abu, Nva, 2-aminopentoic acid,or 2-aminohexaanoic acid

SEQ ID NO: 231 - protein, 39 aa, Oscillatoria limnetica; identical to SEQ ID NO: 140
  SITE 36: note = X is A, V, I, S, M, H, L, F, Y, G or W or can be a unnatural aliphatic amino acid residue such as Nle, Abu, Nva, 2-aminopentoic acid,or 2-aminohexaanoic acid
  SITE 37: note = X is A, V, I, S, M, H, L, F, Y, G or W or can be a unnatural aliphatic amino acid residue such as Nle, Abu, Nva, 2-aminopentoic acid,or 2-aminohexaanoic acid

SEQ ID NO: 232 - protein, 39 aa, Synechococcus elongatus; identical to SEQ ID NO: 142
  SITE 36: note = X is A, V, I, S, M, H, L, F, Y, G or W or can be a unnatural aliphatic amino acid residue such as Nle, Abu, Nva, 2-aminopentoic acid,or 2-aminohexaanoic acid
  SITE 37: note = X is A, V, I, S, M, H, L, F, Y, G or W or can be a unnatural aliphatic amino acid residue such as Nle, Abu, Nva, 2-aminopentoic acid,or 2-aminohexaanoic acid

SEQ ID NO: 233 - protein, 39 aa, Synechococcus PCC7002; identical to SEQ ID NO: 143
  SITE 36: note = X is A, V, I, S, M, H, L, F, Y, G or W or can be a unnatural aliphatic amino acid residue such as Nle, Abu, Nva, 2-aminopentoic acid,or 2-aminohexaanoic acid
  SITE 37: note = X is A, V, I, S, M, H, L, F, Y, G or W or can be a unnatural aliphatic amino acid residue such as Nle, Abu, Nva, 2-aminopentoic acid,or 2-aminohexaanoic acid

SEQ ID NO: 234 - protein, 38 aa, Thermosynechococcus elongatus; identical to SEQ ID NO: 144
  SITE 35: note = X is A, V, I, S, M, H, L, F, Y, G or W or can be a unnatural aliphatic amino acid residue such as Nle, Abu, Nva, 2-aminopentoic acid,or 2-aminohexaanoic acid
  SITE 36: note = X is A, V, I, S, M, H, L, F, Y, G or W or can be a unnatural aliphatic amino acid residue such as Nle, Abu, Nva, 2-aminopentoic acid,or 2-aminohexaanoic acid

SEQ ID NO: 235 - protein, 39 aa, Trichodesmium erythraeum; identical to SEQ ID NO: 145
  SITE 36: note = X is A, V, I, S, M, H, L, F, Y, G or W or can be a unnatural aliphatic amino acid residue such as Nle, Abu, Nva, 2-aminopentoic acid,or 2-aminohexaanoic acid
  SITE 37: note = X is A, V, I, S, M, H, L, F, Y, G or W or can be a unnatural aliphatic amino acid residue such as Nle, Abu, Nva, 2-aminopentoic acid,or 2-aminohexaanoic acid

SEQ ID NO: 236 - protein, 38 aa, Thermosynechococcus vulcanus; identical to SEQ ID NO: 146
  SITE 35: note = X is A, V, I, S, M, H, L, F, Y, G or W or can be a unnatural aliphatic amino acid residue such as Nle, Abu, Nva, 2-aminopentoic acid,or 2-aminohexaanoic acid
  SITE 36: note = X is A, V, I, S, M, H, L, F, Y, G or W or can be a unnatural aliphatic amino acid residue such as Nle, Abu, Nva, 2-aminopentoic acid,or 2-aminohexaanoic acid

SEQ ID NO: 237 - protein, 39 aa, Nostoc punctiforme; identical to SEQ ID NO: 129
  SITE 36: note = X is A, V, I, S, M, H, L, F, Y, G or W or can be a unnatural aliphatic amino acid residue such as Nle, Abu, Nva, 2-aminopentoic acid,or 2-aminohexaanoic acid
  SITE 37: note = X is A, I, V, L, Y, G or F

SEQ ID NO: 238 - protein, 39 aa, Synechocystis PCC6803; identical to SEQ ID NO: 130
  SITE 36: note = X is A, V, I, S, M, H, L, F, Y, G or W or can be a unnatural aliphatic amino acid residue such as Nle, Abu, Nva, 2-aminopentoic acid,or 2-aminohexaanoic acid
  SITE 37: note = X is A, I, V, L, Y, G or F

SEQ ID NO: 239 - protein, 39 aa, Aphanothece halophytica; identical to SEQ ID NO: 131
  SITE 36: note = X is A, V, I, S, M, H, L, F, Y, G or W or can be a unnatural aliphatic amino acid residue such as Nle, Abu, Nva, 2-aminopentoic acid,or 2-aminohexaanoic acid
  SITE 37: note = X is A, I, V, L, Y, G or F

SEQ ID NO: 240 - protein, 39 aa, Aphanizomenon ovalisporum; identical to SEQ ID NO: 132
  SITE 36: note = X is A, V, I, S, M, H, L, F, Y, G or W or can be a unnatural aliphatic amino acid residue such as Nle, Abu, Nva, 2-aminopentoic acid,or 2-aminohexaanoic acid
  SITE 37: note = X is A, I, V, L, Y, G or F

SEQ ID NO: 241 - protein, 39 aa, Anabaena PCC7120; identical to SEQ ID NO: 133
  SITE 36: note = X is A, V, I, S, M, H, L, F, Y, G or W or can be a unnatural aliphatic amino acid residue such as Nle, Abu, Nva, 2-aminopentoic acid,or 2-aminohexaanoic acid
  SITE 37: note = X is A, I, V, L, Y, G or F

SEQ ID NO: 242 - protein, 39 aa, Anabaena variabilis; identical to SEQ ID NO: 134
  SITE 36: note = X is A, V, I, S, M, H, L, F, Y, G or W or can be a unnatural aliphatic amino acid residue such as Nle, Abu, Nva, 2-aminopentoic acid,or 2-aminohexaanoic acid
  SITE 37: note = X is A, I, V, L, Y, G or F

SEQ ID NO: 243 - protein, 39 aa, Cylindrospermopsis raciborskii; identical to SEQ ID NO: 135
  SITE 36: note = X is A, V, I, S, M, H, L, F, Y, G or W or can be a unnatural aliphatic amino acid residue such as Nle, Abu, Nva, 2-aminopentoic acid,or 2-aminohexaanoic acid
  SITE 37: note = X is A, I, V, L, Y, G or F

SEQ ID NO: 244 - protein, 39 aa, Cyanothece CCY0110; identical to SEQ ID NO: 136
  SITE 36: note = X is A, V, I, S, M, H, L, F, Y, G or W or can be a unnatural aliphatic amino acid residue such as Nle, Abu, Nva, 2-aminopentoic acid,or 2-aminohexaanoic acid
  SITE 37: note = X is A, I, V, L, Y, G or F

SEQ ID NO: 245 - protein, 39 aa, Cyanothece PCC8801; identical to SEQ ID NO: 137
  SITE 36: note = X is A, V, I, S, M, H, L, F, Y, G or W or can be a unnatural aliphatic amino acid residue such as Nle, Abu, Nva, 2-aminopentoic acid,or 2-aminohexaanoic acid
  SITE 37: note = X is A, I, V, L, Y, G or F

SEQ ID NO: 246 - protein, 39 aa, Crocosphaera watsonii; identical to SEQ ID NO: 138
  SITE 36: note = X is A, V, I, S, M, H, L, F, Y, G or W or can be a unnatural aliphatic amino acid residue such as Nle, Abu, Nva, 2-aminopentoic acid,or 2-aminohexaanoic acid
  SITE 37: note = X is A, I, V, L, Y, G or F

SEQ ID NO: 247 - protein, 39 aa, Microcystis aeruginosa; identical to SEQ ID NO: 139
  SITE 36: note = X is A, V, I, S, M, H, L, F, Y, G or W or can be a unnatural aliphatic amino acid residue such as Nle, Abu, Nva, 2-aminopentoic acid,or 2-aminohexaanoic acid
  SITE 37: note = X is A, I, V, L, Y, G or F

SEQ ID NO: 248 - protein, 39 aa, Microcoleus chthonoplastes; identical to SEQ ID NO: 140
  SITE 36: note = X is A, V, I, S, M, H, L, F, Y, G or W or can be a unnatural aliphatic amino acid residue such as Nle, Abu, Nva, 2-aminopentoic acid,or 2-aminohexaanoic acid
  SITE 37: note = X is A, I, V, L, Y, G or F

SEQ ID NO: 249 - protein, 39 aa, Oscillatoria limnetica; identical to SEQ ID NO: 140
  SITE 36: note = X is A, V, I, S, M, H, L, F, Y, G or W or can be a unnatural aliphatic amino acid residue such as Nle, Abu, Nva, 2-aminopentoic acid,or 2-aminohexaanoic acid
  SITE 37: note = X is A, I, V, L, Y, G or F

SEQ ID NO: 250 - protein, 39 aa, Synechococcus elongatus; identical to SEQ ID NO: 142
  SITE 36: note = X is A, V, I, S, M, H, L, F, Y, G or W or can be a unnatural aliphatic amino acid residue such as Nle, Abu, Nva, 2-aminopentoic acid,or 2-aminohexaanoic acid
  SITE 37: note = X is A, I, V, L, Y, G or F

SEQ ID NO: 251 - protein, 39 aa, Synechococcus PCC7002; identical to SEQ ID NO: 143
  SITE 36: note = X is A, V, I, S, M, H, L, F, Y, G or W or can be a unnatural aliphatic amino acid residue such as Nle, Abu, Nva, 2-aminopentoic acid,or 2-aminohexaanoic acid
  SITE 37: note = X is A, I, V, L, Y, G or F

SEQ ID NO: 252 - protein, 38 aa, Thermosynechococcus elongatus; identical to SEQ ID NO: 144
  SITE 35: note = X is A, V, I, S, M, H, L, F, Y, G or W or can be a unnatural aliphatic amino acid residue such as Nle, Abu, Nva, 2-aminopentoic acid,or 2-aminohexaanoic acid
  SITE 36: note = X is A, I, V, L, Y, G or F

SEQ ID NO: 253 - protein, 39 aa, Trichodesmium erythraeum; identical to SEQ ID NO: 145
  SITE 36: note = X is A, V, I, S, M, H, L, F, Y, G or W or can be a unnatural aliphatic amino acid residue such as Nle, Abu, Nva, 2-aminopentoic acid,or 2-aminohexaanoic acid
  SITE 37: note = X is A, I, V, L, Y, G or F

SEQ ID NO: 254 - protein, 38 aa, Thermosynechococcus vulcanus; identical to SEQ ID NO: 146
  SITE 35: note = X is A, V, I, S, M, H, L, F, Y, G or W or can be a unnatural aliphatic amino acid residue such as Nle, Abu, Nva, 2-aminopentoic acid,or 2-aminohexaanoic acid
  SITE 36: note = X is A, I, V, L, Y, G or F

SEQ ID NO: 255 - protein, 39 aa, Nostoc punctiforme; identical to SEQ ID NO: 183
  SITE 36: note = X is A, V, I, S, M, H, L, F, Y, G or W or can be a unnatural aliphatic amino acid residue such as Nle, Abu, Nva, 2-aminopentoic acid,or 2-aminohexaanoic acid

SEQ ID NO: 256 - protein, 39 aa, Synechocystis PCC6803; identical to SEQ ID NO: 184
  SITE 36: note = X is A, V, I, S, M, H, L, F, Y, G or W or can be a unnatural aliphatic amino acid residue such as Nle, Abu, Nva, 2-aminopentoic acid,or 2-aminohexaanoic acid

SEQ ID NO: 257 - protein, 39 aa, Aphanothece halophytica; identical to SEQ ID NO: 185
  SITE 36: note = X is A, V, I, S, M, H, L, F, Y, G or W or can be a unnatural aliphatic amino acid residue such as Nle, Abu, Nva, 2-aminopentoic acid,or 2-aminohexaanoic acid

SEQ ID NO: 258 - protein, 39 aa, Aphanizomenon ovalisporum; identical to SEQ ID NO: 186
  SITE 36: note = X is A, V, I, S, M, H, L, F, Y, G or W or can be a unnatural aliphatic amino acid residue such as Nle, Abu, Nva, 2-aminopentoic acid,or 2-aminohexaanoic acid

SEQ ID NO: 259 - protein, 39 aa, Anabaena PCC7120; identical to SEQ ID NO: 187
  SITE 36: note = X is A, V, I, S, M, H, L, F, Y, G or W or can be a unnatural aliphatic amino acid residue such as Nle, Abu, Nva, 2-aminopentoic acid,or 2-aminohexaanoic acid

SEQ ID NO: 260 - protein, 39 aa, Anabaena variabilis; identical to SEQ ID NO: 188
  SITE 36: note = X is A, V, I, S, M, H, L, F, Y, G or W or can be a unnatural aliphatic amino acid residue such as Nle, Abu, Nva, 2-aminopentoic acid,or 2-aminohexaanoic acid

SEQ ID NO: 261 - protein, 39 aa, Cylindrospermopsis raciborskii; identical to SEQ ID NO: 189
  SITE 36: note = X is A, V, I, S, M, H, L, F, Y, G or W or can be a unnatural aliphatic amino acid residue such as Nle, Abu, Nva, 2-aminopentoic acid,or 2-aminohexaanoic acid

SEQ ID NO: 262 - protein, 39 aa, Cyanothece CCY0110; identical to SEQ ID NO: 190
  SITE 36: note = X is A, V, I, S, M, H, L, F, Y, G or W or can be a unnatural aliphatic amino acid residue such as Nle, Abu, Nva, 2-aminopentoic acid,or 2-aminohexaanoic acid

SEQ ID NO: 263 - protein, 39 aa, Cyanothece PCC8801; identical to SEQ ID NO: 191
  SITE 36: note = X is A, V, I, S, M, H, L, F, Y, G or W or can be a unnatural aliphatic amino acid residue such as Nle, Abu, Nva, 2-aminopentoic acid,or 2-aminohexaanoic acid

SEQ ID NO: 264 - protein, 39 aa, Crocosphaera watsonii; identical to SEQ ID NO: 192
  SITE 36: note = X is A, V, I, S, M, H, L, F, Y, G or W or can be a unnatural aliphatic amino acid residue such as Nle, Abu, Nva, 2-aminopentoic acid,or 2-aminohexaanoic acid

SEQ ID NO: 265 - protein, 39 aa, Microcystis aeruginosa; identical to SEQ ID NO: 193
  SITE 36: note = X is A, V, I, S, M, H, L, F, Y, G or W or can be a unnatural aliphatic amino acid residue such as Nle, Abu, Nva, 2-aminopentoic acid,or 2-aminohexaanoic acid

SEQ ID NO: 266 - protein, 39 aa, Microcoleus chthonoplastes; identical to SEQ ID NO: 194
  SITE 36: note = X is A, V, I, S, M, H, L, F, Y, G or W or can be a unnatural aliphatic amino acid residue such as Nle, Abu, Nva, 2-aminopentoic acid,or 2-aminohexaanoic acid

SEQ ID NO: 267 - protein, 39 aa, Oscillatoria limnetica; identical to SEQ ID NO: 194
  SITE 36: note = X is A, V, I, S, M, H, L, F, Y, G or W or can be a unnatural aliphatic amino acid residue such as Nle, Abu, Nva, 2-aminopentoic acid,or 2-aminohexaanoic acid

SEQ ID NO: 268 - protein, 39 aa, Synechococcus elongatus; identical to SEQ ID NO: 196
  SITE 36: note = X is A, V, I, S, M, H, L, F, Y, G or W or can be a unnatural aliphatic amino acid residue such as Nle, Abu, Nva, 2-aminopentoic acid,or 2-aminohexaanoic acid

SEQ ID NO: 269 - protein, 39 aa, Synechococcus PCC7002; identical to SEQ ID NO: 197
  SITE 36: note = X is A, V, I, S, M, H, L, F, Y, G or W or can be a unnatural aliphatic amino acid residue such as Nle, Abu, Nva, 2-aminopentoic acid,or 2-aminohexaanoic acid

SEQ ID NO: 270 - protein, 38 aa, Thermosynechococcus elongatus; identical to SEQ ID NO: 198
  SITE 35: note = X is A, V, I, S, M, H, L, F, Y, G or W or can be a unnatural aliphatic amino acid residue such as Nle, Abu, Nva, 2-aminopentoic acid,or 2-aminohexaanoic acid

SEQ ID NO: 271 - protein, 39 aa, Trichodesmium erythraeum; identical to SEQ ID NO: 199
  SITE 36: note = X is A, V, I, S, M, H, L, F, Y, G or W or can be a unnatural aliphatic amino acid residue such as Nle, Abu, Nva, 2-aminopentoic acid,or 2-aminohexaanoic acid

SEQ ID NO: 272 - protein, 38 aa, Thermosynechococcus vulcanus; identical to SEQ ID NO: 200
  SITE 35: note = X is A, V, I, S, M, H, L, F, Y, G or W or can be a unnatural aliphatic amino acid residue such as Nle, Abu, Nva, 2-aminopentoic acid,or 2-aminohexaanoic acid

SEQ ID NO: 273 - protein, 39 aa, Nostoc punctiforme; identical to SEQ ID NO: 129
  SITE 36: note = X is A, I, V, L, Y, G or F
  SITE 37: note = X is any amino acid excluding C

SEQ ID NO: 274 - protein, 39 aa, Synechocystis PCC6803; identical to SEQ ID NO: 130
  SITE 36: note = X is A, I, V, L, Y, G or F
  SITE 37: note = X is any amino acid excluding C

SEQ ID NO: 275 - protein, 39 aa, Aphanothece halophytica; identical to SEQ ID NO: 131
  SITE 36: note = X is A, I, V, L, Y, G or F
  SITE 37: note = X is any amino acid excluding C

SEQ ID NO: 276 - protein, 39 aa, Aphanizomenon ovalisporum; identical to SEQ ID NO: 132
  SITE 36: note = X is A, I, V, L, Y, G or F
  SITE 37: note = X is any amino acid excluding C

SEQ ID NO: 277 - protein, 39 aa, Anabaena PCC7120; identical to SEQ ID NO: 133
  SITE 36: note = X is A, I, V, L, Y, G or F
  SITE 37: note = X is any amino acid excluding C

SEQ ID NO: 278 - protein, 39 aa, Anabaena variabilis; identical to SEQ ID NO: 134
  SITE 36: note = X is A, I, V, L, Y, G or F
  SITE 37: note = X is any amino acid excluding C

SEQ ID NO: 279 - protein, 39 aa, Cylindrospermopsis raciborskii; identical to SEQ ID NO: 135
  SITE 36: note = X is A, I, V, L, Y, G or F
  SITE 37: note = X is any amino acid excluding C

SEQ ID NO: 280 - protein, 39 aa, Cyanothece CCY0110; identical to SEQ ID NO: 136
  SITE 36: note = X is A, I, V, L, Y, G or F
  SITE 37: note = X is any amino acid excluding C

SEQ ID NO: 281 - protein, 39 aa, Cyanothece PCC8801; identical to SEQ ID NO: 137
  SITE 36: note = X is A, I, V, L, Y, G or F
  SITE 37: note = X is any amino acid excluding C

SEQ ID NO: 282 - protein, 39 aa, Crocosphaera watsonii; identical to SEQ ID NO: 138
  SITE 36: note = X is A, I, V, L, Y, G or F
  SITE 37: note = X is any amino acid excluding C

SEQ ID NO: 283 - protein, 39 aa, Microcystis aeruginosa; identical to SEQ ID NO: 139
  SITE 36: note = X is A, I, V, L, Y, G or F
  SITE 37: note = X is any amino acid excluding C

SEQ ID NO: 284 - protein, 39 aa, Microcoleus chthonoplastes; identical to SEQ ID NO: 140
  SITE 36: note = X is A, I, V, L, Y, G or F
  SITE 37: note = X is any amino acid excluding C

SEQ ID NO: 285 - protein, 39 aa, Oscillatoria limnetica; identical to SEQ ID NO: 140
  SITE 36: note = X is A, I, V, L, Y, G or F
  SITE 37: note = X is any amino acid excluding C

SEQ ID NO: 286 - protein, 39 aa, Synechococcus elongatus; identical to SEQ ID NO: 142
  SITE 36: note = X is A, I, V, L, Y, G or F
  SITE 37: note = X is any amino acid excluding C

SEQ ID NO: 287 - protein, 39 aa, Synechococcus PCC7002; identical to SEQ ID NO: 143
  SITE 36: note = X is A, I, V, L, Y, G or F
  SITE 37: note = X is any amino acid excluding C

SEQ ID NO: 288 - protein, 38 aa, Thermosynechococcus elongatus; identical to SEQ ID NO: 144
  SITE 35: note = X is A, I, V, L, Y, G or F
  SITE 36: note = X is any amino acid excluding C

SEQ ID NO: 289 - protein, 39 aa, Trichodesmium erythraeum; identical to SEQ ID NO: 145
  SITE 36: note = X is A, I, V, L, Y, G or F
  SITE 37: note = X is any amino acid excluding C

SEQ ID NO: 290 - protein, 38 aa, Thermosynechococcus vulcanus; identical to SEQ ID NO: 146
  SITE 35: note = X is A, I, V, L, Y, G or F
  SITE 36: note = X is any amino acid excluding C

SEQ ID NO: 291 - protein, 39 aa, Nostoc punctiforme; identical to SEQ ID NO: 129
  SITE 36: note = X is A, I, V, L, Y, G or F
  SITE 37: note = X is A, V, I, S, M, H, L, F, Y, G or W or can be a unnatural aliphatic amino acid residue such as Nle, Abu, Nva, 2-aminopentoic acid,or 2-aminohexaanoic acid

SEQ ID NO: 292 - protein, 39 aa, Synechocystis PCC6803; identical to SEQ ID NO: 130
  SITE 36: note = X is A, I, V, L, Y, G or F
  SITE 37: note = X is A, V, I, S, M, H, L, F, Y, G or W or can be a unnatural aliphatic amino acid residue such as Nle, Abu, Nva, 2-aminopentoic acid,or 2-aminohexaanoic acid

SEQ ID NO: 293 - protein, 39 aa, Aphanothece halophytica; identical to SEQ ID NO: 131
  SITE 36: note = X is A, I, V, L, Y, G or F
  SITE 37: note = X is A, V, I, S, M, H, L, F, Y, G or W or can be a unnatural aliphatic amino acid residue such as Nle, Abu, Nva, 2-aminopentoic acid,or 2-aminohexaanoic acid

SEQ ID NO: 294 - protein, 39 aa, Aphanizomenon ovalisporum; identical to SEQ ID NO: 132
  SITE 36: note = X is A, I, V, L, Y, G or F
  SITE 37: note = X is A, V, I, S, M, H, L, F, Y, G or W or can be a unnatural aliphatic amino acid residue such as Nle, Abu, Nva, 2-aminopentoic acid,or 2-aminohexaanoic acid

SEQ ID NO: 295 - protein, 39 aa, Anabaena PCC7120; identical to SEQ ID NO: 133
  SITE 36: note = X is A, I, V, L, Y, G or F
  SITE 37: note = X is A, V, I, S, M, H, L, F, Y, G or W or can be a unnatural aliphatic amino acid residue such as Nle, Abu, Nva, 2-aminopentoic acid,or 2-aminohexaanoic acid

SEQ ID NO: 296 - protein, 39 aa, Anabaena variabilis; identical to SEQ ID NO: 134
  SITE 36: note = X is A, I, V, L, Y, G or F
  SITE 37: note = X is A, V, I, S, M, H, L, F, Y, G or W or can be a unnatural aliphatic amino acid residue such as Nle, Abu, Nva, 2-aminopentoic acid,or 2-aminohexaanoic acid

SEQ ID NO: 297 - protein, 39 aa, Cylindrospermopsis raciborskii; identical to SEQ ID NO: 135
  SITE 36: note = X is A, I, V, L, Y, G or F
  SITE 37: note = X is A, V, I, S, M, H, L, F, Y, G or W or can be a unnatural aliphatic amino acid residue such as Nle, Abu, Nva, 2-aminopentoic acid,or 2-aminohexaanoic acid

SEQ ID NO: 298 - protein, 39 aa, Cyanothece CCY0110; identical to SEQ ID NO: 136
  SITE 36: note = X is A, I, V, L, Y, G or F
  SITE 37: note = X is A, V, I, S, M, H, L, F, Y, G or W or can be a unnatural aliphatic amino acid residue such as Nle, Abu, Nva, 2-aminopentoic acid,or 2-aminohexaanoic acid

SEQ ID NO: 299 - protein, 39 aa, Cyanothece PCC8801; identical to SEQ ID NO: 137
  SITE 36: note = X is A, I, V, L, Y, G or F
  SITE 37: note = X is A, V, I, S, M, H, L, F, Y, G or W or can be a unnatural aliphatic amino acid residue such as Nle, Abu, Nva, 2-aminopentoic acid,or 2-aminohexaanoic acid

SEQ ID NO: 300 - protein, 39 aa, Crocosphaera watsonii; identical to SEQ ID NO: 138
  SITE 36: note = X is A, I, V, L, Y, G or F
  SITE 37: note = X is A, V, I, S, M, H, L, F, Y, G or W or can be a unnatural aliphatic amino acid residue such as Nle, Abu, Nva, 2-aminopentoic acid,or 2-aminohexaanoic acid

SEQ ID NO: 301 - protein, 39 aa, Microcystis aeruginosa; identical to SEQ ID NO: 139
  SITE 36: note = X is A, I, V, L, Y, G or F
  SITE 37: note = X is A, V, I, S, M, H, L, F, Y, G or W or can be a unnatural aliphatic amino acid residue such as Nle, Abu, Nva, 2-aminopentoic acid,or 2-aminohexaanoic acid

SEQ ID NO: 302 - protein, 39 aa, Microcoleus chthonoplastes; identical to SEQ ID NO: 140
  SITE 36: note = X is A, I, V, L, Y, G or F
  SITE 37: note = X is A, V, I, S, M, H, L, F, Y, G or W or can be a unnatural aliphatic amino acid residue such as Nle, Abu, Nva, 2-aminopentoic acid,or 2-aminohexaanoic acid

SEQ ID NO: 303 - protein, 39 aa, Oscillatoria limnetica; identical to SEQ ID NO: 140
  SITE 36: note = X is A, I, V, L, Y, G or F
  SITE 37: note = X is A, V, I, S, M, H, L, F, Y, G or W or can be a unnatural aliphatic amino acid residue such as Nle, Abu, Nva, 2-aminopentoic acid,or 2-aminohexaanoic acid

SEQ ID NO: 304 - protein, 39 aa, Synechococcus elongatus; identical to SEQ ID NO: 142
  SITE 36: note = X is A, I, V, L, Y, G or F
  SITE 37: note = X is A, V, I, S, M, H, L, F, Y, G or W or can be a unnatural aliphatic amino acid residue such as Nle, Abu, Nva, 2-aminopentoic acid,or 2-aminohexaanoic acid

SEQ ID NO: 305 - protein, 39 aa, Synechococcus PCC7002; identical to SEQ ID NO: 143
  SITE 36: note = X is A, I, V, L, Y, G or F
  SITE 37: note = X is A, V, I, S, M, H, L, F, Y, G or W or can be a unnatural aliphatic amino acid residue such as Nle, Abu, Nva, 2-aminopentoic acid,or 2-aminohexaanoic acid

SEQ ID NO: 306 - protein, 38 aa, Thermosynechococcus elongatus; identical to SEQ ID NO: 144
  SITE 35: note = X is A, I, V, L, Y, G or F
  SITE 36: note = X is A, V, I, S, M, H, L, F, Y, G or W or can be a unnatural aliphatic amino acid residue such as Nle, Abu, Nva, 2-aminopentoic acid,or 2-aminohexaanoic acid

SEQ ID NO: 307 - protein, 39 aa, Trichodesmium erythraeum; identical to SEQ ID NO: 145
  SITE 36: note = X is A, I, V, L, Y, G or F
  SITE 37: note = X is A, V, I, S, M, H, L, F, Y, G or W or can be a unnatural aliphatic amino acid residue such as Nle, Abu, Nva, 2-aminopentoic acid,or 2-aminohexaanoic acid

SEQ ID NO: 308 - protein, 38 aa, Thermosynechococcus vulcanus; identical to SEQ ID NO: 146
  SITE 35: note = X is A, I, V, L, Y, G or F
  SITE 36: note = X is A, V, I, S, M, H, L, F, Y, G or W or can be a unnatural aliphatic amino acid residue such as Nle, Abu, Nva, 2-aminopentoic acid,or 2-aminohexaanoic acid

SEQ ID NO: 309 - protein, 39 aa, Nostoc punctiforme; identical to SEQ ID NO: 129
  SITE 36: note = X is A, I, V, L, Y, G or F
  SITE 37: note = X is A, I, V, L, Y, G or F

SEQ ID NO: 310 - protein, 39 aa, Synechocystis PCC6803; identical to SEQ ID NO: 130
  SITE 36: note = X is A, I, V, L, Y, G or F
  SITE 37: note = X is A, I, V, L, Y, G or F

SEQ ID NO: 311 - protein, 39 aa, Aphanothece halophytica; identical to SEQ ID NO: 131
  SITE 36: note = X is A, I, V, L, Y, G or F
  SITE 37: note = X is A, I, V, L, Y, G or F

SEQ ID NO: 312 - protein, 39 aa, Aphanizomenon ovalisporum; identical to SEQ ID NO: 132
  SITE 36: note = X is A, I, V, L, Y, G or F
  SITE 37: note = X is A, I, V, L, Y, G or F

SEQ ID NO: 313 - protein, 39 aa, Anabaena PCC7120; identical to SEQ ID NO: 133
  SITE 36: note = X is A, I, V, L, Y, G or F
  SITE 37: note = X is A, I, V, L, Y, G or F

SEQ ID NO: 314 - protein, 39 aa, Anabaena variabilis; identical to SEQ ID NO: 134
  SITE 36: note = X is A, I, V, L, Y, G or F
  SITE 37: note = X is A, I, V, L, Y, G or F

SEQ ID NO: 315 - protein, 39 aa, Cylindrospermopsis raciborskii; identical to SEQ ID NO: 135
  SITE 36: note = X is A, I, V, L, Y, G or F
  SITE 37: note = X is A, I, V, L, Y, G or F

SEQ ID NO: 316 - protein, 39 aa, Cyanothece CCY0110; identical to SEQ ID NO: 136
  SITE 36: note = X is A, I, V, L, Y, G or F
  SITE 37: note = X is A, I, V, L, Y, G or F

SEQ ID NO: 317 - protein, 39 aa, Cyanothece PCC8801; identical to SEQ ID NO: 137
  SITE 36: note = X is A, I, V, L, Y, G or F
  SITE 37: note = X is A, I, V, L, Y, G or F

SEQ ID NO: 318 - protein, 39 aa, Crocosphaera watsonii; identical to SEQ ID NO: 138
  SITE 36: note = X is A, I, V, L, Y, G or F
  SITE 37: note = X is A, I, V, L, Y, G or F

SEQ ID NO: 319 - protein, 39 aa, Microcystis aeruginosa; identical to SEQ ID NO: 139
  SITE 36: note = X is A, I, V, L, Y, G or F
  SITE 37: note = X is A, I, V, L, Y, G or F

SEQ ID NO: 320 - protein, 39 aa, Microcoleus chthonoplastes; identical to SEQ ID NO: 140
  SITE 36: note = X is A, I, V, L, Y, G or F
  SITE 37: note = X is A, I, V, L, Y, G or F

SEQ ID NO: 321 - protein, 39 aa, Oscillatoria limnetica; identical to SEQ ID NO: 140
  SITE 36: note = X is A, I, V, L, Y, G or F
  SITE 37: note = X is A, I, V, L, Y, G or F

SEQ ID NO: 322 - protein, 39 aa, Synechococcus elongatus; identical to SEQ ID NO: 142
  SITE 36: note = X is A, I, V, L, Y, G or F
  SITE 37: note = X is A, I, V, L, Y, G or F

SEQ ID NO: 323 - protein, 39 aa, Synechococcus PCC7002; identical to SEQ ID NO: 143
  SITE 36: note = X is A, I, V, L, Y, G or F
  SITE 37: note = X is A, I, V, L, Y, G or F

SEQ ID NO: 324 - protein, 38 aa, Thermosynechococcus elongatus; identical to SEQ ID NO: 144
  SITE 35: note = X is A, I, V, L, Y, G or F
  SITE 36: note = X is A, I, V, L, Y, G or F

SEQ ID NO: 325 - protein, 39 aa, Trichodesmium erythraeum; identical to SEQ ID NO: 145
  SITE 36: note = X is A, I, V, L, Y, G or F
  SITE 37: note = X is A, I, V, L, Y, G or F

SEQ ID NO: 326 - protein, 38 aa, Thermosynechococcus vulcanus; identical to SEQ ID NO: 146
  SITE 35: note = X is A, I, V, L, Y, G or F
  SITE 36: note = X is A, I, V, L, Y, G or F

SEQ ID NO: 327 - protein, 39 aa, Nostoc punctiforme; identical to SEQ ID NO: 183
  SITE 36: note = X is A, I, V, L, Y, G or F

SEQ ID NO: 328 - protein, 39 aa, Synechocystis PCC6803; identical to SEQ ID NO: 184
  SITE 36: note = X is A, I, V, L, Y, G or F

SEQ ID NO: 329 - protein, 39 aa, Aphanothece halophytica; identical to SEQ ID NO: 185
  SITE 36: note = X is A, I, V, L, Y, G or F

SEQ ID NO: 330 - protein, 39 aa, Aphanizomenon ovalisporum; identical to SEQ ID NO: 186
  SITE 36: note = X is A, I, V, L, Y, G or F

SEQ ID NO: 331 - protein, 39 aa, Anabaena PCC7120; identical to SEQ ID NO: 187
  SITE 36: note = X is A, I, V, L, Y, G or F

SEQ ID NO: 332 - protein, 39 aa, Anabaena variabilis; identical to SEQ ID NO: 188
  SITE 36: note = X is A, I, V, L, Y, G or F

SEQ ID NO: 333 - protein, 39 aa, Cylindrospermopsis raciborskii; identical to SEQ ID NO: 189
  SITE 36: note = X is A, I, V, L, Y, G or F

SEQ ID NO: 334 - protein, 39 aa, Cyanothece CCY0110; identical to SEQ ID NO: 190
  SITE 36: note = X is A, I, V, L, Y, G or F

SEQ ID NO: 335 - protein, 39 aa, Cyanothece PCC8801; identical to SEQ ID NO: 191
  SITE 36: note = X is A, I, V, L, Y, G or F

SEQ ID NO: 336 - protein, 39 aa, Crocosphaera watsonii; identical to SEQ ID NO: 192
  SITE 36: note = X is A, I, V, L, Y, G or F

SEQ ID NO: 337 - protein, 39 aa, Microcystis aeruginosa; identical to SEQ ID NO: 193
  SITE 36: note = X is A, I, V, L, Y, G or F

SEQ ID NO: 338 - protein, 39 aa, Microcoleus chthonoplastes; identical to SEQ ID NO: 194
  SITE 36: note = X is A, I, V, L, Y, G or F

SEQ ID NO: 339 - protein, 39 aa, Oscillatoria limnetica; identical to SEQ ID NO: 194
  SITE 36: note = X is A, I, V, L, Y, G or F

SEQ ID NO: 340 - protein, 39 aa, Synechococcus elongatus; identical to SEQ ID NO: 196
  SITE 36: note = X is A, I, V, L, Y, G or F

SEQ ID NO: 341 - protein, 39 aa, Synechococcus PCC7002; identical to SEQ ID NO: 197
  SITE 36: note = X is A, I, V, L, Y, G or F

SEQ ID NO: 342 - protein, 38 aa, Thermosynechococcus elongatus; identical to SEQ ID NO: 198
  SITE 35: note = X is A, I, V, L, Y, G or F

SEQ ID NO: 343 - protein, 39 aa, Trichodesmium erythraeum; identical to SEQ ID NO: 199
  SITE 36: note = X is A, I, V, L, Y, G or F

SEQ ID NO: 344 - protein, 38 aa, Thermosynechococcus vulcanus; identical to SEQ ID NO: 200
  SITE 35: note = X is A, I, V, L, Y, G or F

SEQ ID NO: 345 - protein, 39 aa, Nostoc punctiforme
  SITE 37: note = X is any amino acid excluding C
MIKIATRKYLGKQNVYDIGVERDHNFALKNGFIASAXFN

SEQ ID NO: 346 - protein, 39 aa, Synechocystis PCC6803
  SITE 37: note = X is any amino acid excluding C
MVKVIGRRSLGVQRIFDIGLPQDHNFLLANGAIAAAXFN

SEQ ID NO: 347 - protein, 39 aa, Aphanothece halophytica
  SITE 37: note = X is any amino acid excluding C
MVKIIKRQSLGRQNVYDVCVETDHNFVLANGCVASAXFN

SEQ ID NO: 348 - protein, 39 aa, Aphanizomenon ovalisporum
  SITE 37: note = X is any amino acid excluding C
MVKITARKFVGRENVYDIGVEHHHNFAIKNGLIASAXFN

SEQ ID NO: 349 - protein, 39 aa, Anabaena PCC7120
  SITE 37: note = X is any amino acid excluding C
MIKIASRKFLGVENVYDIGVRRDHNFFIKNGLIASAXFN

SEQ ID NO: 350 - protein, 39 aa, Anabaena variabilis
  SITE 37: note = X is any amino acid excluding C
MIKIASRKFLGVENVYDIGVGRDHNFFVKNGLIASAXFN

SEQ ID NO: 351 - protein, 39 aa, Cylindrospermopsis raciborskii
  SITE 37: note = X is any amino acid excluding C
MVKIVSRRYLGKADVYDIGVAKDHNFIIKNGLVASAXFN

SEQ ID NO: 352 - protein, 39 aa, Cyanothece CCY0110
  SITE 37: note = X is any amino acid excluding C
MVKIIERRSLGKQNVYDIGVEKDHNFLLSNNLIASAXFN

SEQ ID NO: 353 - protein, 39 aa, Cyanothece PCC8801
  SITE 37: note = X is any amino acid excluding C
MVKIVSYRSLGKQFVYDIGVAQDHNFLLANGSIASAXFN

SEQ ID NO: 354 - protein, 39 aa, Crocosphaera watsonii
  SITE 37: note = X is any amino acid excluding C
MVKIIGCRSLGTQKVYDIGVEKDHNFLLANGSIASAXFN

SEQ ID NO: 355 - protein, 39 aa, Microcystis aeruginosa
  SITE 37: note = X is any amino acid excluding C
MVKIIGRQSLGRKPVYDIGVEKDHNFLLGNGLIASAXFN

SEQ ID NO: 356 - protein, 39 aa, Microcoleus chthonoplastes
  SITE 37: note = X is any amino acid excluding C
MVKIVRRQSLGVQNVYDIGVEKDHNFCLASGEIASAXFN

SEQ ID NO: 357 - protein, 39 aa, Oscillatoria limnetica; identical to SEQ ID NO: 356
  SITE 37: note = X is any amino acid excluding C

SEQ ID NO: 358 - protein, 39 aa, Synechococcus elongatus
  SITE 37: note = X is any amino acid excluding C
MVKIVRRRSLGVQPVYDLGVATVHNFVLANGLVASAXFN

SEQ ID NO: 359 - protein, 39 aa, Synechococcus PCC7002
  SITE 37: note = X is any amino acid excluding C
MVKIIRRKFIGHAPTYDIGLSQDHNFLLGQGLIAAAXFN

SEQ ID NO: 360 - protein, 38 aa, Thermosynechococcus elongatus
  SITE 36: note = X is any amino acid excluding C
MKIVGRRLMGWQAVYDIGLAADHNFVLANGAIAAAXFN

SEQ ID NO: 361 - protein, 39 aa, Trichodesmium erythraeum
  SITE 37: note = X is any amino acid excluding C
MVKIVSRKLAKTENVYDIGVTKDHNFVLANGLIASAXFN

SEQ ID NO: 362 - protein, 38 aa, Thermosynechococcus vulcanus
  SITE 36: note = X is any amino acid excluding C
MKIVGRRLVGWQAVYDIGLAGDHNFLLANGAIAAAXFN

SEQ ID NO: 363 - protein, 39 aa, Nostoc punctiforme; identical to SEQ ID NO: 345
  SITE 37: note = X is A, V, I, S, M, H, L, F, Y, G or W or can be a unnatural aliphatic amino acid residue such as Nle, Abu, Nva, 2-aminopentoic acid,or 2-aminohexaanoic acid

SEQ ID NO: 364 - protein, 39 aa, Synechocystis PCC6803; identical to SEQ ID NO: 346
  SITE 37: note = X is A, V, I, S, M, H, L, F, Y, G or W or can be a unnatural aliphatic amino acid residue such as Nle, Abu, Nva, 2-aminopentoic acid,or 2-aminohexaanoic acid

SEQ ID NO: 365 - protein, 39 aa, Aphanothece halophytica; identical to SEQ ID NO: 347
  SITE 37: note = X is A, V, I, S, M, H, L, F, Y, G or W or can be a unnatural aliphatic amino acid residue such as Nle, Abu, Nva, 2-aminopentoic acid,or 2-aminohexaanoic acid

SEQ ID NO: 366 - protein, 39 aa, Aphanizomenon ovalisporum; identical to SEQ ID NO: 348
  SITE 37: note = X is A, V, I, S, M, H, L, F, Y, G or W or can be a unnatural aliphatic amino acid residue such as Nle, Abu, Nva, 2-aminopentoic acid,or 2-aminohexaanoic acid

SEQ ID NO: 367 - protein, 39 aa, Anabaena PCC7120; identical to SEQ ID NO: 349
  SITE 37: note = X is A, V, I, S, M, H, L, F, Y, G or W or can be a unnatural aliphatic amino acid residue such as Nle, Abu, Nva, 2-aminopentoic acid,or 2-aminohexaanoic acid

SEQ ID NO: 368 - protein, 39 aa, Anabaena variabilis; identical to SEQ ID NO: 350
  SITE 37: note = X is A, V, I, S, M, H, L, F, Y, G or W or can be a unnatural aliphatic amino acid residue such as Nle, Abu, Nva, 2-aminopentoic acid,or 2-aminohexaanoic acid

SEQ ID NO: 369 - protein, 39 aa, Cylindrospermopsis raciborskii; identical to SEQ ID NO: 351
  SITE 37: note = X is A, V, I, S, M, H, L, F, Y, G or W or can be a unnatural aliphatic amino acid residue such as Nle, Abu, Nva, 2-aminopentoic acid,or 2-aminohexaanoic acid

SEQ ID NO: 370 - protein, 39 aa, Cyanothece CCY0110; identical to SEQ ID NO: 352
  SITE 37: note = X is A, V, I, S, M, H, L, F, Y, G or W or can be a unnatural aliphatic amino acid residue such as Nle, Abu, Nva, 2-aminopentoic acid,or 2-aminohexaanoic acid

SEQ ID NO: 371 - protein, 39 aa, Cyanothece PCC8801; identical to SEQ ID NO: 353
  SITE 37: note = X is A, V, I, S, M, H, L, F, Y, G or W or can be a unnatural aliphatic amino acid residue such as Nle, Abu, Nva, 2-aminopentoic acid,or 2-aminohexaanoic acid

SEQ ID NO: 372 - protein, 39 aa, Crocosphaera watsonii; identical to SEQ ID NO: 354
  SITE 37: note = X is A, V, I, S, M, H, L, F, Y, G or W or can be a unnatural aliphatic amino acid residue such as Nle, Abu, Nva, 2-aminopentoic acid,or 2-aminohexaanoic acid

SEQ ID NO: 373 - protein, 39 aa, Microcystis aeruginosa; identical to SEQ ID NO: 355
  SITE 37: note = X is A, V, I, S, M, H, L, F, Y, G or W or can be a unnatural aliphatic amino acid residue such as Nle, Abu, Nva, 2-aminopentoic acid,or 2-aminohexaanoic acid

SEQ ID NO: 374 - protein, 39 aa, Microcoleus chthonoplastes; identical to SEQ ID NO: 356
  SITE 37: note = X is A, V, I, S, M, H, L, F, Y, G or W or can be a unnatural aliphatic amino acid residue such as Nle, Abu, Nva, 2-aminopentoic acid,or 2-aminohexaanoic acid

SEQ ID NO: 375 - protein, 39 aa, Oscillatoria limnetica; identical to SEQ ID NO: 356
  SITE 37: note = X is A, V, I, S, M, H, L, F, Y, G or W or can be a unnatural aliphatic amino acid residue such as Nle, Abu, Nva, 2-aminopentoic acid,or 2-aminohexaanoic acid

SEQ ID NO: 376 - protein, 39 aa, Synechococcus elongatus; identical to SEQ ID NO: 358
  SITE 37: note = X is A, V, I, S, M, H, L, F, Y, G or W or can be a unnatural aliphatic amino acid residue such as Nle, Abu, Nva, 2-aminopentoic acid,or 2-aminohexaanoic acid

SEQ ID NO: 377 - protein, 39 aa, Synechococcus PCC7002; identical to SEQ ID NO: 359
  SITE 37: note = X is A, V, I, S, M, H, L, F, Y, G or W or can be a unnatural aliphatic amino acid residue such as Nle, Abu, Nva, 2-aminopentoic acid,or 2-aminohexaanoic acid

SEQ ID NO: 378 - protein, 38 aa, Thermosynechococcus elongatus; identical to SEQ ID NO: 360
  SITE 36: note = X is A, V, I, S, M, H, L, F, Y, G or W or can be a unnatural aliphatic amino acid residue such as Nle, Abu, Nva, 2-aminopentoic acid,or 2-aminohexaanoic acid

SEQ ID NO: 379 - protein, 39 aa, Trichodesmium erythraeum; identical to SEQ ID NO: 361
  SITE 37: note = X is A, V, I, S, M, H, L, F, Y, G or W or can be a unnatural aliphatic amino acid residue such as Nle, Abu, Nva, 2-aminopentoic acid,or 2-aminohexaanoic acid

SEQ ID NO: 380 - protein, 38 aa, Thermosynechococcus vulcanus; identical to SEQ ID NO: 362
  SITE 36: note = X is A, V, I, S, M, H, L, F, Y, G or W or can be a unnatural aliphatic amino acid residue such as Nle, Abu, Nva, 2-aminopentoic acid,or 2-aminohexaanoic acid

SEQ ID NO: 381 - protein, 39 aa, Nostoc punctiforme; identical to SEQ ID NO: 345
  SITE 37: note = X is A, I, V, L, Y, G or F

SEQ ID NO: 382 - protein, 39 aa, Synechocystis PCC6803; identical to SEQ ID NO: 346
  SITE 37: note = X is A, I, V, L, Y, G or F

SEQ ID NO: 383 - protein, 39 aa, Aphanothece halophytica; identical to SEQ ID NO: 347
  SITE 37: note = X is A, I, V, L, Y, G or F

SEQ ID NO: 384 - protein, 39 aa, Aphanizomenon ovalisporum; identical to SEQ ID NO: 348
  SITE 37: note = X is A, I, V, L, Y, G or F

SEQ ID NO: 385 - protein, 39 aa, Anabaena PCC7120; identical to SEQ ID NO: 349
  SITE 37: note = X is A, I, V, L, Y, G or F

SEQ ID NO: 386 - protein, 39 aa, Anabaena variabilis; identical to SEQ ID NO: 350
  SITE 37: note = X is A, I, V, L, Y, G or F

SEQ ID NO: 387 - protein, 39 aa, Cylindrospermopsis raciborskii; identical to SEQ ID NO: 351
  SITE 37: note = X is A, I, V, L, Y, G or F

SEQ ID NO: 388 - protein, 39 aa, Cyanothece CCY0110; identical to SEQ ID NO: 352
  SITE 37: note = X is A, I, V, L, Y, G or F

SEQ ID NO: 389 - protein, 39 aa, Cyanothece PCC8801; identical to SEQ ID NO: 353
  SITE 37: note = X is A, I, V, L, Y, G or F

SEQ ID NO: 390 - protein, 39 aa, Crocosphaera watsonii; identical to SEQ ID NO: 354
  SITE 37: note = X is A, I, V, L, Y, G or F

SEQ ID NO: 391 - protein, 39 aa, Microcystis aeruginosa; identical to SEQ ID NO: 355
  SITE 37: note = X is A, I, V, L, Y, G or F

SEQ ID NO: 392 - protein, 39 aa, Microcoleus chthonoplastes; identical to SEQ ID NO: 356
  SITE 37: note = X is A, I, V, L, Y, G or F

SEQ ID NO: 393 - protein, 39 aa, Oscillatoria limnetica; identical to SEQ ID NO: 356
  SITE 37: note = X is A, I, V, L, Y, G or F

SEQ ID NO: 394 - protein, 39 aa, Synechococcus elongatus; identical to SEQ ID NO: 358
  SITE 37: note = X is A, I, V, L, Y, G or F

SEQ ID NO: 395 - protein, 39 aa, Synechococcus PCC7002; identical to SEQ ID NO: 359
  SITE 37: note = X is A, I, V, L, Y, G or F

SEQ ID NO: 396 - protein, 38 aa, Thermosynechococcus elongatus; identical to SEQ ID NO: 360
  SITE 36: note = X is A, I, V, L, Y, G or F

SEQ ID NO: 397 - protein, 39 aa, Trichodesmium erythraeum; identical to SEQ ID NO: 361
  SITE 37: note = X is A, I, V, L, Y, G or F

SEQ ID NO: 398 - protein, 38 aa, Thermosynechococcus vulcanus; identical to SEQ ID NO: 362
  SITE 36: note = X is A, I, V, L, Y, G or F

SEQ ID NO: 399 - protein, 39 aa, Nostoc punctiforme
MIKIATRKYLGKQNVYDIGVERDHNFALKNGFIASAAFN

SEQ ID NO: 400 - protein, 39 aa, Synechocystis PCC6803
MVKVIGRRSLGVQRIFDIGLPQDHNFLLANGAIAAAAFN

SEQ ID NO: 401 - protein, 39 aa, Aphanothece halophytica
MVKIIKRQSLGRQNVYDVCVETDHNFVLANGCVASAAFN

SEQ ID NO: 402 - protein, 39 aa, Aphanizomenon ovalisporum
MVKITARKFVGRENVYDIGVEHHHNFAIKNGLIASAAFN

SEQ ID NO: 403 - protein, 39 aa, Anabaena PCC7120
MIKIASRKFLGVENVYDIGVRRDHNFFIKNGLIASAAFN

SEQ ID NO: 404 - protein, 39 aa, Anabaena variabilis
MIKIASRKFLGVENVYDIGVGRDHNFFVKNGLIASAAFN

SEQ ID NO: 405 - protein, 39 aa, Cylindrospermopsis raciborskii
MVKIVSRRYLGKADVYDIGVAKDHNFIIKNGLVASAAFN

SEQ ID NO: 406 - protein, 39 aa, Cyanothece CCY0110
MVKIIERRSLGKQNVYDIGVEKDHNFLLSNNLIASAAFN

SEQ ID NO: 407 - protein, 39 aa, Cyanothece PCC8801
MVKIVSYRSLGKQFVYDIGVAQDHNFLLANGSIASAAFN

SEQ ID NO: 408 - protein, 39 aa, Crocosphaera watsonii
MVKIIGCRSLGTQKVYDIGVEKDHNFLLANGSIASAAFN

SEQ ID NO: 409 - protein, 39 aa, Microcystis aeruginosa
MVKIIGRQSLGRKPVYDIGVEKDHNFLLGNGLIASAAFN

SEQ ID NO: 410 - protein, 39 aa, Microcoleus chthonoplastes
MVKIVRRQSLGVQNVYDIGVEKDHNFCLASGEIASAAFN

SEQ ID NO: 411 - protein, 39 aa, Oscillatoria limnetica; identical to SEQ ID NO: 410

SEQ ID NO: 412 - protein, 39 aa, Synechococcus elongatus
MVKIVRRRSLGVQPVYDLGVATVHNFVLANGLVASAAFN

SEQ ID NO: 413 - protein, 39 aa, Synechococcus PCC7002
MVKIIRRKFIGHAPTYDIGLSQDHNFLLGQGLIAAAAFN

SEQ ID NO: 414 - protein, 38 aa, Thermosynechococcus elongatus
MKIVGRRLMGWQAVYDIGLAADHNFVLANGAIAAAAFN

SEQ ID NO: 415 - protein, 39 aa, Trichodesmium erythraeum
MVKIVSRKLAKTENVYDIGVTKDHNFVLANGLIASAAFN

SEQ ID NO: 416 - protein, 38 aa, Thermosynechococcus vulcanus
MKIVGRRLVGWQAVYDIGLAGDHNFLLANGAIAAAAFN

SEQ ID NO: 417 - protein, 43 aa, Nostoc punctiforme
  SITE 36: note = X is any amino acid excluding N and/or Q
  SITE 37: note = X is any amino acid excluding C
MIKIATRKYLGKQNVYDIGVERDHNFALKNGFIASXXFNSGGC

SEQ ID NO: 418 - protein, 43 aa, Synechocystis PCC6803
  SITE 36: note = X is any amino acid excluding N and/or Q
  SITE 37: note = X is any amino acid excluding C
MVKVIGRRSLGVQRIFDIGLPQDHNFLLANGAIAAXXFNSGGC

SEQ ID NO: 419 - protein, 43 aa, Aphanothece halophytica
  SITE 36: note = X is any amino acid excluding N and/or Q
  SITE 37: note = X is any amino acid excluding C
MVKIIKRQSLGRQNVYDVCVETDHNFVLANGCVASXXFNSGGC

SEQ ID NO: 420 - protein, 43 aa, Aphanizomenon ovalisporum
  SITE 36: note = X is any amino acid excluding N and/or Q
  SITE 37: note = X is any amino acid excluding C
MVKITARKFVGRENVYDIGVEHHHNFAIKNGLIASXXFNSGGC

SEQ ID NO: 421 - protein, 43 aa, Anabaena PCC7120
  SITE 36: note = X is any amino acid excluding N and/or Q
  SITE 37: note = X is any amino acid excluding C
MIKIASRKFLGVENVYDIGVRRDHNFFIKNGLIASXXFNSGGC

SEQ ID NO: 422 - protein, 43 aa, Anabaena variabilis
  SITE 36: note = X is any amino acid excluding N and/or Q
  SITE 37: note = X is any amino acid excluding C
MIKIASRKFLGVENVYDIGVGRDHNFFVKNGLIASXXFNSGGC

SEQ ID NO: 423 - protein, 43 aa, Cylindrospermopsis raciborskii
  SITE 36: note = X is any amino acid excluding N and/or Q
  SITE 37: note = X is any amino acid excluding C
MVKIVSRRYLGKADVYDIGVAKDHNFIIKNGLVASXXFNSGGC

SEQ ID NO: 424 - protein, 43 aa, Cyanothece CCY0110
  SITE 36: note = X is any amino acid excluding N and/or Q
  SITE 37: note = X is any amino acid excluding C
MVKIIERRSLGKQNVYDIGVEKDHNFLLSNNLIASXXFNSGGC

SEQ ID NO: 425 - protein, 43 aa, Cyanothece PCC8801
  SITE 36: note = X is any amino acid excluding N and/or Q
  SITE 37: note = X is any amino acid excluding C
MVKIVSYRSLGKQFVYDIGVAQDHNFLLANGSIASXXFNSGGC

SEQ ID NO: 426 - protein, 43 aa, Crocosphaera watsonii
  SITE 36: note = X is any amino acid excluding N and/or Q
  SITE 37: note = X is any amino acid excluding C
MVKIIGCRSLGTQKVYDIGVEKDHNFLLANGSIASXXFNSGGC

SEQ ID NO: 427 - protein, 43 aa, Microcystis aeruginosa
  SITE 36: note = X is any amino acid excluding N and/or Q
  SITE 37: note = X is any amino acid excluding C
MVKIIGRQSLGRKPVYDIGVEKDHNFLLGNGLIASXXFNSGGC

SEQ ID NO: 428 - protein, 43 aa, Microcoleus chthonoplastes
  SITE 36: note = X is any amino acid excluding N and/or Q
  SITE 37: note = X is any amino acid excluding C
MVKIVRRQSLGVQNVYDIGVEKDHNFCLASGEIASXXFNSGGC

SEQ ID NO: 429 - protein, 43 aa, Oscillatoria limnetica; identical to SEQ ID NO: 428
  SITE 36: note = X is any amino acid excluding N and/or Q
  SITE 37: note = X is any amino acid excluding C

SEQ ID NO: 430 - protein, 43 aa, Synechococcus elongatus
  SITE 36: note = X is any amino acid excluding N and/or Q
  SITE 37: note = X is any amino acid excluding C
MVKIVRRRSLGVQPVYDLGVATVHNFVLANGLVASXXFNSGGC

SEQ ID NO: 431 - protein, 43 aa, Synechococcus PCC7002
  SITE 36: note = X is any amino acid excluding N and/or Q
  SITE 37: note = X is any amino acid excluding C
MVKIIRRKFIGHAPTYDIGLSQDHNFLLGQGLIAAXXFNSGGC

SEQ ID NO: 432 - protein, 42 aa, Thermosynechococcus elongatus
  SITE 35: note = X is any amino acid excluding N and/or Q
  SITE 36: note = X is any amino acid excluding C
MKIVGRRLMGWQAVYDIGLAADHNFVLANGAIAAXXFNSGGC

SEQ ID NO: 433 - protein, 43 aa, Trichodesmium erythraeum
  SITE 36: note = X is any amino acid excluding N and/or Q
  SITE 37: note = X is any amino acid excluding N
MVKIVSRKLAKTENVYDIGVTKDHNFVLANGLIASXXFNSGGC

SEQ ID NO: 434 - protein, 42 aa, Thermosynechococcus vulcanus
  SITE 35: note = X is any amino acid excluding N and/or Q
  SITE 36: note = X is any amino acid excluding C
MKIVGRRLVGWQAVYDIGLAGDHNFLLANGAIAAXXFNSGGC

SEQ ID NO: 435 - protein, 43 aa, Nostoc punctiforme; identical to SEQ ID NO: 417
  SITE 36: note = X is any amino acid excluding N and/or Q
  SITE 37: note = X is A, V, I, S, M, H, L, F, Y, G or W or can be a unnatural aliphatic amino acid residue such as Nle, Abu, Nva, 2-aminopentoic acid,or 2-aminohexaanoic acid

SEQ ID NO: 436 - protein, 43 aa, Synechocystis PCC6803; identical to SEQ ID NO: 418
  SITE 36: note = X is any amino acid excluding N and/or Q
  SITE 37: note = X is A, V, I, S, M, H, L, F, Y, G or W or can be a unnatural aliphatic amino acid residue such as Nle, Abu, Nva, 2-aminopentoic acid,or 2-aminohexaanoic acid

SEQ ID NO: 437 - protein, 43 aa, Aphanothece halophytica; identical to SEQ ID NO: 419
  SITE 36: note = X is any amino acid excluding N and/or Q
  SITE 37: note = X is A, V, I, S, M, H, L, F, Y, G or W or can be a unnatural aliphatic amino acid residue such as Nle, Abu, Nva, 2-aminopentoic acid,or 2-aminohexaanoic acid

SEQ ID NO: 438 - protein, 43 aa, Aphanizomenon ovalisporum; identical to SEQ ID NO: 420
  SITE 36: note = X is any amino acid excluding N and/or Q
  SITE 37: note = X is A, V, I, S, M, H, L, F, Y, G or W or can be a unnatural aliphatic amino acid residue such as Nle, Abu, Nva, 2-aminopentoic acid,or 2-aminohexaanoic acid

SEQ ID NO: 439 - protein, 43 aa, Anabaena PCC7120; identical to SEQ ID NO: 421
  SITE 36: note = X is any amino acid excluding N and/or Q
  SITE 37: note = X is A, V, I, S, M, H, L, F, Y, G or W or can be a unnatural aliphatic amino acid residue such as Nle, Abu, Nva, 2-aminopentoic acid,or 2-aminohexaanoic acid

SEQ ID NO: 440 - protein, 43 aa, Anabaena variabilis; identical to SEQ ID NO: 422
  SITE 36: note = X is any amino acid excluding N and/or Q
  SITE 37: note = X is A, V, I, S, M, H, L, F, Y, G or W or can be a unnatural aliphatic amino acid residue such as Nle, Abu, Nva, 2-aminopentoic acid,or 2-aminohexaanoic acid

SEQ ID NO: 441 - protein, 43 aa, Cylindrospermopsis raciborskii; identical to SEQ ID NO: 423
  SITE 36: note = X is any amino acid excluding N and/or Q
  SITE 37: note = X is A, V, I, S, M, H, L, F, Y, G or W or can be a unnatural aliphatic amino acid residue such as Nle, Abu, Nva, 2-aminopentoic acid,or 2-aminohexaanoic acid

SEQ ID NO: 442 - protein, 43 aa, Cyanothece CCY0110; identical to SEQ ID NO: 424
  SITE 36: note = X is any amino acid excluding N and/or Q
  SITE 37: note = X is A, V, I, S, M, H, L, F, Y, G or W or can be a unnatural aliphatic amino acid residue such as Nle, Abu, Nva, 2-aminopentoic acid,or 2-aminohexaanoic acid

SEQ ID NO: 443 - protein, 43 aa, Cyanothece PCC8801; identical to SEQ ID NO: 425
  SITE 36: note = X is any amino acid excluding N and/or Q
  SITE 37: note = X is A, V, I, S, M, H, L, F, Y, G or W or can be a unnatural aliphatic amino acid residue such as Nle, Abu, Nva, 2-aminopentoic acid,or 2-aminohexaanoic acid

SEQ ID NO: 444 - protein, 43 aa, Crocosphaera watsonii; identical to SEQ ID NO: 426
  SITE 36: note = X is any amino acid excluding N and/or Q
  SITE 37: note = X is A, V, I, S, M, H, L, F, Y, G or W or can be a unnatural aliphatic amino acid residue such as Nle, Abu, Nva, 2-aminopentoic acid,or 2-aminohexaanoic acid

SEQ ID NO: 445 - protein, 43 aa, Microcystis aeruginosa; identical to SEQ ID NO: 427
  SITE 36: note = X is any amino acid excluding N and/or Q
  SITE 37: note = X is A, V, I, S, M, H, L, F, Y, G or W or can be a unnatural aliphatic amino acid residue such as Nle, Abu, Nva, 2-aminopentoic acid,or 2-aminohexaanoic acid

SEQ ID NO: 446 - protein, 43 aa, Microcoleus chthonoplastes; identical to SEQ ID NO: 428
  SITE 36: note = X is any amino acid excluding N and/or Q
  SITE 37: note = X is A, V, I, S, M, H, L, F, Y, G or W or can be a unnatural aliphatic amino acid residue such as Nle, Abu, Nva, 2-aminopentoic acid,or 2-aminohexaanoic acid

SEQ ID NO: 447 - protein, 43 aa, Oscillatoria limnetica; identical to SEQ ID NO: 428
  SITE 36: note = X is any amino acid excluding N and/or Q
  SITE 37: note = X is A, V, I, S, M, H, L, F, Y, G or W or can be a unnatural aliphatic amino acid residue such as Nle, Abu, Nva, 2-aminopentoic acid,or 2-aminohexaanoic acid

SEQ ID NO: 448 - protein, 43 aa, Synechococcus elongatus; identical to SEQ ID NO: 430
  SITE 36: note = X is any amino acid excluding N and/or Q
  SITE 37: note = X is A, V, I, S, M, H, L, F, Y, G or W or can be a unnatural aliphatic amino acid residue such as Nle, Abu, Nva, 2-aminopentoic acid,or 2-aminohexaanoic acid

SEQ ID NO: 449 - protein, 43 aa, Synechococcus PCC7002; identical to SEQ ID NO: 431
  SITE 36: note = X is any amino acid excluding N and/or Q
  SITE 37: note = X is A, V, I, S, M, H, L, F, Y, G or W or can be a unnatural aliphatic amino acid residue such as Nle, Abu, Nva, 2-aminopentoic acid,or 2-aminohexaanoic acid

SEQ ID NO: 450 - protein, 42 aa, Thermosynechococcus elongatus; identical to SEQ ID NO: 432
  SITE 35: note = X is any amino acid excluding N and/or Q
  SITE 36: note = X is A, V, I, S, M, H, L, F, Y, G or W or can be a unnatural aliphatic amino acid residue such as Nle, Abu, Nva, 2-aminopentoic acid,or 2-aminohexaanoic acid

SEQ ID NO: 451 - protein, 43 aa, Trichodesmium erythraeum; identical to SEQ ID NO: 433
  SITE 36: note = X is any amino acid excluding N and/or Q
  SITE 37: note = X is A, V, I, S, M, H, L, F, Y, G or W or can be a unnatural aliphatic amino acid residue such as Nle, Abu, Nva, 2-aminopentoic acid,or 2-aminohexaanoic acid

SEQ ID NO: 452 - protein, 42 aa, Thermosynechococcus vulcanus; identical to SEQ ID NO: 434
  SITE 35: note = X is any amino acid excluding N and/or Q
  SITE 36: note = X is A, V, I, S, M, H, L, F, Y, G or W or can be a unnatural aliphatic amino acid residue such as Nle, Abu, Nva, 2-aminopentoic acid,or 2-aminohexaanoic acid

SEQ ID NO: 453 - protein, 43 aa, Nostoc punctiforme; identical to SEQ ID NO: 417
  SITE 36: note = X is any amino acid excluding N and/or Q
  SITE 37: note = X is A, I, V, L, Y, G or F

SEQ ID NO: 454 - protein, 43 aa, Synechocystis PCC6803; identical to SEQ ID NO: 418
  SITE 36: note = X is any amino acid excluding N and/or Q
  SITE 37: note = X is A, I, V, L, Y, G or F

SEQ ID NO: 455 - protein, 43 aa, Aphanothece halophytica; identical to SEQ ID NO: 419
  SITE 36: note = X is any amino acid excluding N and/or Q
  SITE 37: note = X is A, I, V, L, Y, G or F

SEQ ID NO: 456 - protein, 43 aa, Aphanizomenon ovalisporum; identical to SEQ ID NO: 420
  SITE 36: note = X is any amino acid excluding N and/or Q
  SITE 37: note = X is A, I, V, L, Y, G or F

SEQ ID NO: 457 - protein, 43 aa, Anabaena PCC7120; identical to SEQ ID NO: 421
  SITE 36: note = X is any amino acid excluding N and/or Q
  SITE 37: note = X is A, I, V, L, Y, G or F

SEQ ID NO: 458 - protein, 43 aa, Anabaena variabilis; identical to SEQ ID NO: 422
  SITE 36: note = X is any amino acid excluding N and/or Q
  SITE 37: note = X is A, I, V, L, Y, G or F

SEQ ID NO: 459 - protein, 43 aa, Cylindrospermopsis raciborskii; identical to SEQ ID NO: 423
  SITE 36: note = X is any amino acid excluding N and/or Q
  SITE 37: note = X is A, I, V, L, Y, G or F

SEQ ID NO: 460 - protein, 43 aa, Cyanothece CCY0110; identical to SEQ ID NO: 424
  SITE 36: note = X is any amino acid excluding N and/or Q
  SITE 37: note = X is A, I, V, L, Y, G or F

SEQ ID NO: 461 - protein, 43 aa, Cyanothece PCC8801; identical to SEQ ID NO: 425
  SITE 36: note = X is any amino acid excluding N and/or Q
  SITE 37: note = X is A, I, V, L, Y, G or F

SEQ ID NO: 462 - protein, 43 aa, Crocosphaera watsonii; identical to SEQ ID NO: 426
  SITE 36: note = X is any amino acid excluding N and/or Q
  SITE 37: note = X is A, I, V, L, Y, G or F

SEQ ID NO: 463 - protein, 43 aa, Microcystis aeruginosa; identical to SEQ ID NO: 427
  SITE 36: note = X is any amino acid excluding N and/or Q
  SITE 37: note = X is A, I, V, L, Y, G or F

SEQ ID NO: 464 - protein, 43 aa, Microcoleus chthonoplastes; identical to SEQ ID NO: 428
  SITE 36: note = X is any amino acid excluding N and/or Q
  SITE 37: note = X is A, I, V, L, Y, G or F

SEQ ID NO: 465 - protein, 43 aa, Oscillatoria limnetica; identical to SEQ ID NO: 428
  SITE 36: note = X is any amino acid excluding N and/or Q
  SITE 37: note = X is A, I, V, L, Y, G or F

SEQ ID NO: 466 - protein, 43 aa, Synechococcus elongatus; identical to SEQ ID NO: 430
  SITE 36: note = X is any amino acid excluding N and/or Q
  SITE 37: note = X is A, I, V, L, Y, G or F

SEQ ID NO: 467 - protein, 43 aa, Synechococcus PCC7002; identical to SEQ ID NO: 431
  SITE 36: note = X is any amino acid excluding N and/or Q
  SITE 37: note = X is A, I, V, L, Y, G or F

SEQ ID NO: 468 - protein, 42 aa, Thermosynechococcus elongatus; identical to SEQ ID NO: 432
  SITE 35: note = X is any amino acid excluding N and/or Q
  SITE 36: note = X is A, I, V, L, Y, G or F

SEQ ID NO: 469 - protein, 43 aa, Trichodesmium erythraeum; identical to SEQ ID NO: 433
  SITE 36: note = X is any amino acid excluding N and/or Q
  SITE 37: note = X is A, I, V, L, Y, G or F

SEQ ID NO: 470 - protein, 42 aa, Thermosynechococcus vulcanus; identical to SEQ ID NO: 434
  SITE 35: note = X is any amino acid excluding N and/or Q
  SITE 36: note = X is A, I, V, L, Y, G or F

SEQ ID NO: 471 - protein, 43 aa, Nostoc punctiforme
  SITE 36: note = X is any amino acid excluding N and/or Q
MIKIATRKYLGKQNVYDIGVERDHNFALKNGFIASXAFNSGGC

SEQ ID NO: 472 - protein, 43 aa, Synechocystis PCC6803
  SITE 36: note = X is any amino acid excluding N and/or Q
MVKVIGRRSLGVQRIFDIGLPQDHNFLLANGAIAAXAFNSGGC

SEQ ID NO: 473 - protein, 43 aa, Aphanothece halophytica
  SITE 36: note = X is any amino acid excluding N and/or Q
MVKIIKRQSLGRQNVYDVCVETDHNFVLANGCVASXAFNSGGC

SEQ ID NO: 474 - protein, 43 aa, Aphanizomenon ovalisporum
  SITE 36: note = X is any amino acid excluding N and/or Q
MVKITARKFVGRENVYDIGVEHHHNFAIKNGLIASXAFNSGGC

SEQ ID NO: 475 - protein, 43 aa, Anabaena PCC7120
  SITE 36: note = X is any amino acid excluding N and/or Q
MIKIASRKFLGVENVYDIGVRRDHNFFIKNGLIASXAFNSGGC

SEQ ID NO: 476 - protein, 43 aa, Anabaena variabilis
  SITE 36: note = X is any amino acid excluding N and/or Q
MIKIASRKFLGVENVYDIGVGRDHNFFVKNGLIASXAFNSGGC

SEQ ID NO: 477 - protein, 43 aa, Cylindrospermopsis raciborskii
  SITE 36: note = X is any amino acid excluding N and/or Q
MVKIVSRRYLGKADVYDIGVAKDHNFIIKNGLVASXAFNSGGC

SEQ ID NO: 478 - protein, 43 aa, Cyanothece CCY0110
  SITE 36: note = X is any amino acid excluding N and/or Q
MVKIIERRSLGKQNVYDIGVEKDHNFLLSNNLIASXAFNSGGC

SEQ ID NO: 479 - protein, 43 aa, Cyanothece PCC8801
  SITE 36: note = X is any amino acid excluding N and/or Q
MVKIVSYRSLGKQFVYDIGVAQDHNFLLANGSIASXAFNSGGC

SEQ ID NO: 480 - protein, 43 aa, Crocosphaera watsonii
  SITE 36: note = X is any amino acid excluding N and/or Q
MVKIIGCRSLGTQKVYDIGVEKDHNFLLANGSIASXAFNSGGC

SEQ ID NO: 481 - protein, 43 aa, Microcystis aeruginosa
  SITE 36: note = X is any amino acid excluding N and/or Q
MVKIIGRQSLGRKPVYDIGVEKDHNFLLGNGLIASXAFNSGGC

SEQ ID NO: 482 - protein, 43 aa, Microcoleus chthonoplastes
  SITE 36: note = X is any amino acid excluding N and/or Q
MVKIVRRQSLGVQNVYDIGVEKDHNFCLASGEIASXAFNSGGC

SEQ ID NO: 483 - protein, 43 aa, Oscillatoria limnetica; identical to SEQ ID NO: 482
  SITE 36: note = X is any amino acid excluding N and/or Q

SEQ ID NO: 484 - protein, 43 aa, Synechococcus elongatus
  SITE 36: note = X is any amino acid excluding N and/or Q
MVKIVRRRSLGVQPVYDLGVATVHNFVLANGLVASXAFNSGGC

SEQ ID NO: 485 - protein, 43 aa, Synechococcus PCC7002
  SITE 36: note = X is any amino acid excluding N and/or Q
MVKIIRRKFIGHAPTYDIGLSQDHNFLLGQGLIAAXAFNSGGC

SEQ ID NO: 486 - protein, 42 aa, Thermosynechococcus elongatus
  SITE 35: note = X is any amino acid excluding N and/or Q
MKIVGRRLMGWQAVYDIGLAADHNFVLANGAIAAXAFNSGGC

SEQ ID NO: 487 - protein, 43 aa, Trichodesmium erythraeum
  SITE 36: note = X is any amino acid excluding N and/or Q
MVKIVSRKLAKTENVYDIGVTKDHNFVLANGLIASXAFNSGGC

SEQ ID NO: 488 - protein, 42 aa, Thermosynechococcus vulcanus
  SITE 35: note = X is any amino acid excluding N and/or Q
MKIVGRRLVGWQAVYDIGLAGDHNFLLANGAIAAXAFNSGGC

SEQ ID NO: 489 - protein, 43 aa, Nostoc punctiforme; identical to SEQ ID NO: 417
  SITE 36: note = X is A, V, I, S, M, H, L, F, Y, G or W or can be a unnatural aliphatic amino acid residue such as Nle, Abu, Nva, 2-aminopentoic acid,or 2-aminohexaanoic acid
  SITE 37: note = X is any amino acid excluding C

SEQ ID NO: 490 - protein, 43 aa, Synechocystis PCC6803; identical to SEQ ID NO: 418
  SITE 36: note = X is A, V, I, S, M, H, L, F, Y, G or W or can be a unnatural aliphatic amino acid residue such as Nle, Abu, Nva, 2-aminopentoic acid,or 2-aminohexaanoic acid
  SITE 37: note = X is any amino acid excluding C

SEQ ID NO: 491 - protein, 43 aa, Aphanothece halophytica; identical to SEQ ID NO: 419
  SITE 36: note = X is A, V, I, S, M, H, L, F, Y, G or W or can be a unnatural aliphatic amino acid residue such as Nle, Abu, Nva, 2-aminopentoic acid,or 2-aminohexaanoic acid
  SITE 37: note = X is any amino acid excluding C

SEQ ID NO: 492 - protein, 43 aa, Aphanizomenon ovalisporum; identical to SEQ ID NO: 420
  SITE 36: note = X is A, V, I, S, M, H, L, F, Y, G or W or can be a unnatural aliphatic amino acid residue such as Nle, Abu, Nva, 2-aminopentoic acid,or 2-aminohexaanoic acid
  SITE 37: note = X is any amino acid excluding C

SEQ ID NO: 493 - protein, 43 aa, Anabaena PCC7120; identical to SEQ ID NO: 421
  SITE 36: note = X is A, V, I, S, M, H, L, F, Y, G or W or can be a unnatural aliphatic amino acid residue such as Nle, Abu, Nva, 2-aminopentoic acid,or 2-aminohexaanoic acid
  SITE 37: note = X is any amino acid excluding C

SEQ ID NO: 494 - protein, 43 aa, Anabaena variabilis; identical to SEQ ID NO: 422
  SITE 36: note = X is A, V, I, S, M, H, L, F, Y, G or W or can be a unnatural aliphatic amino acid residue such as Nle, Abu, Nva, 2-aminopentoic acid,or 2-aminohexaanoic acid
  SITE 37: note = X is any amino acid excluding C

SEQ ID NO: 495 - protein, 43 aa, Cylindrospermopsis raciborskii; identical to SEQ ID NO: 423
  SITE 36: note = X is A, V, I, S, M, H, L, F, Y, G or W or can be a unnatural aliphatic amino acid residue such as Nle, Abu, Nva, 2-aminopentoic acid,or 2-aminohexaanoic acid
  SITE 37: note = X is any amino acid excluding C

SEQ ID NO: 496 - protein, 43 aa, Cyanothece CCY0110; identical to SEQ ID NO: 424
  SITE 36: note = X is A, V, I, S, M, H, L, F, Y, G or W or can be a unnatural aliphatic amino acid residue such as Nle, Abu, Nva, 2-aminopentoic acid,or 2-aminohexaanoic acid
  SITE 37: note = X is any amino acid excluding C

SEQ ID NO: 497 - protein, 43 aa, Cyanothece PCC8801; identical to SEQ ID NO: 425
  SITE 36: note = X is A, V, I, S, M, H, L, F, Y, G or W or can be a unnatural aliphatic amino acid residue such as Nle, Abu, Nva, 2-aminopentoic acid,or 2-aminohexaanoic acid
  SITE 37: note = X is any amino acid excluding C

SEQ ID NO: 498 - protein, 43 aa, Crocosphaera watsonii; identical to SEQ ID NO: 426
  SITE 36: note = X is A, V, I, S, M, H, L, F, Y, G or W or can be a unnatural aliphatic amino acid residue such as Nle, Abu, Nva, 2-aminopentoic acid,or 2-aminohexaanoic acid
  SITE 37: note = X is any amino acid excluding C

SEQ ID NO: 499 - protein, 43 aa, Microcystis aeruginosa; identical to SEQ ID NO: 427
  SITE 36: note = X is A, V, I, S, M, H, L, F, Y, G or W or can be a unnatural aliphatic amino acid residue such as Nle, Abu, Nva, 2-aminopentoic acid,or 2-aminohexaanoic acid
  SITE 37: note = X is any amino acid excluding C

SEQ ID NO: 500 - protein, 43 aa, Microcoleus chthonoplastes; identical to SEQ ID NO: 428
  SITE 36: note = X is A, V, I, S, M, H, L, F, Y, G or W or can be a unnatural aliphatic amino acid residue such as Nle, Abu, Nva, 2-aminopentoic acid,or 2-aminohexaanoic acid
  SITE 37: note = X is any amino acid excluding C

SEQ ID NO: 501 - protein, 43 aa, Oscillatoria limnetica; identical to SEQ ID NO: 428
  SITE 36: note = X is A, V, I, S, M, H, L, F, Y, G or W or can be a unnatural aliphatic amino acid residue such as Nle, Abu, Nva, 2-aminopentoic acid,or 2-aminohexaanoic acid
  SITE 37: note = X is any amino acid excluding C

SEQ ID NO: 502 - protein, 43 aa, Synechococcus elongatus; identical to SEQ ID NO: 430
  SITE 36: note = X is A, V, I, S, M, H, L, F, Y, G or W or can be a unnatural aliphatic amino acid residue such as Nle, Abu, Nva, 2-aminopentoic acid,or 2-aminohexaanoic acid
  SITE 37: note = X is any amino acid excluding C

SEQ ID NO: 503 - protein, 43 aa, Synechococcus PCC7002; identical to SEQ ID NO: 431
  SITE 36: note = X is A, V, I, S, M, H, L, F, Y, G or W or can be a unnatural aliphatic amino acid residue such as Nle, Abu, Nva, 2-aminopentoic acid,or 2-aminohexaanoic acid
  SITE 37: note = X is any amino acid excluding C

SEQ ID NO: 504 - protein, 42 aa, Thermosynechococcus elongatus; identical to SEQ ID NO: 432
  SITE 35: note = X is A, V, I, S, M, H, L, F, Y, G or W or can be a unnatural aliphatic amino acid residue such as Nle, Abu, Nva, 2-aminopentoic acid,or 2-aminohexaanoic acid
  SITE 36: note = X is any amino acid excluding C

SEQ ID NO: 505 - protein, 43 aa, Trichodesmium erythraeum; identical to SEQ ID NO: 433
  SITE 36: note = X is A, V, I, S, M, H, L, F, Y, G or W or can be a unnatural aliphatic amino acid residue such as Nle, Abu, Nva, 2-aminopentoic acid,or 2-aminohexaanoic acid
  SITE 37: note = X is any amino acid excluding N

SEQ ID NO: 506 - protein, 42 aa, Thermosynechococcus vulcanus; identical to SEQ ID NO: 434
  SITE 35: note = X is A, V, I, S, M, H, L, F, Y, G or W or can be a unnatural aliphatic amino acid residue such as Nle, Abu, Nva, 2-aminopentoic acid,or 2-aminohexaanoic acid
  SITE 36: note = X is any amino acid excluding C

SEQ ID NO: 507 - protein, 43 aa, Nostoc punctiforme; identical to SEQ ID NO: 417
  SITE 36: note = X is A, V, I, S, M, H, L, F, Y, G or W or can be a unnatural aliphatic amino acid residue such as Nle, Abu, Nva, 2-aminopentoic acid,or 2-aminohexaanoic acid
  SITE 37: note = X is A, V, I, S, M, H, L, F, Y, G or W or can be a unnatural aliphatic amino acid residue such as Nle, Abu, Nva, 2-aminopentoic acid,or 2-aminohexaanoic acid

SEQ ID NO: 508 - protein, 43 aa, Synechocystis PCC6803; identical to SEQ ID NO: 418
  SITE 36: note = X is A, V, I, S, M, H, L, F, Y, G or W or can be a unnatural aliphatic amino acid residue such as Nle, Abu, Nva, 2-aminopentoic acid,or 2-aminohexaanoic acid
  SITE 37: note = X is A, V, I, S, M, H, L, F, Y, G or W or can be a unnatural aliphatic amino acid residue such as Nle, Abu, Nva, 2-aminopentoic acid,or 2-aminohexaanoic acid

SEQ ID NO: 509 - protein, 43 aa, Aphanothece halophytica; identical to SEQ ID NO: 419
  SITE 36: note = X is A, V, I, S, M, H, L, F, Y, G or W or can be a unnatural aliphatic amino acid residue such as Nle, Abu, Nva, 2-aminopentoic acid,or 2-aminohexaanoic acid
  SITE 37: note = X is A, V, I, S, M, H, L, F, Y, G or W or can be a unnatural aliphatic amino acid residue such as Nle, Abu, Nva, 2-aminopentoic acid,or 2-aminohexaanoic acid

SEQ ID NO: 510 - protein, 43 aa, Aphanizomenon ovalisporum; identical to SEQ ID NO: 420
  SITE 36: note = X is A, V, I, S, M, H, L, F, Y, G or W or can be a unnatural aliphatic amino acid residue such as Nle, Abu, Nva, 2-aminopentoic acid,or 2-aminohexaanoic acid
  SITE 37: note = X is A, V, I, S, M, H, L, F, Y, G or W or can be a unnatural aliphatic amino acid residue such as Nle, Abu, Nva, 2-aminopentoic acid,or 2-aminohexaanoic acid

SEQ ID NO: 511 - protein, 43 aa, Anabaena PCC7120; identical to SEQ ID NO: 421
  SITE 36: note = X is A, V, I, S, M, H, L, F, Y, G or W or can be a unnatural aliphatic amino acid residue such as Nle, Abu, Nva, 2-aminopentoic acid,or 2-aminohexaanoic acid
  SITE 37: note = X is A, V, I, S, M, H, L, F, Y, G or W or can be a unnatural aliphatic amino acid residue such as Nle, Abu, Nva, 2-aminopentoic acid,or 2-aminohexaanoic acid

SEQ ID NO: 512 - protein, 43 aa, Anabaena variabilis; identical to SEQ ID NO: 422
  SITE 36: note = X is A, V, I, S, M, H, L, F, Y, G or W or can be a unnatural aliphatic amino acid residue such as Nle, Abu, Nva, 2-aminopentoic acid,or 2-aminohexaanoic acid
  SITE 37: note = X is A, V, I, S, M, H, L, F, Y, G or W or can be a unnatural aliphatic amino acid residue such as Nle, Abu, Nva, 2-aminopentoic acid,or 2-aminohexaanoic acid

SEQ ID NO: 513 - protein, 43 aa, Cylindrospermopsis raciborskii; identical to SEQ ID NO: 423
  SITE 36: note = X is A, V, I, S, M, H, L, F, Y, G or W or can be a unnatural aliphatic amino acid residue such as Nle, Abu, Nva, 2-aminopentoic acid,or 2-aminohexaanoic acid
  SITE 37: note = X is A, V, I, S, M, H, L, F, Y, G or W or can be a unnatural aliphatic amino acid residue such as Nle, Abu, Nva, 2-aminopentoic acid,or 2-aminohexaanoic acid

SEQ ID NO: 514 - protein, 43 aa, Cyanothece CCY0110; identical to SEQ ID NO: 424
  SITE 36: note = X is A, V, I, S, M, H, L, F, Y, G or W or can be a unnatural aliphatic amino acid residue such as Nle, Abu, Nva, 2-aminopentoic acid,or 2-aminohexaanoic acid
  SITE 37: note = X is A, V, I, S, M, H, L, F, Y, G or W or can be a unnatural aliphatic amino acid residue such as Nle, Abu, Nva, 2-aminopentoic acid,or 2-aminohexaanoic acid

SEQ ID NO: 515 - protein, 43 aa, Cyanothece PCC8801; identical to SEQ ID NO: 425
  SITE 36: note = X is A, V, I, S, M, H, L, F, Y, G or W or can be a unnatural aliphatic amino acid residue such as Nle, Abu, Nva, 2-aminopentoic acid,or 2-aminohexaanoic acid
  SITE 37: note = X is A, V, I, S, M, H, L, F, Y, G or W or can be a unnatural aliphatic amino acid residue such as Nle, Abu, Nva, 2-aminopentoic acid,or 2-aminohexaanoic acid

SEQ ID NO: 516 - protein, 43 aa, Crocosphaera watsonii; identical to SEQ ID NO: 426
  SITE 36: note = X is A, V, I, S, M, H, L, F, Y, G or W or can be a unnatural aliphatic amino acid residue such as Nle, Abu, Nva, 2-aminopentoic acid,or 2-aminohexaanoic acid
  SITE 37: note = X is A, V, I, S, M, H, L, F, Y, G or W or can be a unnatural aliphatic amino acid residue such as Nle, Abu, Nva, 2-aminopentoic acid,or 2-aminohexaanoic acid

SEQ ID NO: 517 - protein, 43 aa, Microcystis aeruginosa; identical to SEQ ID NO: 427
  SITE 36: note = X is A, V, I, S, M, H, L, F, Y, G or W or can be a unnatural aliphatic amino acid residue such as Nle, Abu, Nva, 2-aminopentoic acid,or 2-aminohexaanoic acid
  SITE 37: note = X is A, V, I, S, M, H, L, F, Y, G or W or can be a unnatural aliphatic amino acid residue such as Nle, Abu, Nva, 2-aminopentoic acid,or 2-aminohexaanoic acid

SEQ ID NO: 518 - protein, 43 aa, Microcoleus chthonoplastes; identical to SEQ ID NO: 428
  SITE 36: note = X is A, V, I, S, M, H, L, F, Y, G or W or can be a unnatural aliphatic amino acid residue such as Nle, Abu, Nva, 2-aminopentoic acid,or 2-aminohexaanoic acid
  SITE 37: note = X is A, V, I, S, M, H, L, F, Y, G or W or can be a unnatural aliphatic amino acid residue such as Nle, Abu, Nva, 2-aminopentoic acid,or 2-aminohexaanoic acid

SEQ ID NO: 519 - protein, 43 aa, Oscillatoria limnetica; identical to SEQ ID NO: 428
  SITE 36: note = X is A, V, I, S, M, H, L, F, Y, G or W or can be a unnatural aliphatic amino acid residue such as Nle, Abu, Nva, 2-aminopentoic acid,or 2-aminohexaanoic acid
  SITE 37: note = X is A, V, I, S, M, H, L, F, Y, G or W or can be a unnatural aliphatic amino acid residue such as Nle, Abu, Nva, 2-aminopentoic acid,or 2-aminohexaanoic acid

SEQ ID NO: 520 - protein, 43 aa, Synechococcus elongatus; identical to SEQ ID NO: 430
  SITE 36: note = X is A, V, I, S, M, H, L, F, Y, G or W or can be a unnatural aliphatic amino acid residue such as Nle, Abu, Nva, 2-aminopentoic acid,or 2-aminohexaanoic acid
  SITE 37: note = X is A, V, I, S, M, H, L, F, Y, G or W or can be a unnatural aliphatic amino acid residue such as Nle, Abu, Nva, 2-aminopentoic acid,or 2-aminohexaanoic acid

SEQ ID NO: 521 - protein, 43 aa, Synechococcus PCC7002; identical to SEQ ID NO: 431
  SITE 36: note = X is A, V, I, S, M, H, L, F, Y, G or W or can be a unnatural aliphatic amino acid residue such as Nle, Abu, Nva, 2-aminopentoic acid,or 2-aminohexaanoic acid
  SITE 37: note = X is A, V, I, S, M, H, L, F, Y, G or W or can be a unnatural aliphatic amino acid residue such as Nle, Abu, Nva, 2-aminopentoic acid,or 2-aminohexaanoic acid

SEQ ID NO: 522 - protein, 42 aa, Thermosynechococcus elongatus; identical to SEQ ID NO: 432
  SITE 35: note = X is A, V, I, S, M, H, L, F, Y, G or W or can be a unnatural aliphatic amino acid residue such as Nle, Abu, Nva, 2-aminopentoic acid,or 2-aminohexaanoic acid
  SITE 36: note = X is A, V, I, S, M, H, L, F, Y, G or W or can be a unnatural aliphatic amino acid residue such as Nle, Abu, Nva, 2-aminopentoic acid,or 2-aminohexaanoic acid

SEQ ID NO: 523 - protein, 43 aa, Trichodesmium erythraeum; identical to SEQ ID NO: 433
  SITE 36: note = X is A, V, I, S, M, H, L, F, Y, G or W or can be a unnatural aliphatic amino acid residue such as Nle, Abu, Nva, 2-aminopentoic acid,or 2-aminohexaanoic acid
  SITE 37: note = X is A, V, I, S, M, H, L, F, Y, G or W or can be a unnatural aliphatic amino acid residue such as Nle, Abu, Nva, 2-aminopentoic acid,or 2-aminohexaanoic acid

SEQ ID NO: 524 - protein, 42 aa, Thermosynechococcus vulcanus; identical to SEQ ID NO: 434
  SITE 35: note = X is A, V, I, S, M, H, L, F, Y, G or W or can be a unnatural aliphatic amino acid residue such as Nle, Abu, Nva, 2-aminopentoic acid,or 2-aminohexaanoic acid
  SITE 36: note = X is A, V, I, S, M, H, L, F, Y, G or W or can be a unnatural aliphatic amino acid residue such as Nle, Abu, Nva, 2-aminopentoic acid,or 2-aminohexaanoic acid

SEQ ID NO: 525 - protein, 43 aa, Nostoc punctiforme; identical to SEQ ID NO: 417
  SITE 36: note = X is A, V, I, S, M, H, L, F, Y, G or W or can be a unnatural aliphatic amino acid residue such as Nle, Abu, Nva, 2-aminopentoic acid,or 2-aminohexaanoic acid
  SITE 37: note = X is A, I, V, L, Y, G or F

SEQ ID NO: 526 - protein, 43 aa, Synechocystis PCC6803; identical to SEQ ID NO: 418
  SITE 36: note = X is A, V, I, S, M, H, L, F, Y, G or W or can be a unnatural aliphatic amino acid residue such as Nle, Abu, Nva, 2-aminopentoic acid,or 2-aminohexaanoic acid
  SITE 37: note = X is A, I, V, L, Y, G or F

SEQ ID NO: 527 - protein, 43 aa, Aphanothece halophytica; identical to SEQ ID NO: 419
  SITE 36: note = X is A, V, I, S, M, H, L, F, Y, G or W or can be a unnatural aliphatic amino acid residue such as Nle, Abu, Nva, 2-aminopentoic acid,or 2-aminohexaanoic acid
  SITE 37: note = X is A, I, V, L, Y, G or F

SEQ ID NO: 528 - protein, 43 aa, Aphanizomenon ovalisporum; identical to SEQ ID NO: 420
  SITE 36: note = X is A, V, I, S, M, H, L, F, Y, G or W or can be a unnatural aliphatic amino acid residue such as Nle, Abu, Nva, 2-aminopentoic acid,or 2-aminohexaanoic acid
  SITE 37: note = X is A, I, V, L, Y, G or F

SEQ ID NO: 529 - protein, 43 aa, Anabaena PCC7120; identical to SEQ ID NO: 421
  SITE 36: note = X is A, V, I, S, M, H, L, F, Y, G or W or can be a unnatural aliphatic amino acid residue such as Nle, Abu, Nva, 2-aminopentoic acid,or 2-aminohexaanoic acid
  SITE 37: note = X is A, I, V, L, Y, G or F

SEQ ID NO: 530 - protein, 43 aa, Anabaena variabilis; identical to SEQ ID NO: 422
  SITE 36: note = X is A, V, I, S, M, H, L, F, Y, G or W or can be a unnatural aliphatic amino acid residue such as Nle, Abu, Nva, 2-aminopentoic acid,or 2-aminohexaanoic acid
  SITE 37: note = X is A, I, V, L, Y, G or F

SEQ ID NO: 531 - protein, 43 aa, Cylindrospermopsis raciborskii; identical to SEQ ID NO: 423
  SITE 36: note = X is A, V, I, S, M, H, L, F, Y, G or W or can be a unnatural aliphatic amino acid residue such as Nle, Abu, Nva, 2-aminopentoic acid,or 2-aminohexaanoic acid
  SITE 37: note = X is A, I, V, L, Y, G or F

SEQ ID NO: 532 - protein, 43 aa, Cyanothece CCY0110; identical to SEQ ID NO: 424
  SITE 36: note = X is A, V, I, S, M, H, L, F, Y, G or W or can be a unnatural aliphatic amino acid residue such as Nle, Abu, Nva, 2-aminopentoic acid,or 2-aminohexaanoic acid
  SITE 37: note = X is A, I, V, L, Y, G or F

SEQ ID NO: 533 - protein, 43 aa, Cyanothece PCC8801; identical to SEQ ID NO: 425
  SITE 36: note = X is A, V, I, S, M, H, L, F, Y, G or W or can be a unnatural aliphatic amino acid residue such as Nle, Abu, Nva, 2-aminopentoic acid,or 2-aminohexaanoic acid
  SITE 37: note = X is A, I, V, L, Y, G or F

SEQ ID NO: 534 - protein, 43 aa, Crocosphaera watsonii; identical to SEQ ID NO: 426
  SITE 36: note = X is A, V, I, S, M, H, L, F, Y, G or W or can be a unnatural aliphatic amino acid residue such as Nle, Abu, Nva, 2-aminopentoic acid,or 2-aminohexaanoic acid
  SITE 37: note = X is A, I, V, L, Y, G or F

SEQ ID NO: 535 - protein, 43 aa, Microcystis aeruginosa; identical to SEQ ID NO: 427
  SITE 36: note = X is A, V, I, S, M, H, L, F, Y, G or W or can be a unnatural aliphatic amino acid residue such as Nle, Abu, Nva, 2-aminopentoic acid,or 2-aminohexaanoic acid
  SITE 37: note = X is A, I, V, L, Y, G or F

SEQ ID NO: 536 - protein, 43 aa, Microcoleus chthonoplastes; identical to SEQ ID NO: 428
  SITE 36: note = X is A, V, I, S, M, H, L, F, Y, G or W or can be a unnatural aliphatic amino acid residue such as Nle, Abu, Nva, 2-aminopentoic acid,or 2-aminohexaanoic acid
  SITE 37: note = X is A, I, V, L, Y, G or F

SEQ ID NO: 537 - protein, 43 aa, Oscillatoria limnetica; identical to SEQ ID NO: 428
  SITE 36: note = X is A, V, I, S, M, H, L, F, Y, G or W or can be a unnatural aliphatic amino acid residue such as Nle, Abu, Nva, 2-aminopentoic acid,or 2-aminohexaanoic acid
  SITE 37: note = X is A, I, V, L, Y, G or F

SEQ ID NO: 538 - protein, 43 aa, Synechococcus elongatus; identical to SEQ ID NO: 430
  SITE 36: note = X is A, V, I, S, M, H, L, F, Y, G or W or can be a unnatural aliphatic amino acid residue such as Nle, Abu, Nva, 2-aminopentoic acid,or 2-aminohexaanoic acid
  SITE 37: note = X is A, I, V, L, Y, G or F

SEQ ID NO: 539 - protein, 43 aa, Synechococcus PCC7002; identical to SEQ ID NO: 431
  SITE 36: note = X is A, V, I, S, M, H, L, F, Y, G or W or can be a unnatural aliphatic amino acid residue such as Nle, Abu, Nva, 2-aminopentoic acid,or 2-aminohexaanoic acid
  SITE 37: note = X is A, I, V, L, Y, G or F

SEQ ID NO: 540 - protein, 42 aa, Thermosynechococcus elongatus; identical to SEQ ID NO: 432
  SITE 35: note = X is A, V, I, S, M, H, L, F, Y, G or W or can be a unnatural aliphatic amino acid residue such as Nle, Abu, Nva, 2-aminopentoic acid,or 2-aminohexaanoic acid
  SITE 36: note = X is A, I, V, L, Y, G or F

SEQ ID NO: 541 - protein, 43 aa, Trichodesmium erythraeum; identical to SEQ ID NO: 433
  SITE 36: note = X is A, V, I, S, M, H, L, F, Y, G or W or can be a unnatural aliphatic amino acid residue such as Nle, Abu, Nva, 2-aminopentoic acid,or 2-aminohexaanoic acid
  SITE 37: note = X is A, I, V, L, Y, G or F

SEQ ID NO: 542 - protein, 42 aa, Thermosynechococcus vulcanus; identical to SEQ ID NO: 434
  SITE 35: note = X is A, V, I, S, M, H, L, F, Y, G or W or can be a unnatural aliphatic amino acid residue such as Nle, Abu, Nva, 2-aminopentoic acid,or 2-aminohexaanoic acid
  SITE 36: note = X is A, I, V, L, Y, G or F

SEQ ID NO: 543 - protein, 43 aa, Nostoc punctiforme; identical to SEQ ID NO: 471
  SITE 36: note = X is A, V, I, S, M, H, L, F, Y, G or W or can be a unnatural aliphatic amino acid residue such as Nle, Abu, Nva, 2-aminopentoic acid,or 2-aminohexaanoic acid

SEQ ID NO: 544 - protein, 43 aa, Synechocystis PCC6803; identical to SEQ ID NO: 472
  SITE 36: note = X is A, V, I, S, M, H, L, F, Y, G or W or can be a unnatural aliphatic amino acid residue such as Nle, Abu, Nva, 2-aminopentoic acid,or 2-aminohexaanoic acid

SEQ ID NO: 545 - protein, 43 aa, Aphanothece halophytica; identical to SEQ ID NO: 473
  SITE 36: note = X is A, V, I, S, M, H, L, F, Y, G or W or can be a unnatural aliphatic amino acid residue such as Nle, Abu, Nva, 2-aminopentoic acid,or 2-aminohexaanoic acid

SEQ ID NO: 546 - protein, 43 aa, Aphanizomenon ovalisporum; identical to SEQ ID NO: 474
  SITE 36: note = X is A, V, I, S, M, H, L, F, Y, G or W or can be a unnatural aliphatic amino acid residue such as Nle, Abu, Nva, 2-aminopentoic acid,or 2-aminohexaanoic acid

SEQ ID NO: 547 - protein, 43 aa, Anabaena PCC7120; identical to SEQ ID NO: 475
  SITE 36: note = X is A, V, I, S, M, H, L, F, Y, G or W or can be a unnatural aliphatic amino acid residue such as Nle, Abu, Nva, 2-aminopentoic acid,or 2-aminohexaanoic acid

SEQ ID NO: 548 - protein, 43 aa, Anabaena variabilis; identical to SEQ ID NO: 476
  SITE 36: note = X is A, V, I, S, M, H, L, F, Y, G or W or can be a unnatural aliphatic amino acid residue such as Nle, Abu, Nva, 2-aminopentoic acid,or 2-aminohexaanoic acid

SEQ ID NO: 549 - protein, 43 aa, Cylindrospermopsis raciborskii; identical to SEQ ID NO: 477
  SITE 36: note = X is A, V, I, S, M, H, L, F, Y, G or W or can be a unnatural aliphatic amino acid residue such as Nle, Abu, Nva, 2-aminopentoic acid,or 2-aminohexaanoic acid

SEQ ID NO: 550 - protein, 43 aa, Cyanothece CCY0110; identical to SEQ ID NO: 478
  SITE 36: note = X is A, V, I, S, M, H, L, F, Y, G or W or can be a unnatural aliphatic amino acid residue such as Nle, Abu, Nva, 2-aminopentoic acid,or 2-aminohexaanoic acid

SEQ ID NO: 551 - protein, 43 aa, Cyanothece PCC8801; identical to SEQ ID NO: 479
  SITE 36: note = X is A, V, I, S, M, H, L, F, Y, G or W or can be a unnatural aliphatic amino acid residue such as Nle, Abu, Nva, 2-aminopentoic acid,or 2-aminohexaanoic acid

SEQ ID NO: 552 - protein, 43 aa, Crocosphaera watsonii; identical to SEQ ID NO: 480
  SITE 36: note = X is A, V, I, S, M, H, L, F, Y, G or W or can be a unnatural aliphatic amino acid residue such as Nle, Abu, Nva, 2-aminopentoic acid,or 2-aminohexaanoic acid

SEQ ID NO: 553 - protein, 43 aa, Microcystis aeruginosa; identical to SEQ ID NO: 481
  SITE 36: note = X is A, V, I, S, M, H, L, F, Y, G or W or can be a unnatural aliphatic amino acid residue such as Nle, Abu, Nva, 2-aminopentoic acid,or 2-aminohexaanoic acid

SEQ ID NO: 554 - protein, 43 aa, Microcoleus chthonoplastes; identical to SEQ ID NO: 482
  SITE 36: note = X is A, V, I, S, M, H, L, F, Y, G or W or can be a unnatural aliphatic amino acid residue such as Nle, Abu, Nva, 2-aminopentoic acid,or 2-aminohexaanoic acid

SEQ ID NO: 555 - protein, 43 aa, Oscillatoria limnetica; identical to SEQ ID NO: 482
  SITE 36: note = X is A, V, I, S, M, H, L, F, Y, G or W or can be a unnatural aliphatic amino acid residue such as Nle, Abu, Nva, 2-aminopentoic acid,or 2-aminohexaanoic acid

SEQ ID NO: 556 - protein, 43 aa, Synechococcus elongatus; identical to SEQ ID NO: 484
  SITE 36: note = X is A, V, I, S, M, H, L, F, Y, G or W or can be a unnatural aliphatic amino acid residue such as Nle, Abu, Nva, 2-aminopentoic acid,or 2-aminohexaanoic acid

SEQ ID NO: 557 - protein, 43 aa, Synechococcus PCC7002; identical to SEQ ID NO: 485
  SITE 36: note = X is A, V, I, S, M, H, L, F, Y, G or W or can be a unnatural aliphatic amino acid residue such as Nle, Abu, Nva, 2-aminopentoic acid,or 2-aminohexaanoic acid

SEQ ID NO: 558 - protein, 42 aa, Thermosynechococcus elongatus; identical to SEQ ID NO: 486
  SITE 35: note = X is A, V, I, S, M, H, L, F, Y, G or W or can be a unnatural aliphatic amino acid residue such as Nle, Abu, Nva, 2-aminopentoic acid,or 2-aminohexaanoic acid

SEQ ID NO: 559 - protein, 43 aa, Trichodesmium erythraeum; identical to SEQ ID NO: 487
  SITE 36: note = X is A, V, I, S, M, H, L, F, Y, G or W or can be a unnatural aliphatic amino acid residue such as Nle, Abu, Nva, 2-aminopentoic acid,or 2-aminohexaanoic acid

SEQ ID NO: 560 - protein, 42 aa, Thermosynechococcus vulcanus; identical to SEQ ID NO: 488
  SITE 35: note = X is A, V, I, S, M, H, L, F, Y, G or W or can be a unnatural aliphatic amino acid residue such as Nle, Abu, Nva, 2-aminopentoic acid,or 2-aminohexaanoic acid

SEQ ID NO: 561 - protein, 43 aa, Nostoc punctiforme; identical to SEQ ID NO: 417
  SITE 36: note = X is A, I, V, L, Y, G or F
  SITE 37: note = X is any amino acid excluding C

SEQ ID NO: 562 - protein, 43 aa, Synechocystis PCC6803; identical to SEQ ID NO: 418
  SITE 36: note = X is A, I, V, L, Y, G or F
  SITE 37: note = X is any amino acid excluding C

SEQ ID NO: 563 - protein, 43 aa, Aphanothece halophytica; identical to SEQ ID NO: 419
  SITE 36: note = X is A, I, V, L, Y, G or F
  SITE 37: note = X is any amino acid excluding C

SEQ ID NO: 564 - protein, 43 aa, Aphanizomenon ovalisporum; identical to SEQ ID NO: 420
  SITE 36: note = X is A, I, V, L, Y, G or F
  SITE 37: note = X is any amino acid excluding C

SEQ ID NO: 565 - protein, 43 aa, Anabaena PCC7120; identical to SEQ ID NO: 421
  SITE 36: note = X is A, I, V, L, Y, G or F
  SITE 37: note = X is any amino acid excluding C

SEQ ID NO: 566 - protein, 43 aa, Anabaena variabilis; identical to SEQ ID NO: 422
  SITE 36: note = X is A, I, V, L, Y, G or F
  SITE 37: note = X is any amino acid excluding C

SEQ ID NO: 567 - protein, 43 aa, Cylindrospermopsis raciborskii; identical to SEQ ID NO: 423
  SITE 36: note = X is A, I, V, L, Y, G or F
  SITE 37: note = X is any amino acid excluding C

SEQ ID NO: 568 - protein, 43 aa, Cyanothece CCY0110; identical to SEQ ID NO: 424
  SITE 36: note = X is A, I, V, L, Y, G or F
  SITE 37: note = X is any amino acid excluding C

SEQ ID NO: 569 - protein, 43 aa, Cyanothece PCC8801; identical to SEQ ID NO: 425
  SITE 36: note = X is A, I, V, L, Y, G or F
  SITE 37: note = X is any amino acid excluding C

SEQ ID NO: 570 - protein, 43 aa, Crocosphaera watsonii; identical to SEQ ID NO: 426
  SITE 36: note = X is A, I, V, L, Y, G or F
  SITE 37: note = X is any amino acid excluding C

SEQ ID NO: 571 - protein, 43 aa, Microcystis aeruginosa; identical to SEQ ID NO: 427
  SITE 36: note = X is A, I, V, L, Y, G or F
  SITE 37: note = X is any amino acid excluding C

SEQ ID NO: 572 - protein, 43 aa, Microcoleus chthonoplastes; identical to SEQ ID NO: 428
  SITE 36: note = X is A, I, V, L, Y, G or F
  SITE 37: note = X is any amino acid excluding C

SEQ ID NO: 573 - protein, 43 aa, Oscillatoria limnetica; identical to SEQ ID NO: 428
  SITE 36: note = X is A, I, V, L, Y, G or F
  SITE 37: note = X is any amino acid excluding C

SEQ ID NO: 574 - protein, 43 aa, Synechococcus elongatus; identical to SEQ ID NO: 430
  SITE 36: note = X is A, I, V, L, Y, G or F
  SITE 37: note = X is any amino acid excluding C

SEQ ID NO: 575 - protein, 43 aa, Synechococcus PCC7002; identical to SEQ ID NO: 431
  SITE 36: note = X is A, I, V, L, Y, G or F
  SITE 37: note = X is any amino acid excluding C

SEQ ID NO: 576 - protein, 42 aa, Thermosynechococcus elongatus; identical to SEQ ID NO: 432
  SITE 35: note = X is A, I, V, L, Y, G or F
  SITE 36: note = X is any amino acid excluding C

SEQ ID NO: 577 - protein, 43 aa, Trichodesmium erythraeum; identical to SEQ ID NO: 433
  SITE 36: note = X is A, I, V, L, Y, G or F
  SITE 37: note = X is any amino acid excluding C

SEQ ID NO: 578 - protein, 42 aa, Thermosynechococcus vulcanus; identical to SEQ ID NO: 434
  SITE 35: note = X is A, I, V, L, Y, G or F
  SITE 36: note = X is any amino acid excluding C

SEQ ID NO: 579 - protein, 43 aa, Nostoc punctiforme; identical to SEQ ID NO: 417
  SITE 36: note = X is A, I, V, L, Y, G or F
  SITE 37: note = X is A, V, I, S, M, H, L, F, Y, G or W or can be a unnatural aliphatic amino acid residue such as Nle, Abu, Nva, 2-aminopentoic acid,or 2-aminohexaanoic acid

SEQ ID NO: 580 - protein, 43 aa, Synechocystis PCC6803; identical to SEQ ID NO: 418
  SITE 36: note = X is A, I, V, L, Y, G or F
  SITE 37: note = X is A, V, I, S, M, H, L, F, Y, G or W or can be a unnatural aliphatic amino acid residue such as Nle, Abu, Nva, 2-aminopentoic acid,or 2-aminohexaanoic acid

SEQ ID NO: 581 - protein, 43 aa, Aphanothece halophytica; identical to SEQ ID NO: 419
  SITE 36: note = X is A, I, V, L, Y, G or F
  SITE 37: note = X is A, V, I, S, M, H, L, F, Y, G or W or can be a unnatural aliphatic amino acid residue such as Nle, Abu, Nva, 2-aminopentoic acid,or 2-aminohexaanoic acid

SEQ ID NO: 582 - protein, 43 aa, Aphanizomenon ovalisporum; identical to SEQ ID NO: 420
  SITE 36: note = X is A, I, V, L, Y, G or F
  SITE 37: note = X is A, V, I, S, M, H, L, F, Y, G or W or can be a unnatural aliphatic amino acid residue such as Nle, Abu, Nva, 2-aminopentoic acid,or 2-aminohexaanoic acid

SEQ ID NO: 583 - protein, 43 aa, Anabaena PCC7120; identical to SEQ ID NO: 421
  SITE 36: note = X is A, I, V, L, Y, G or F
  SITE 37: note = X is A, V, I, S, M, H, L, F, Y, G or W or can be a unnatural aliphatic amino acid residue such as Nle, Abu, Nva, 2-aminopentoic acid,or 2-aminohexaanoic acid

SEQ ID NO: 584 - protein, 43 aa, Anabaena variabilis; identical to SEQ ID NO: 422
  SITE 36: note = X is A, I, V, L, Y, G or F
  SITE 37: note = X is A, V, I, S, M, H, L, F, Y, G or W or can be a unnatural aliphatic amino acid residue such as Nle, Abu, Nva, 2-aminopentoic acid,or 2-aminohexaanoic acid

SEQ ID NO: 585 - protein, 43 aa, Cylindrospermopsis raciborskii; identical to SEQ ID NO: 423
  SITE 36: note = X is A, I, V, L, Y, G or F
  SITE 37: note = X is A, V, I, S, M, H, L, F, Y, G or W or can be a unnatural aliphatic amino acid residue such as Nle, Abu, Nva, 2-aminopentoic acid,or 2-aminohexaanoic acid

SEQ ID NO: 586 - protein, 43 aa, Cyanothece CCY0110; identical to SEQ ID NO: 424
  SITE 36: note = X is A, I, V, L, Y, G or F
  SITE 37: note = X is A, V, I, S, M, H, L, F, Y, G or W or can be a unnatural aliphatic amino acid residue such as Nle, Abu, Nva, 2-aminopentoic acid,or 2-aminohexaanoic acid

SEQ ID NO: 587 - protein, 43 aa, Cyanothece PCC8801; identical to SEQ ID NO: 425
  SITE 36: note = X is A, I, V, L, Y, G or F
  SITE 37: note = X is A, V, I, S, M, H, L, F, Y, G or W or can be a unnatural aliphatic amino acid residue such as Nle, Abu, Nva, 2-aminopentoic acid,or 2-aminohexaanoic acid

SEQ ID NO: 588 - protein, 43 aa, Crocosphaera watsonii; identical to SEQ ID NO: 426
  SITE 36: note = X is A, I, V, L, Y, G or F
  SITE 37: note = X is A, V, I, S, M, H, L, F, Y, G or W or can be a unnatural aliphatic amino acid residue such as Nle, Abu, Nva, 2-aminopentoic acid,or 2-aminohexaanoic acid

SEQ ID NO: 589 - protein, 43 aa, Microcystis aeruginosa; identical to SEQ ID NO: 427
  SITE 36: note = X is A, I, V, L, Y, G or F
  SITE 37: note = X is A, V, I, S, M, H, L, F, Y, G or W or can be a unnatural aliphatic amino acid residue such as Nle, Abu, Nva, 2-aminopentoic acid,or 2-aminohexaanoic acid

SEQ ID NO: 590 - protein, 43 aa, Microcoleus chthonoplastes; identical to SEQ ID NO: 428
  SITE 36: note = X is A, I, V, L, Y, G or F
  SITE 37: note = X is A, V, I, S, M, H, L, F, Y, G or W or can be a unnatural aliphatic amino acid residue such as Nle, Abu, Nva, 2-aminopentoic acid,or 2-aminohexaanoic acid

SEQ ID NO: 591 - protein, 43 aa, Oscillatoria limnetica; identical to SEQ ID NO: 428
  SITE 36: note = X is A, I, V, L, Y, G or F
  SITE 37: note = X is A, V, I, S, M, H, L, F, Y, G or W or can be a unnatural aliphatic amino acid residue such as Nle, Abu, Nva, 2-aminopentoic acid,or 2-aminohexaanoic acid

SEQ ID NO: 592 - protein, 43 aa, Synechococcus elongatus; identical to SEQ ID NO: 430
  SITE 36: note = X is A, I, V, L, Y, G or F
  SITE 37: note = X is A, V, I, S, M, H, L, F, Y, G or W or can be a unnatural aliphatic amino acid residue such as Nle, Abu, Nva, 2-aminopentoic acid,or 2-aminohexaanoic acid

SEQ ID NO: 593 - protein, 43 aa, Synechococcus PCC7002; identical to SEQ ID NO: 431
  SITE 36: note = X is A, I, V, L, Y, G or F
  SITE 37: note = X is A, V, I, S, M, H, L, F, Y, G or W or can be a unnatural aliphatic amino acid residue such as Nle, Abu, Nva, 2-aminopentoic acid,or 2-aminohexaanoic acid

SEQ ID NO: 594 - protein, 42 aa, Thermosynechococcus elongatus; identical to SEQ ID NO: 432
  SITE 35: note = X is A, I, V, L, Y, G or F
  SITE 36: note = X is A, V, I, S, M, H, L, F, Y, G or W or can be a unnatural aliphatic amino acid residue such as Nle, Abu, Nva, 2-aminopentoic acid,or 2-aminohexaanoic acid

SEQ ID NO: 595 - protein, 43 aa, Trichodesmium erythraeum; identical to SEQ ID NO: 433
  SITE 36: note = X is A, I, V, L, Y, G or F
  SITE 37: note = X is A, V, I, S, M, H, L, F, Y, G or W or can be a unnatural aliphatic amino acid residue such as Nle, Abu, Nva, 2-aminopentoic acid,or 2-aminohexaanoic acid

SEQ ID NO: 596 - protein, 42 aa, Thermosynechococcus vulcanus; identical to SEQ ID NO: 434
  SITE 35: note = X is A, I, V, L, Y, G or F
  SITE 36: note = X is A, V, I, S, M, H, L, F, Y, G or W or can be a unnatural aliphatic amino acid residue such as Nle, Abu, Nva, 2-aminopentoic acid,or 2-aminohexaanoic acid

SEQ ID NO: 597 - protein, 43 aa, Nostoc punctiforme; identical to SEQ ID NO: 417
  SITE 36: note = X is A, I, V, L, Y, G or F
  SITE 37: note = X is A, I, V, L, Y, G or F

SEQ ID NO: 598 - protein, 43 aa, Synechocystis PCC6803; identical to SEQ ID NO: 418
  SITE 36: note = X is A, I, V, L, Y, G or F
  SITE 37: note = X is A, I, V, L, Y, G or F

SEQ ID NO: 599 - protein, 43 aa, Aphanothece halophytica; identical to SEQ ID NO: 419
  SITE 36: note = X is A, I, V, L, Y, G or F
  SITE 37: note = X is A, I, V, L, Y, G or F

SEQ ID NO: 600 - protein, 43 aa, Aphanizomenon ovalisporum; identical to SEQ ID NO: 420
  SITE 36: note = X is A, I, V, L, Y, G or F
  SITE 37: note = X is A, I, V, L, Y, G or F

SEQ ID NO: 601 - protein, 43 aa, Anabaena PCC7120; identical to SEQ ID NO: 421
  SITE 36: note = X is A, I, V, L, Y, G or F
  SITE 37: note = X is A, I, V, L, Y, G or F

SEQ ID NO: 602 - protein, 43 aa, Anabaena variabilis; identical to SEQ ID NO: 422
  SITE 36: note = X is A, I, V, L, Y, G or F
  SITE 37: note = X is A, I, V, L, Y, G or F

SEQ ID NO: 603 - protein, 43 aa, Cylindrospermopsis raciborskii; identical to SEQ ID NO: 423
  SITE 36: note = X is A, I, V, L, Y, G or F
  SITE 37: note = X is A, I, V, L, Y, G or F

SEQ ID NO: 604 - protein, 43 aa, Cyanothece CCY0110; identical to SEQ ID NO: 424
  SITE 36: note = X is A, I, V, L, Y, G or F
  SITE 37: note = X is A, I, V, L, Y, G or F

SEQ ID NO: 605 - protein, 43 aa, Cyanothece PCC8801; identical to SEQ ID NO: 425
  SITE 36: note = X is A, I, V, L, Y, G or F
  SITE 37: note = X is A, I, V, L, Y, G or F

SEQ ID NO: 606 - protein, 43 aa, Crocosphaera watsonii; identical to SEQ ID NO: 426
  SITE 36: note = X is A, I, V, L, Y, G or F
  SITE 37: note = X is A, I, V, L, Y, G or F

SEQ ID NO: 607 - protein, 43 aa, Microcystis aeruginosa; identical to SEQ ID NO: 427
  SITE 36: note = X is A, I, V, L, Y, G or F
  SITE 37: note = X is A, I, V, L, Y, G or F

SEQ ID NO: 608 - protein, 43 aa, Microcoleus chthonoplastes; identical to SEQ ID NO: 428
  SITE 36: note = X is A, I, V, L, Y, G or F
  SITE 37: note = X is A, I, V, L, Y, G or F

SEQ ID NO: 609 - protein, 43 aa, Oscillatoria limnetica; identical to SEQ ID NO: 428
  SITE 36: note = X is A, I, V, L, Y, G or F
  SITE 37: note = X is A, I, V, L, Y, G or F

SEQ ID NO: 610 - protein, 43 aa, Synechococcus elongatus; identical to SEQ ID NO: 430
  SITE 36: note = X is A, I, V, L, Y, G or F
  SITE 37: note = X is A, I, V, L, Y, G or F

SEQ ID NO: 611 - protein, 43 aa, Synechococcus PCC7002; identical to SEQ ID NO: 431
  SITE 36: note = X is A, I, V, L, Y, G or F
  SITE 37: note = X is A, I, V, L, Y, G or F

SEQ ID NO: 612 - protein, 42 aa, Thermosynechococcus elongatus; identical to SEQ ID NO: 432
  SITE 35: note = X is A, I, V, L, Y, G or F
  SITE 36: note = X is A, I, V, L, Y, G or F

SEQ ID NO: 613 - protein, 43 aa, Trichodesmium erythraeum; identical to SEQ ID NO: 433
  SITE 36: note = X is A, I, V, L, Y, G or F
  SITE 37: note = X is A, I, V, L, Y, G or F

SEQ ID NO: 614 - protein, 42 aa, Thermosynechococcus vulcanus; identical to SEQ ID NO: 434
  SITE 35: note = X is A, I, V, L, Y, G or F
  SITE 36: note = X is A, I, V, L, Y, G or F

SEQ ID NO: 615 - protein, 43 aa, Nostoc punctiforme; identical to SEQ ID NO: 471
  SITE 36: note = X is A, I, V, L, Y, G or F

SEQ ID NO: 616 - protein, 43 aa, Synechocystis PCC6803; identical to SEQ ID NO: 472
  SITE 36: note = X is A, I, V, L, Y, G or F

SEQ ID NO: 617 - protein, 43 aa, Aphanothece halophytica; identical to SEQ ID NO: 473
  SITE 36: note = X is A, I, V, L, Y, G or F

SEQ ID NO: 618 - protein, 43 aa, Aphanizomenon ovalisporum; identical to SEQ ID NO: 474
  SITE 36: note = X is A, I, V, L, Y, G or F

SEQ ID NO: 619 - protein, 43 aa, Anabaena PCC7120; identical to SEQ ID NO: 475
  SITE 36: note = X is A, I, V, L, Y, G or F

SEQ ID NO: 620 - protein, 43 aa, Anabaena variabilis; identical to SEQ ID NO: 476
  SITE 36: note = X is A, I, V, L, Y, G or F

SEQ ID NO: 621 - protein, 43 aa, Cylindrospermopsis raciborskii; identical to SEQ ID NO: 477
  SITE 36: note = X is A, I, V, L, Y, G or F

SEQ ID NO: 622 - protein, 43 aa, Cyanothece CCY0110; identical to SEQ ID NO: 478
  SITE 36: note = X is A, I, V, L, Y, G or F

SEQ ID NO: 623 - protein, 43 aa, Cyanothece PCC8801; identical to SEQ ID NO: 479
  SITE 36: note = X is A, I, V, L, Y, G or F

SEQ ID NO: 624 - protein, 43 aa, Crocosphaera watsonii; identical to SEQ ID NO: 480
  SITE 36: note = X is A, I, V, L, Y, G or F

SEQ ID NO: 625 - protein, 43 aa, Microcystis aeruginosa; identical to SEQ ID NO: 481
  SITE 36: note = X is A, I, V, L, Y, G or F

SEQ ID NO: 626 - protein, 43 aa, Microcoleus chthonoplastes; identical to SEQ ID NO: 482
  SITE 36: note = X is A, I, V, L, Y, G or F

SEQ ID NO: 627 - protein, 43 aa, Oscillatoria limnetica; identical to SEQ ID NO: 482
  SITE 36: note = X is A, I, V, L, Y, G or F

SEQ ID NO: 628 - protein, 43 aa, Synechococcus elongatus; identical to SEQ ID NO: 484
  SITE 36: note = X is A, I, V, L, Y, G or F

SEQ ID NO: 629 - protein, 43 aa, Synechococcus PCC7002; identical to SEQ ID NO: 485
  SITE 36: note = X is A, I, V, L, Y, G or F

SEQ ID NO: 630 - protein, 42 aa, Thermosynechococcus elongatus; identical to SEQ ID NO: 486
  SITE 35: note = X is A, I, V, L, Y, G or F

SEQ ID NO: 631 - protein, 43 aa, Trichodesmium erythraeum; identical to SEQ ID NO: 487
  SITE 36: note = X is A, I, V, L, Y, G or F

SEQ ID NO: 632 - protein, 42 aa, Thermosynechococcus vulcanus; identical to SEQ ID NO: 488
  SITE 35: note = X is A, I, V, L, Y, G or F

SEQ ID NO: 633 - protein, 43 aa, Nostoc punctiforme
  SITE 37: note = X is any amino acid excluding C
MIKIATRKYLGKQNVYDIGVERDHNFALKNGFIASAXFNSGGC

SEQ ID NO: 634 - protein, 39 aa, Synechocystis PCC6803; identical to SEQ ID NO: 346
  SITE 37: note = X is any amino acid excluding C

SEQ ID NO: 635 - protein, 39 aa, Aphanothece halophytica; identical to SEQ ID NO: 347
  SITE 37: note = X is any amino acid excluding C

SEQ ID NO: 636 - protein, 43 aa, Aphanizomenon ovalisporum
  SITE 37: note = X is any amino acid excluding C
MVKITARKFVGRENVYDIGVEHHHNFAIKNGLIASAXFNSGGC

SEQ ID NO: 637 - protein, 43 aa, Anabaena PCC7120
  SITE 37: note = X is any amino acid excluding C
MIKIASRKFLGVENVYDIGVRRDHNFFIKNGLIASAXFNSGGC

SEQ ID NO: 638 - protein, 43 aa, Anabaena variabilis
  SITE 37: note = X is any amino acid excluding C
MIKIASRKFLGVENVYDIGVGRDHNFFVKNGLIASAXFNSGGC

SEQ ID NO: 639 - protein, 43 aa, Cylindrospermopsis raciborskii
  SITE 37: note = X is any amino acid excluding C
MVKIVSRRYLGKADVYDIGVAKDHNFIIKNGLVASAXFNSGGC

SEQ ID NO: 640 - protein, 43 aa, Cyanothece CCY0110
  SITE 37: note = X is any amino acid excluding C
MVKIIERRSLGKQNVYDIGVEKDHNFLLSNNLIASAXFNSGGC

SEQ ID NO: 641 - protein, 43 aa, Cyanothece PCC8801
  SITE 37: note = X is any amino acid excluding C
MVKIVSYRSLGKQFVYDIGVAQDHNFLLANGSIASAXFNSGGC

SEQ ID NO: 642 - protein, 43 aa, Crocosphaera watsonii
  SITE 37: note = X is any amino acid excluding C
MVKIIGCRSLGTQKVYDIGVEKDHNFLLANGSIASAXFNSGGC

SEQ ID NO: 643 - protein, 43 aa, Microcystis aeruginosa
  SITE 37: note = X is any amino acid excluding C
MVKIIGRQSLGRKPVYDIGVEKDHNFLLGNGLIASAXFNSGGC

SEQ ID NO: 644 - protein, 43 aa, Microcoleus chthonoplastes
  SITE 37: note = X is any amino acid excluding C
MVKIVRRQSLGVQNVYDIGVEKDHNFCLASGEIASAXFNSGGC

SEQ ID NO: 645 - protein, 43 aa, Oscillatoria limnetica; identical to SEQ ID NO: 644
  SITE 37: note = X is any amino acid excluding C

SEQ ID NO: 646 - protein, 43 aa, Synechococcus elongatus
  SITE 37: note = X is any amino acid excluding C
MVKIVRRRSLGVQPVYDLGVATVHNFVLANGLVASAXFNSGGC

SEQ ID NO: 647 - protein, 43 aa, Synechococcus PCC7002
  SITE 37: note = X is any amino acid excluding C
MVKIIRRKFIGHAPTYDIGLSQDHNFLLGQGLIAAAXFNSGGC

SEQ ID NO: 648 - protein, 42 aa, Thermosynechococcus elongatus
  SITE 36: note = X is any amino acid excluding C
MKIVGRRLMGWQAVYDIGLAADHNFVLANGAIAAAXFNSGGC

SEQ ID NO: 649 - protein, 43 aa, Trichodesmium erythraeum
  SITE 37: note = X is any amino acid excluding C
MVKIVSRKLAKTENVYDIGVTKDHNFVLANGLIASAXFNSGGC

SEQ ID NO: 650 - protein, 42 aa, Thermosynechococcus vulcanus
  SITE 36: note = X is any amino acid excluding C
MKIVGRRLVGWQAVYDIGLAGDHNFLLANGAIAAAXFNSGGC

SEQ ID NO: 651 - protein, 43 aa, Nostoc punctiforme; identical to SEQ ID NO: 633
  SITE 37: note = X is A, V, I, S, M, H, L, F, Y, G or W or can be a unnatural aliphatic amino acid residue such as Nle, Abu, Nva, 2-aminopentoic acid,or 2-aminohexaanoic acid

SEQ ID NO: 652 - protein, 43 aa, Synechocystis PCC6803
  SITE 37: note = X is A, V, I, S, M, H, L, F, Y, G or W or can be a unnatural aliphatic amino acid residue such as Nle, Abu, Nva, 2-aminopentoic acid,or 2-aminohexaanoic acid
MVKVIGRRSLGVQRIFDIGLPQDHNFLLANGAIAAAXFNSGGC

SEQ ID NO: 653 - protein, 43 aa, Aphanothece halophytica
  SITE 37: note = X is A, V, I, S, M, H, L, F, Y, G or W or can be a unnatural aliphatic amino acid residue such as Nle, Abu, Nva, 2-aminopentoic acid,or 2-aminohexaanoic acid
MVKIIKRQSLGRQNVYDVCVETDHNFVLANGCVASAXFNSGGC

SEQ ID NO: 654 - protein, 43 aa, Aphanizomenon ovalisporum; identical to SEQ ID NO: 636
  SITE 37: note = X is A, V, I, S, M, H, L, F, Y, G or W or can be a unnatural aliphatic amino acid residue such as Nle, Abu, Nva, 2-aminopentoic acid,or 2-aminohexaanoic acid

SEQ ID NO: 655 - protein, 43 aa, Anabaena PCC7120; identical to SEQ ID NO: 637
  SITE 37: note = X is A, V, I, S, M, H, L, F, Y, G or W or can be a unnatural aliphatic amino acid residue such as Nle, Abu, Nva, 2-aminopentoic acid,or 2-aminohexaanoic acid

SEQ ID NO: 656 - protein, 43 aa, Anabaena variabilis; identical to SEQ ID NO: 638
  SITE 37: note = X is A, V, I, S, M, H, L, F, Y, G or W or can be a unnatural aliphatic amino acid residue such as Nle, Abu, Nva, 2-aminopentoic acid,or 2-aminohexaanoic acid

SEQ ID NO: 657 - protein, 43 aa, Cylindrospermopsis raciborskii; identical to SEQ ID NO: 639
  SITE 37: note = X is A, V, I, S, M, H, L, F, Y, G or W or can be a unnatural aliphatic amino acid residue such as Nle, Abu, Nva, 2-aminopentoic acid,or 2-aminohexaanoic acid

SEQ ID NO: 658 - protein, 43 aa, Cyanothece CCY0110; identical to SEQ ID NO: 640
  SITE 37: note = X is A, V, I, S, M, H, L, F, Y, G or W or can be a unnatural aliphatic amino acid residue such as Nle, Abu, Nva, 2-aminopentoic acid,or 2-aminohexaanoic acid

SEQ ID NO: 659 - protein, 43 aa, Cyanothece PCC8801; identical to SEQ ID NO: 641
  SITE 37: note = X is A, V, I, S, M, H, L, F, Y, G or W or can be a unnatural aliphatic amino acid residue such as Nle, Abu, Nva, 2-aminopentoic acid,or 2-aminohexaanoic acid

SEQ ID NO: 660 - protein, 43 aa, Crocosphaera watsonii; identical to SEQ ID NO: 642
  SITE 37: note = X is A, V, I, S, M, H, L, F, Y, G or W or can be a unnatural aliphatic amino acid residue such as Nle, Abu, Nva, 2-aminopentoic acid,or 2-aminohexaanoic acid

SEQ ID NO: 661 - protein, 43 aa, Microcystis aeruginosa; identical to SEQ ID NO: 643
  SITE 37: note = X is A, V, I, S, M, H, L, F, Y, G or W or can be a unnatural aliphatic amino acid residue such as Nle, Abu, Nva, 2-aminopentoic acid,or 2-aminohexaanoic acid

SEQ ID NO: 662 - protein, 43 aa, Microcoleus chthonoplastes; identical to SEQ ID NO: 644
  SITE 37: note = X is A, V, I, S, M, H, L, F, Y, G or W or can be a unnatural aliphatic amino acid residue such as Nle, Abu, Nva, 2-aminopentoic acid,or 2-aminohexaanoic acid

SEQ ID NO: 663 - protein, 43 aa, Oscillatoria limnetica; identical to SEQ ID NO: 644
  SITE 37: note = X is A, V, I, S, M, H, L, F, Y, G or W or can be a unnatural aliphatic amino acid residue such as Nle, Abu, Nva, 2-aminopentoic acid,or 2-aminohexaanoic acid

SEQ ID NO: 664 - protein, 43 aa, Synechococcus elongatus; identical to SEQ ID NO: 646
  SITE 37: note = X is A, V, I, S, M, H, L, F, Y, G or W or can be a unnatural aliphatic amino acid residue such as Nle, Abu, Nva, 2-aminopentoic acid,or 2-aminohexaanoic acid

SEQ ID NO: 665 - protein, 43 aa, Synechococcus PCC7002; identical to SEQ ID NO: 647
  SITE 37: note = X is A, V, I, S, M, H, L, F, Y, G or W or can be a unnatural aliphatic amino acid residue such as Nle, Abu, Nva, 2-aminopentoic acid,or 2-aminohexaanoic acid

SEQ ID NO: 666 - protein, 42 aa, Thermosynechococcus elongatus; identical to SEQ ID NO: 648
  SITE 36: note = X is A, V, I, S, M, H, L, F, Y, G or W or can be a unnatural aliphatic amino acid residue such as Nle, Abu, Nva, 2-aminopentoic acid,or 2-aminohexaanoic acid

SEQ ID NO: 667 - protein, 43 aa, Trichodesmium erythraeum; identical to SEQ ID NO: 649
  SITE 37: note = X is A, V, I, S, M, H, L, F, Y, G or W or can be a unnatural aliphatic amino acid residue such as Nle, Abu, Nva, 2-aminopentoic acid,or 2-aminohexaanoic acid

SEQ ID NO: 668 - protein, 42 aa, Thermosynechococcus vulcanus; identical to SEQ ID NO: 650
  SITE 36: note = X is A, V, I, S, M, H, L, F, Y, G or W or can be a unnatural aliphatic amino acid residue such as Nle, Abu, Nva, 2-aminopentoic acid,or 2-aminohexaanoic acid

SEQ ID NO: 669 - protein, 43 aa, Nostoc punctiforme; identical to SEQ ID NO: 633
  SITE 37: note = X is A, I, V, L, Y, G or F

SEQ ID NO: 670 - protein, 43 aa, Synechocystis PCC6803; identical to SEQ ID NO: 652
  SITE 37: note = X is A, I, V, L, Y, G or F

SEQ ID NO: 671 - protein, 43 aa, Aphanothece halophytica; identical to SEQ ID NO: 653
  SITE 37: note = X is A, I, V, L, Y, G or F

SEQ ID NO: 672 - protein, 43 aa, Aphanizomenon ovalisporum; identical to SEQ ID NO: 636
  SITE 37: note = X is A, I, V, L, Y, G or F

SEQ ID NO: 673 - protein, 43 aa, Anabaena PCC7120; identical to SEQ ID NO: 637
  SITE 37: note = X is A, I, V, L, Y, G or F

SEQ ID NO: 674 - protein, 43 aa, Anabaena variabilis; identical to SEQ ID NO: 638
  SITE 37: note = X is A, I, V, L, Y, G or F

SEQ ID NO: 675 - protein, 43 aa, Cylindrospermopsis raciborskii; identical to SEQ ID NO: 639
  SITE 37: note = X is A, I, V, L, Y, G or F

SEQ ID NO: 676 - protein, 43 aa, Cyanothece CCY0110; identical to SEQ ID NO: 640
  SITE 37: note = X is A, I, V, L, Y, G or F

SEQ ID NO: 677 - protein, 43 aa, Cyanothece PCC8801; identical to SEQ ID NO: 641
  SITE 37: note = X is A, I, V, L, Y, G or F

SEQ ID NO: 678 - protein, 43 aa, Crocosphaera watsonii; identical to SEQ ID NO: 642
  SITE 37: note = X is A, I, V, L, Y, G or F

SEQ ID NO: 679 - protein, 43 aa, Microcystis aeruginosa; identical to SEQ ID NO: 643
  SITE 37: note = X is A, I, V, L, Y, G or F

SEQ ID NO: 680 - protein, 43 aa, Microcoleus chthonoplastes; identical to SEQ ID NO: 644
  SITE 37: note = X is A, I, V, L, Y, G or F

SEQ ID NO: 681 - protein, 43 aa, Oscillatoria limnetica; identical to SEQ ID NO: 644
  SITE 37: note = X is A, I, V, L, Y, G or F

SEQ ID NO: 682 - protein, 43 aa, Synechococcus elongatus; identical to SEQ ID NO: 646
  SITE 37: note = X is A, I, V, L, Y, G or F

SEQ ID NO: 683 - protein, 43 aa, Synechococcus PCC7002; identical to SEQ ID NO: 647
  SITE 37: note = X is A, I, V, L, Y, G or F

SEQ ID NO: 684 - protein, 42 aa, Thermosynechococcus elongatus; identical to SEQ ID NO: 648
  SITE 36: note = X is A, I, V, L, Y, G or F

SEQ ID NO: 685 - protein, 43 aa, Trichodesmium erythraeum; identical to SEQ ID NO: 649
  SITE 37: note = X is A, I, V, L, Y, G or F

SEQ ID NO: 686 - protein, 42 aa, Thermosynechococcus vulcanus; identical to SEQ ID NO: 650
  SITE 36: note = X is A, I, V, L, Y, G or F

SEQ ID NO: 687 - protein, 43 aa, Nostoc punctiforme
MIKIATRKYLGKQNVYDIGVERDHNFALKNGFIASAAFNSGGC

SEQ ID NO: 688 - protein, 43 aa, Synechocystis PCC6803
MVKVIGRRSLGVQRIFDIGLPQDHNFLLANGAIAAAAFNSGGC

SEQ ID NO: 689 - protein, 43 aa, Aphanothece halophytica
MVKIIKRQSLGRQNVYDVCVETDHNFVLANGCVASAAFNSGGC

SEQ ID NO: 690 - protein, 43 aa, Aphanizomenon ovalisporum
MVKITARKFVGRENVYDIGVEHHHNFAIKNGLIASAAFNSGGC

SEQ ID NO: 691 - protein, 39 aa, Anabaena PCC7120; identical to SEQ ID NO: 403

SEQ ID NO: 692 - protein, 43 aa, Anabaena variabilis
MIKIASRKFLGVENVYDIGVGRDHNFFVKNGLIASAAFNSGGC

SEQ ID NO: 693 - protein, 43 aa, Cylindrospermopsis raciborskii
MVKIVSRRYLGKADVYDIGVAKDHNFIIKNGLVASAAFNSGGC

SEQ ID NO: 694 - protein, 43 aa, Cyanothece CCY0110
MVKIIERRSLGKQNVYDIGVEKDHNFLLSNNLIASAAFNSGGC

SEQ ID NO: 695 - protein, 43 aa, Cyanothece PCC8801
MVKIVSYRSLGKQFVYDIGVAQDHNFLLANGSIASAAFNSGGC

SEQ ID NO: 696 - protein, 43 aa, Crocosphaera watsonii
MVKIIGCRSLGTQKVYDIGVEKDHNFLLANGSIASAAFNSGGC

SEQ ID NO: 697 - protein, 43 aa, Microcystis aeruginosa
MVKIIGRQSLGRKPVYDIGVEKDHNFLLGNGLIASAAFNSGGC

SEQ ID NO: 698 - protein, 43 aa, Microcoleus chthonoplastes
MVKIVRRQSLGVQNVYDIGVEKDHNFCLASGEIASAAFNSGGC

SEQ ID NO: 699 - protein, 43 aa, Oscillatoria limnetica; identical to SEQ ID NO: 698

SEQ ID NO: 700 - protein, 43 aa, Synechococcus elongatus
MVKIVRRRSLGVQPVYDLGVATVHNFVLANGLVASAAFNSGGC

SEQ ID NO: 701 - protein, 43 aa, Synechococcus PCC7002
MVKIIRRKFIGHAPTYDIGLSQDHNFLLGQGLIAAAAFNSGGC

SEQ ID NO: 702 - protein, 42 aa, Thermosynechococcus elongatus
MKIVGRRLMGWQAVYDIGLAADHNFVLANGAIAAAAFNSGGC

SEQ ID NO: 703 - protein, 43 aa, Trichodesmium erythraeum
MVKIVSRKLAKTENVYDIGVTKDHNFVLANGLIASAAFNSGGC

SEQ ID NO: 704 - protein, 42 aa, Thermosynechococcus vulcanus
MKIVGRRLVGWQAVYDIGLAGDHNFLLANGAIAAAAFNSGGC

SEQ ID NO: 705 - protein, 4 aa, synthetic construct
  source 1..4: note = Linker
SGGC

SEQ ID NO: 706 - protein, 8 aa, synthetic construct
  source 1..8: note = Linker
AAFNSGGC

SEQ ID NO: 707 - protein, 35 aa, synthetic construct
  source 1..35: note = C-fragment consensus sequence
VKIISRQSLGKQNVYDIGVEKDHNFLLANGLIASN

SEQ ID NO: 708 - protein, 35 aa, synthetic construct
  SITE 35: note = X is any amino acid exclusing N and/or Q
  source 1..35: note = C-fragment consensus sequence
VKIISRQSLGKQNVYDIGVEKDHNFLLANGLIASX

SEQ ID NO: 709 - protein, 35 aa, synthetic construct; identical to SEQ ID NO: 708
  SITE 35: note = X is A, V, I, S, M, H, L, F, Y, G or W or can be a unnatural aliphatic amino acid residue such as Nle, Abu, Nva, 2-aminopentoic acid,or 2-aminohexaanoic acid
  source 1..35: note = C-fragment consensus sequence

SEQ ID NO: 710 - protein, 35 aa, synthetic construct; identical to SEQ ID NO: 708
  SITE 35: note = X is A, I, V, L, Y, G or F
  source 1..35: note = C-fragment consensus sequence

SEQ ID NO: 711 - protein, 35 aa, synthetic construct
  source 1..35: note = C-fragment consensus sequence
VKIISRQSLGKQNVYDIGVEKDHNFLLANGLIASA

SEQ ID NO: 712 - protein, 36 aa, synthetic construct
  SITE 35: note = X is any amino acid exclusing N and/or Q
  SITE 36: note = X is any amino acid excluding C
  source 1..36: note = C-fragment consensus sequence
VKIISRQSLGKQNVYDIGVEKDHNFLLANGLIASXX

SEQ ID NO: 713 - protein, 36 aa, synthetic construct; identical to SEQ ID NO: 712
  SITE 35: note = X is any amino acid excluding N and/or Q
  SITE 36: note = X is A, V, I, S, M, H, L, F, Y, G or W or can be a unnatural aliphatic amino acid residue such as Nle, Abu, Nva, 2-aminopentoic acid,or 2-aminohexaanoic acid
  source 1..36: note = C-fragment consensus sequence

SEQ ID NO: 714 - protein, 36 aa, synthetic construct; identical to SEQ ID NO: 712
  SITE 35: note = X is any amino acid excluding N and/or Q
  SITE 36: note = X is A, I, V, L, Y, G or F
  source 1..36: note = C-fragment consensus sequence

SEQ ID NO: 715 - protein, 36 aa, synthetic construct
  SITE 35: note = X is any amino acid excluding N and/or Q
  source 1..36: note = C-fragment consensus sequence
VKIISRQSLGKQNVYDIGVEKDHNFLLANGLIASXA

SEQ ID NO: 716 - protein, 36 aa, synthetic construct; identical to SEQ ID NO: 712
  SITE 35: note = X is A, V, I, S, M, H, L, F, Y, G or W or can be a unnatural aliphatic amino acid residue such as Nle, Abu, Nva, 2-aminopentoic acid,or 2-aminohexaanoic acid
  SITE 36: note = X is any amino acid excluding C
  source 1..36: note = C-fragment consensus sequence

SEQ ID NO: 717 - protein, 36 aa, synthetic construct; identical to SEQ ID NO: 712
  SITE 35: note = X is A, V, I, S, M, H, L, F, Y, G or W or can be a unnatural aliphatic amino acid residue such as Nle, Abu, Nva, 2-aminopentoic acid,or 2-aminohexaanoic acid
  SITE 36: note = X is A, V, I, S, M, H, L, F, Y, G or W or can be a unnatural aliphatic amino acid residue such as Nle, Abu, Nva, 2-aminopentoic acid,or 2-aminohexaanoic acid
  source 1..36: note = C-fragment consensus sequence

SEQ ID NO: 718 - protein, 36 aa, synthetic construct; identical to SEQ ID NO: 712
  SITE 35: note = X is A, V, I, S, M, H, L, F, Y, G or W or can be a unnatural aliphatic amino acid residue such as Nle, Abu, Nva, 2-aminopentoic acid,or 2-aminohexaanoic acid
  SITE 36: note = X is A, I, V, L, Y, G or F
  source 1..36: note = C-fragment consensus sequence

SEQ ID NO: 719 - protein, 36 aa, synthetic construct; identical to SEQ ID NO: 715
  SITE 35: note = X is A, V, I, S, M, H, L, F, Y, G or W or can be a unnatural aliphatic amino acid residue such as Nle, Abu, Nva, 2-aminopentoic acid,or 2-aminohexaanoic acid
  source 1..36: note = C-fragment consensus sequence

SEQ ID NO: 720 - protein, 36 aa, synthetic construct; identical to SEQ ID NO: 712
  SITE 35: note = X is A, I, V, L, Y, G or F
  SITE 36: note = X is any amino acid excluding C
  source 1..36: note = C-fragment consensus sequence

SEQ ID NO: 721 - protein, 36 aa, synthetic construct; identical to SEQ ID NO: 712
  SITE 35: note = X is A, I, V, L, Y, G or F
  SITE 36: note = X is A, V, I, S, M, H, L, F, Y, G or W or can be a unnatural aliphatic amino acid residue such as Nle, Abu, Nva, 2-aminopentoic acid,or 2-aminohexaanoic acid
  source 1..36: note = C-fragment consensus sequence

SEQ ID NO: 722 - protein, 36 aa, synthetic construct; identical to SEQ ID NO: 712
  SITE 35: note = X is A, I, V, L, Y, G or F
  SITE 36: note = X is A, I, V, L, Y, G or F
  source 1..36: note = C-fragment consensus sequence

SEQ ID NO: 723 - protein, 36 aa, synthetic construct; identical to SEQ ID NO: 715
  SITE 35: note = X is A, I, V, L, Y, G or F
  source 1..36: note = C-fragment consensus sequence

SEQ ID NO: 724 - protein, 36 aa, synthetic construct
  SITE 36: note = X is any amino acid excluding C
  source 1..36: note = C-fragment consensus sequence
VKIISRQSLGKQNVYDIGVEKDHNFLLANGLIASAX

SEQ ID NO: 725 - protein, 36 aa, synthetic construct; identical to SEQ ID NO: 724
  SITE 36: note = X is A, V, I, S, M, H, L, F, Y, G or W or can be a unnatural aliphatic amino acid residue such as Nle, Abu, Nva, 2-aminopentoic acid,or 2-aminohexaanoic acid
  source 1..36: note = C-fragment consensus sequence

SEQ ID NO: 726 - protein, 36 aa, synthetic construct; identical to SEQ ID NO: 724
  SITE 36: note = X is A, I, V, L, Y, G or F
  source 1..36: note = C-fragment consensus sequence

SEQ ID NO: 727 - protein, 36 aa, synthetic construct
  source 1..36: note = C-fragment consensus sequence
VKIISRQSLGKQNVYDIGVEKDHNFLLANGLIASAA

SEQ ID NO: 728 - protein, 38 aa, synthetic construct
  SITE 35: note = X is any amino acid exclusing N and/or Q
  SITE 36: note = X is any amino acid excluding C
  source 1..38: note = C-fragment consensus sequence
VKIISRQSLGKQNVYDIGVEKDHNFLLANGLIASXXFN

SEQ ID NO: 729 - protein, 38 aa, synthetic construct; identical to SEQ ID NO: 728
  SITE 35: note = X is any amino acid excluding N and/or Q
  SITE 36: note = X is A, V, I, S, M, H, L, F, Y, G or W or can be a unnatural aliphatic amino acid residue such as Nle, Abu, Nva, 2-aminopentoic acid,or 2-aminohexaanoic acid
  source 1..38: note = C-fragment consensus sequence

SEQ ID NO: 730 - protein, 38 aa, synthetic construct; identical to SEQ ID NO: 728
  SITE 35: note = X is any amino acid excluding N and/or Q
  SITE 36: note = X is A, I, V, L, Y, G or F
  source 1..38: note = C-fragment consensus sequence

SEQ ID NO: 731 - protein, 38 aa, synthetic construct
  SITE 35: note = X is any amino acid excluding N and/or Q
  source 1..38: note = C-fragment consensus sequence
VKIISRQSLGKQNVYDIGVEKDHNFLLANGLIASXAFN

SEQ ID NO: 732 - protein, 38 aa, synthetic construct; identical to SEQ ID NO: 728
  SITE 35: note = X is A, V, I, S, M, H, L, F, Y, G or W or can be a unnatural aliphatic amino acid residue such as Nle, Abu, Nva, 2-aminopentoic acid,or 2-aminohexaanoic acid
  SITE 36: note = X is any amino acid excluding C
  source 1..38: note = C-fragment consensus sequence

SEQ ID NO: 733 - protein, 38 aa, synthetic construct; identical to SEQ ID NO: 728
  SITE 35: note = X is A, V, I, S, M, H, L, F, Y, G or W or can be a unnatural aliphatic amino acid residue such as Nle, Abu, Nva, 2-aminopentoic acid,or 2-aminohexaanoic acid
  SITE 36: note = X is A, V, I, S, M, H, L, F, Y, G or W or can be a unnatural aliphatic amino acid residue such as Nle, Abu, Nva, 2-aminopentoic acid,or 2-aminohexaanoic acid
  source 1..38: note = C-fragment consensus sequence

SEQ ID NO: 734 - protein, 38 aa, synthetic construct; identical to SEQ ID NO: 728
  SITE 35: note = X is A, V, I, S, M, H, L, F, Y, G or W or can be a unnatural aliphatic amino acid residue such as Nle, Abu, Nva, 2-aminopentoic acid,or 2-aminohexaanoic acid
  SITE 36: note = X is A, I, V, L, Y, G or F
  source 1..38: note = C-fragment consensus sequence

SEQ ID NO: 735 - protein, 38 aa, synthetic construct; identical to SEQ ID NO: 731
  SITE 35: note = X is A, V, I, S, M, H, L, F, Y, G or W or can be a unnatural aliphatic amino acid residue such as Nle, Abu, Nva, 2-aminopentoic acid,or 2-aminohexaanoic acid
  source 1..38: note = C-fragment consensus sequence

SEQ ID NO: 736 - protein, 38 aa, synthetic construct; identical to SEQ ID NO: 728
  SITE 35: note = X is A, I, V, L, Y, G or F
  SITE 36: note = X is any amino acid excluding C
  source 1..38: note = C-fragment consensus sequence

SEQ ID NO: 737 - protein, 38 aa, synthetic construct; identical to SEQ ID NO: 728
  SITE 35: note = X is A, I, V, L, Y, G or F
  SITE 36: note = X is A, V, I, S, M, H, L, F, Y, G or W or can be a unnatural aliphatic amino acid residue such as Nle, Abu, Nva, 2-aminopentoic acid,or 2-aminohexaanoic acid
  source 1..38: note = C-fragment consensus sequence

SEQ ID NO: 738 - protein, 38 aa, synthetic construct; identical to SEQ ID NO: 728
  SITE 35: note = X is A, I, V, L, Y, G or F
  SITE 36: note = X is A, I, V, L, Y, G or F
  source 1..38: note = C-fragment consensus sequence

SEQ ID NO: 739 - protein, 38 aa, synthetic construct; identical to SEQ ID NO: 731
  SITE 35: note = X is A, I, V, L, Y, G or F
  source 1..38: note = C-fragment consensus sequence

SEQ ID NO: 740 - protein, 38 aa, synthetic construct
  SITE 36: note = X is any amino acid excluding C
  source 1..38: note = C-fragment consensus sequence
VKIISRQSLGKQNVYDIGVEKDHNFLLANGLIASAXFN

SEQ ID NO: 741 - protein, 38 aa, synthetic construct; identical to SEQ ID NO: 740
  SITE 36: note = X is A, V, I, S, M, H, L, F, Y, G or W or can be a unnatural aliphatic amino acid residue such as Nle, Abu, Nva, 2-aminopentoic acid,or 2-aminohexaanoic acid
  source 1..38: note = C-fragment consensus sequence

SEQ ID NO: 742 - protein, 38 aa, synthetic construct; identical to SEQ ID NO: 740
  SITE 36: note = X is A, I, V, L, Y, G or F
  source 1..38: note = C-fragment consensus sequence

SEQ ID NO: 743 - protein, 38 aa, synthetic construct
  source 1..38: note = C-fragment consensus sequence
VKIISRQSLGKQNVYDIGVEKDHNFLLANGLIASAAFN

SEQ ID NO: 744 - protein, 42 aa, synthetic construct
  SITE 35: note = X is any amino acid exclusing N and/or Q
  SITE 36: note = X is any amino acid excluding C
  source 1..42: note = C-fragment consensus sequence
VKIISRQSLGKQNVYDIGVEKDHNFLLANGLIASXXFNSGGC

SEQ ID NO: 745 - protein, 42 aa, synthetic construct; identical to SEQ ID NO: 744
  SITE 35: note = X is any amino acid excluding N and/or Q
  SITE 36: note = X is A, V, I, S, M, H, L, F, Y, G or W or can be a unnatural aliphatic amino acid residue such as Nle, Abu, Nva, 2-aminopentoic acid,or 2-aminohexaanoic acid
  source 1..42: note = C-fragment consensus sequence

SEQ ID NO: 746 - protein, 42 aa, synthetic construct; identical to SEQ ID NO: 744
  SITE 35: note = X is any amino acid excluding N and/or Q
  SITE 36: note = X is A, I, V, L, Y, G or F
  source 1..42: note = C-fragment consensus sequence

SEQ ID NO: 747 - protein, 42 aa, synthetic construct
  SITE 35: note = X is any amino acid excluding N and/or Q
  source 1..42: note = C-fragment consensus sequence
VKIISRQSLGKQNVYDIGVEKDHNFLLANGLIASXAFNSGGC

SEQ ID NO: 748 - protein, 42 aa, synthetic construct; identical to SEQ ID NO: 744
  SITE 35: note = X is A, V, I, S, M, H, L, F, Y, G or W or can be a unnatural aliphatic amino acid residue such as Nle, Abu, Nva, 2-aminopentoic acid,or 2-aminohexaanoic acid
  SITE 36: note = X is any amino acid excluding C
  source 1..42: note = C-fragment consensus sequence

SEQ ID NO: 749 - protein, 42 aa, synthetic construct; identical to SEQ ID NO: 744
  SITE 35: note = X is A, V, I, S, M, H, L, F, Y, G or W or can be a unnatural aliphatic amino acid residue such as Nle, Abu, Nva, 2-aminopentoic acid,or 2-aminohexaanoic acid
  SITE 36: note = X is A, V, I, S, M, H, L, F, Y, G or W or can be a unnatural aliphatic amino acid residue such as Nle, Abu, Nva, 2-aminopentoic acid,or 2-aminohexaanoic acid
  source 1..42: note = C-fragment consensus sequence

SEQ ID NO: 750 - protein, 42 aa, synthetic construct; identical to SEQ ID NO: 744
  SITE 35: note = X is A, V, I, S, M, H, L, F, Y, G or W or can be a unnatural aliphatic amino acid residue such as Nle, Abu, Nva, 2-aminopentoic acid,or 2-aminohexaanoic acid
  SITE 36: note = X is A, I, V, L, Y, G or F
  source 1..42: note = C-fragment consensus sequence

SEQ ID NO: 751 - protein, 42 aa, synthetic construct; identical to SEQ ID NO: 747
  SITE 35: note = X is A, V, I, S, M, H, L, F, Y, G or W or can be a unnatural aliphatic amino acid residue such as Nle, Abu, Nva, 2-aminopentoic acid,or 2-aminohexaanoic acid
  source 1..42: note = C-fragment consensus sequence

SEQ ID NO: 752 - protein, 42 aa, synthetic construct; identical to SEQ ID NO: 744
  SITE 35: note = X is A, I, V, L, Y, G or F
  SITE 36: note = X is any amino acid excluding C
  source 1..42: note = C-fragment consensus sequence

SEQ ID NO: 753 - protein, 42 aa, synthetic construct; identical to SEQ ID NO: 744
  SITE 35: note = X is A, I, V, L, Y, G or F
  SITE 36: note = X is A, V, I, S, M, H, L, F, Y, G or W or can be a unnatural aliphatic amino acid residue such as Nle, Abu, Nva, 2-aminopentoic acid,or 2-aminohexaanoic acid
  source 1..42: note = C-fragment consensus sequence

SEQ ID NO: 754 - protein, 42 aa, synthetic construct; identical to SEQ ID NO: 744
  SITE 35: note = X is A, I, V, L, Y, G or F
  SITE 36: note = X is A, I, V, L, Y, G or F
  source 1..42: note = C-fragment consensus sequence

SEQ ID NO: 755 - protein, 42 aa, synthetic construct; identical to SEQ ID NO: 747
  SITE 35: note = X is A, I, V, L, Y, G or F
  source 1..42: note = C-fragment consensus sequence

SEQ ID NO: 756 - protein, 42 aa, synthetic construct
  SITE 36: note = X is any amino acid excluding C
  source 1..42: note = C-fragment consensus sequence
VKIISRQSLGKQNVYDIGVEKDHNFLLANGLIASAXFNSGGC

SEQ ID NO: 757 - protein, 42 aa, synthetic construct; identical to SEQ ID NO: 756
  SITE 36: note = X is A, V, I, S, M, H, L, F, Y, G or W or can be a unnatural aliphatic amino acid residue such as Nle, Abu, Nva, 2-aminopentoic acid,or 2-aminohexaanoic acid
  source 1..42: note = C-fragment consensus sequence

SEQ ID NO: 758 - protein, 42 aa, synthetic construct; identical to SEQ ID NO: 756
  SITE 36: note = X is A, I, V, L, Y, G or F
  source 1..42: note = C-fragment consensus sequence

SEQ ID NO: 759 - protein, 42 aa, synthetic construct
  source 1..42: note = C-fragment consensus sequence
VKIISRQSLGKQNVYDIGVEKDHNFLLANGLIASAAFNSGGC

SEQ ID NO: 760 - protein, 10 aa, synthetic construct
  source 1..10: note = c-myc epitope tag
EQKLISEEDL

SEQ ID NO: 761 - protein, 102 aa, synthetic construct
  SITE 28: note = X is A or S
  SITE 59: note = X is A or S
  source 1..102: note = N-fragment modified consensus sequence
CLSYDTEILTVEYGAVPIGKIVEENIEXTVYSVDENGFVYTQPIAQWHDRGEQEVFEYXLEDGSTIRATKDHKFMTEDGEMLPIDEIFEQGLDLKQVKGLPD

SEQ ID NO: 762 - protein, 196 aa, synthetic construct
  source 1..196: note = Synthetic peptide
MHHHHHHGGMQIFVKTLTGKTITLEVESSDTIDNVKSKIQDKEGIPPDQQELIFAGKQLEDGRTLSDYNIQKESTLHLVLRLRGGGGGGKFAEYCLSYETEILTVEYGLLPIGKIVEKRIECTVYSVDNNGNIYTQPVAQWHDRGEQEVFEYCLEDGSLIRATKDHKFMTVDGQMLPIDEIFERELDLMRVDNLPN

SEQ ID NO: 763 - protein, 192 aa, synthetic construct
  source 1..192: note = Synthetic peptide
MHHHHHHGGMQIFVKTLTGKTITLEVESSDTIDNVKSKIQDKEGIPPDQQELIFAGKQLEDGRTLSDYNIQKESTLHLVLRLRGGKFAEYCLSYETEILTVEYGLLPIGKIVEKRIECTVYSVDNNGNIYTQPVAQWHDRGEQEVFEYCLEDGSLIRATKDHKFMTVDGQMLPIDEIFERELDLMRVDNLPN

SEQ ID NO: 764 - protein, 156 aa, synthetic construct
  source 1..156: note = Synthetic peptide
GIKIATRKYLGKQNVYDIGVERDHNFALKNGFIASNCFNSGLVPRGSASMSDSEVNQEAKPEVKPEVKPETHINLKVSDGSSEIFFKIKKTTPLRRLMEAFAKRQGKEMDSLRFLYDGIRIQADQTPEDLDMEDNDIIEAHREQIGGYPYDVPDYA

SEQ ID NO: 765 - protein, 283 aa, synthetic construct
  source 1..283: note = Synthetic peptide
MQIFVKTLTGKTITLEVEPSDTIENVKAKIQDKEGIPPDQQRLIFAGKQLEDGRTLSDYNIQKESTLHLVLRLRGGCITGDALVALPEGESVRIADIVPGARPNSDNAIDLKVLDRHGNPVLADRLFHSGEHPVYTVRTVEGLRVTGTANHPLLCLVDVAGVPTLLWKLIDEIKPGDYAVIQRSAFSVDCAGFARGKPEFAPTTYTVGVPGLVRFLEAHHRDPDAQAIADELTDGRFYYAKVASVTDAGVQPVYSLRVDTADHAFITNGFVSHATEAHHHHHH

SEQ ID NO: 766 - protein, 222 aa, synthetic construct
  source 1..222: note = Synthetic peptide
MQIFVKTLTGKTITLEVEPSDTIENVKAKIQDKEGIPPDQQRLIFAGKQLEDGRTLSDYNIQKESTLHLVLRLRGGCLSYETEILTVEYGLLPIGKIVEKRIECTVYSVDNNGNIYTQPVAQWHDRGEQEVFEYCLEDGSLIRATKDHKFMTVDGQMLPIDEIFERELDLMRVDNLPNIKIATRKYLGKQNVYDIGVERDHNFALKNGFIASAAFNHHHHHH

SEQ ID NO: 767 - protein, 222 aa, synthetic construct
  source 1..222: note = Synthetic peptide
MQIFVKTLTGKTITLEVEPSDTIENVKAKIQDKEGIPPDQQRLIFAGKQLEDGRTLSDYNIQKESTLHLVLRLRGGCLSYDTEVLTVEYGFVPIGEIVDKGIECSVFSIDSNGIVYTQPIAQWHHRGKQEVFEYCLEDGSIIKATKDHKFMTQDGKMLPIDEIFEQELDLLQVKGLPEIKIASRKFLGVENVYDIGVGRDHNFFVKNGLIASAAFNHHHHHH

SEQ ID NO: 768 - protein, 224 aa, synthetic construct
  source 1..224: note = Synthetic peptide
MQIFVKTLTGKTITLEVEPSDTIENVKAKIQDKEGIPPDQQRLIFAGKQLEDGRTLSDYNIQKESTLHLVLRLRGGCLSYDTQILTVEYGAVAIGEIVEKQIECTVYSVDENGYVYTQPIAQWHNRGEQEVFEYLLEDGATIRATKDHKFMTDEDQMLPIDQIFEQGLELKQVEVLQPVFVKIVRRQSLGVQNVYDIGVEKDHNFCLASGEIASAAFNHHHHHH

SEQ ID NO: 769 - protein, 283 aa, synthetic construct
  source 1..283: note = Synthetic peptide
MQIFVKTLTGKTITLEVEPSDTIENVKAKIQDKEGIPPDQQRLIFAGKQLEDGRTLSDYNIQKESTLHLVLRLRGGCITGDALVALPEGESVRIADIVPGARPNSDNAIDLKVLDRHGNPVLADRLFHSGEHPVYTVRTVEGLRVTGTANHPLLCLVDVAGVPTLLWKLIDEIKPGDYAVIQRSAFSVDCAGFARGKPEFAPTTYTVGVPGLVRFLEAHHRDPDAQAIADELTDGRFYYAKVASVTDAGVQPVYSLRVDTADHAFITNGFVSHAAEAHHHHHH

SEQ ID NO: 770 - protein, 201 aa, synthetic construct
  source 1..201: note = Synthetic peptide
MEAIAKYDFKATADDELSFKRGDILKVLNEECDQNWYKAELNGKDGFIPKNYIEMCLSYDTEVLTVEYGFVPIGEIVDKGIECSVFSIDSNGIVYTQPIAQWHHRGKQEVFEYCLEDGSIIKATKDHKFMTQDGKMLPIDEIFEQELDLLQVKGLPEIKIASRKFLGVENVYDIGVGRDHNFFVKNGLIASAAFNHHHHHH

SEQ ID NO: 771 - protein, 202 aa, synthetic construct
  source 1..202: note = Synthetic peptide
MEAIAKYDFKATADDELSFKRGDILKVLNEECDQNWYKAELNGKDGFIPKNYIEMGCLSYDTEVLTVEYGFVPIGEIVDKGIECSVFSIDSNGIVYTQPIAQWHHRGKQEVFEYCLEDGSIIKATKDHKFMTQDGKMLPIDEIFEQELDLLQVKGLPEIKIASRKFLGVENVYDIGVGRDHNFFVKNGLIASAAFNHHHHHH

SEQ ID NO: 772 - protein, 203 aa, synthetic construct
  source 1..203: note = Synthetic peptide
MEAIAKYDFKATADDELSFKRGDILKVLNEECDQNWYKAELNGKDGFIPKNYIEMCLSYDTQILTVEYGAVAIGEIVEKQIECTVYSVDENGYVYTQPIAQWHNRGEQEVFEYLLEDGATIRATKDHKFMTDEDQMLPIDQIFEQGLELKQVEVLQPVFVKIVRRQSLGVQNVYDIGVEKDHNFCLASGEIASAAFNHHHHHH

SEQ ID NO: 773 - protein, 243 aa, synthetic construct
  source 1..243: note = Synthetic peptide
MLEKHSWYHGPVSRNAAEYLLSSGINGSFLVRESESSPGQRSISLRYEGRVYHYRINTASDGKLYVSSESRFNTLAELVHHHSTVADGLITTLHYPACLSYDTEVLTVEYGFVPIGEIVDKGIECSVFSIDSNGIVYTQPIAQWHHRGKQEVFEYCLEDGSIIKATKDHKFMTQDGKMLPIDEIFEQELDLLQVKGLPEIKIASRKFLGVENVYDIGVGRDHNFFVKNGLIASAAFNHHHHHH

SEQ ID NO: 774 - protein, 385 aa, synthetic construct
  source 1..385: note = Synthetic peptide
MVSKGEELFTGVVPILVELDGDVNGHKFSVSGEGEGDATYGKLTLKFICTTGKLPVPWPTLVTTLTYGVQCFSRYPDHMKQHDFFKSAMPEGYVQERTIFFKDDGNYKTRAEVKFEGDTLVNRIELKGIDFKEDGNILGHKLEYNYNSHNVYIMADKQKNGIKVNFKIRHNIEDGSVQLADHYQQNTPIGDGPVLLPDNHYLSTQSALSKDPNEKRDHMVLLEFVTAAGITLGMDELYKCLSYDTEVLTVEYGFVPIGEIVDKGIECSVFSIDSNGIVYTQPIAQWHHRGKQEVFEYCLEDGSIIKATKDHKFMTQDGKMLPIDEIFEQELDLLQVKGLPEIKIASRKFLGVENVYDIGVGRDHNFFVKNGLIASAAFNHHHHHH

SEQ ID NO: 775 - protein, 505 aa, synthetic construct
  source 1..505: note = Synthetic peptide
MVNPGTKSKLPKPVQDLIKMIFDVESMKKAMVEYEIDLQKMPLGKLSKRQIQAAYSILSEVQQAVSQGSSDSQILDLSNRFYTLIPHDFGMKKPPLLNNADSVQAKAEMLDNLLDIEVAYSLLRGGSDDSSKDPIDVNYEKLKTDIKVVDRDSEEAEIIRKYVKNTHATTHNAYDLEVIDIFKIEREGECQRYKPFKQLHNRRLLWHGSRTTNFAGILSQGLRIAPPEAPVTGYMFGKGIYFADMVSKSANYCHTSQGDPIGLILLGEVALGNMYELKHASHISKLPKGKHSVKGLGKTTPDPSANISLDGVDVPLGTGISSGVNDTSLLYNEYIVYDIAQVNLKYLLKLKFNFKTSLWCLSYDTEVLTVEYGFVPIGEIVDKGIECSVFSIDSNGIVYTQPIAQWHHRGKQEVFEYCLEDGSIIKATKDHKFMTQDGKMLPIDEIFEQELDLLQVKGLPEIKIASRKFLGVENVYDIGVGRDHNFFVKNGLIASAAFNHHHHHH

SEQ ID NO: 776 - protein, 39 aa, Nostoc punctiforme
MIKIATRKYLGKQNVYDIGVERDHNDALKNGFIASNCFN

SEQ ID NO: 777 - protein, 43 aa, Nostoc punctiforme
MIKIATRKYLGKQNVYDIGVERDHNDALKNGFIASAAFNSGGC